European Patent Application EP 4 467 984 A2, published November 27, 2024. Title: Fibrosis Biomarker Assay. Applicant: Nordic Biosciences A/S. The sequence listing filed with the application follows.

SEQUENCE LISTING (2248 sequences)

SEQ ID NO: 1 - protein, 10 aa, Homo sapiens
PGIPGRNGDP

SEQ ID NO: 2 - protein, 10 aa, Homo sapiens
ESCPTGPQNY

SEQ ID NO: 3 - protein, 10 aa, Homo sapiens
PKGDTGPRGP

SEQ ID NO: 4 - protein, 25 aa, Homo sapiens
  MOD_RES 16..17: note = proline or hydroxyproline
  MOD_RES 20: note = proline or hydroxyproline
VPGPMGPSGPRGLPGXXGAXGPQGF

SEQ ID NO: 5 - protein, 26 aa, Homo sapiens
  MOD_RES 17..18: note = proline or hydroxyproline
  MOD_RES 21: note = proline or hydroxyproline
SVPGPMGPSGPRGLPGXXGAXGPQGF

SEQ ID NO: 6 - protein, 28 aa, Homo sapiens
  MOD_RES 8: note = methionine or oxidised methionine
  MOD_RES 19..20: note = proline or hydroxyproline
  MOD_RES 23: note = proline or hydroxyproline
GISVPGPXGPSGPRGLPGXXGAXGPQGF

SEQ ID NO: 7 - protein, 29 aa, Homo sapiens
  MOD_RES 23..24: note = proline or hydroxy proline
  MOD_RES 26: note = proline or hydroxy proline
GFQGPPGEPGEPGASGPMGPRGXXGXPGK

SEQ ID NO: 8 - protein, 25 aa, Homo sapiens
  MOD_RES 5: note = methionine or oxidised methionine
  MOD_RES 17: note = proline or hydroxyproline
  MOD_RES 20: note = proline or hydroxyproline
VPGPXGPSGPRGLPGPXGAXGPQGF

SEQ ID NO: 9 - protein, 37 aa, Homo sapiens
  MOD_RES 17: note = lysine or hydroxylysine
  MOD_RES 23: note = proline or hydroxyproline
  MOD_RES 29: note = proline or hydroxyproline
FSGLDGAKGDAGPAGPXGEPGSXGENGAXGQMGPRGL

SEQ ID NO: 10 - protein, 17 aa, Homo sapiens
  MOD_RES 3: note = proline or hydroxyproline
  MOD_RES 9: note = proline or hydroxyproline
  MOD_RES 12: note = proline or hydroxyproline
GLXGERGRXGAXGPAGA

SEQ ID NO: 11 - protein, 23 aa, Homo sapiens
  MOD_RES 6: note = proline or hydroxyproline
  MOD_RES 9: note = proline or hydroxyproline
  MOD_RES 20: note = proline or hydroxyproline
GLTGSXGSXGPDGKTGPPGXAGQ

SEQ ID NO: 12 - protein, 31 aa, Homo sapiens
  MOD_RES 5: note = proline or hydroxyproline
  MOD_RES 14: note = proline or hydroxyproline
  MOD_RES 20: note = proline or hydroxyproline
  MOD_RES 26: note = proline or hydroxyproline
ERGSXGPAGPKGSXGEAGRXGEAGLXGAKGL

SEQ ID NO: 13 - protein, 32 aa, Homo sapiens
  MOD_RES 6: note = proline or hydroxyproline
  MOD_RES 8: note = proline or hydroxyproline
  MOD_RES 21: note = proline or hydroxyproline
  MOD_RES 27: note = proline or hydroxyproline
  MOD_RES 31: note = proline or hydroxyproline
GERGSXGXAGPKGSPGEAGRXGEAGLXGAKGL

SEQ ID NO: 14 - protein, 23 aa, Homo sapiens
  MOD_RES 6: note = proline or hydroxyproline
  MOD_RES 9: note = proline or hydroxyproline
  MOD_RES 20: note = proline or hydroxyproline
GLTGSXGSXGPDGKTGPPGXAGQ

SEQ ID NO: 15 - protein, 35 aa, Homo sapiens
GLTGSPGSPGPDGKTGPPGPAGQDGRPGPPGPPGA

SEQ ID NO: 16 - protein, 38 aa, Homo sapiens
GLTGSPGSPGPDGKTGPPGPAGQDGRPGPPGPPGARGQ

SEQ ID NO: 17 - protein, 17 aa, Homo sapiens
GQDGRPGPPGPPGARGQ

SEQ ID NO: 18 - protein, 38 aa, Homo sapiens; identical to SEQ ID NO: 16

SEQ ID NO: 19 - protein, 33 aa, Homo sapiens
  MOD_RES 12: note = proline or hydroxyproline
  MOD_RES 30: note = proline or hydroxyproline
GKDGEAGAQGPXGPAGPAGERGEQGPAGSXGFQ

SEQ ID NO: 20 - protein, 15 aa, Homo sapiens
  MOD_RES 12: note = proline or hydroxyproline
GERGEQGPAGSXGFQ

SEQ ID NO: 21 - protein, 47 aa, Homo sapiens
  MOD_RES 5: note = proline or hydroxyproline
  MOD_RES 7: note = proline or hydroxyproline
  MOD_RES 40: note = proline or hydroxyproline
  MOD_RES 44: note = proline or hydroxyproline
ERGVXGXPGAVGPAGKDGEAGAQGPPGPAGPAGERGEQGXAGSXGFQ

SEQ ID NO: 22 - protein, 10 aa, Homo sapiens
PKGDTGPRGP

SEQ ID NO: 23 - protein, 6 aa, Homo sapiens
ISVPGP

SEQ ID NO: 24 - protein, 6 aa, Homo sapiens
VPGPMG

SEQ ID NO: 25 - protein, 6 aa, Homo sapiens
PGPMGP

SEQ ID NO: 26 - protein, 6 aa, Homo sapiens
LPGPGG

SEQ ID NO: 27 - protein, 6 aa, Homo sapiens
FQGPPG

SEQ ID NO: 28 - protein, 6 aa, Homo sapiens
KNGDDG

SEQ ID NO: 29 - protein, 6 aa, Homo sapiens
ARGLPG

SEQ ID NO: 30 - protein, 6 aa, Homo sapiens
SGLDGA

SEQ ID NO: 31 - protein, 6 aa, Homo sapiens
LDGAKG

SEQ ID NO: 32 - protein, 6 aa, Homo sapiens
LPGERG

SEQ ID NO: 33 - protein, 6 aa, Homo sapiens
VRGEPG

SEQ ID NO: 34 - protein, 6 aa, Homo sapiens
PGAKGA

SEQ ID NO: 35 - protein, 6 aa, Homo sapiens
GGPPGP

SEQ ID NO: 36 - protein, 6 aa, Homo sapiens
NSGEPG

SEQ ID NO: 37 - protein, 6 aa, Homo sapiens
DGVAGP

SEQ ID NO: 38 - protein, 6 aa, Homo sapiens
ERGSPG

SEQ ID NO: 39 - protein, 6 aa, Homo sapiens
LTGSPG

SEQ ID NO: 40 - protein, 6 aa, Homo sapiens
QDGRPG

SEQ ID NO: 41 - protein, 6 aa, Homo sapiens
RGVPGP

SEQ ID NO: 42 - protein, 6 aa, Homo sapiens
VGPAGK

SEQ ID NO: 43 - protein, 6 aa, Homo sapiens
ERGEQG

SEQ ID NO: 44 - protein, 6 aa, Homo sapiens
RGEQGP

SEQ ID NO: 45 - protein, 6 aa, Homo sapiens
PGERGV

SEQ ID NO: 46 - protein, 6 aa, Homo sapiens
ANGAPG

SEQ ID NO: 47 - protein, 6 aa, Homo sapiens
ARGAPG

SEQ ID NO: 48 - protein, 6 aa, Homo sapiens
PGDRGE

SEQ ID NO: 49 - protein, 6 aa, Homo sapiens
AKGDAG

SEQ ID NO: 50 - protein, 6 aa, Homo sapiens
PIGNVG

SEQ ID NO: 51 - protein, 6 aa, Homo sapiens
AAGRVG

SEQ ID NO: 52 - protein, 6 aa, Homo sapiens
  MOD_RES 2: note = proline or hydroxyproline
  MOD_RES 4: note = proline or hydroxyproline
PXGXAG

SEQ ID NO: 53 - protein, 6 aa, Homo sapiens
GADGPA

SEQ ID NO: 54 - protein, 6 aa, Homo sapiens
GPQGIA

SEQ ID NO: 55 - protein, 6 aa, Homo sapiens
GQRGVV

SEQ ID NO: 56 - protein, 6 aa, Homo sapiens
QRGVVG

SEQ ID NO: 57 - protein, 6 aa, Homo sapiens
GLPGQR

SEQ ID NO: 58 - protein, 6 aa, Homo sapiens
PGLPGP

SEQ ID NO: 59 - protein, 6 aa, Homo sapiens
PMGPPG

SEQ ID NO: 60 - protein, 6 aa, Homo sapiens
MGPPGL

SEQ ID NO: 61 - protein, 6 aa, Homo sapiens
DKGETG

SEQ ID NO: 62 - protein, 6 aa, Homo sapiens
  MOD_RES 5: note = proline or hydroxyproline
LQGPXG

SEQ ID NO: 63 - protein, 6 aa, Homo sapiens
SAGAPG

SEQ ID NO: 64 - protein, 6 aa, Homo sapiens
RTGDAG

SEQ ID NO: 65 - protein, 5 aa, Homo sapiens
FDFSF

SEQ ID NO: 66 - protein, 5 aa, Homo sapiens
FDFSF

SEQ ID NO: 67 - protein, 6 aa, Homo sapiens
ATGAAG

SEQ ID NO: 68 - protein, 6 aa, Homo sapiens
AKGEAG

SEQ ID NO: 69 - protein, 6 aa, Homo sapiens
GIAGAP

SEQ ID NO: 70 - protein, 6 aa, Homo sapiens
IAGAPG

SEQ ID NO: 71 - protein, 6 aa, Homo sapiens
VQGPPG

SEQ ID NO: 72 - protein, 6 aa, Homo sapiens
  MOD_RES 4..5: note = proline or hydroxproline
LPGXXG

SEQ ID NO: 73 - protein, 6 aa, Homo sapiens
AGPKGS

SEQ ID NO: 74 - protein, 6 aa, Homo sapiens
RGSPGP

SEQ ID NO: 75 - protein, 6 aa, Homo sapiens
FAGPPG

SEQ ID NO: 76 - protein, 6 aa, Homo sapiens
QAGVMG

SEQ ID NO: 77 - protein, 6 aa, Homo sapiens
ARGQAG

SEQ ID NO: 78 - protein, 6 aa, Homo sapiens
NVGAPG

SEQ ID NO: 79 - protein, 6 aa, Homo sapiens
PAGERG

SEQ ID NO: 80 - protein, 6 aa, Homo sapiens
KDGEAG

SEQ ID NO: 81 - protein, 6 aa, Homo sapiens
GEVGPP

SEQ ID NO: 82 - protein, 6 aa, Homo sapiens
ARGERG

SEQ ID NO: 83 - protein, 6 aa, Homo sapiens
QGLPGP

SEQ ID NO: 84 - protein, 6 aa, Homo sapiens
IAGQRG

SEQ ID NO: 85 - protein, 6 aa, Homo sapiens
LTGPIG

SEQ ID NO: 86 - protein, 6 aa, Homo sapiens
AGLPGP

SEQ ID NO: 87 - protein, 6 aa, Homo sapiens
RGVVGL

SEQ ID NO: 88 - protein, 6 aa, Homo sapiens
AGPPGA

SEQ ID NO: 89 - protein, 6 aa, Homo sapiens
LAGPPG

SEQ ID NO: 90 - protein, 6 aa, Homo sapiens
EPGKQG

SEQ ID NO: 91 - protein, 6 aa, Homo sapiens
ATGFPG

SEQ ID NO: 92 - protein, 6 aa, Homo sapiens
PSGASG

SEQ ID NO: 93 - protein, 6 aa, Homo sapiens
GKQGPS

SEQ ID NO: 94 - protein, 6 aa, Homo sapiens
GPPGPA

SEQ ID NO: 95 - protein, 6 aa, Homo sapiens
AGQRGV

SEQ ID NO: 96 - protein, 6 aa, Homo sapiens
ARGPAG

SEQ ID NO: 97 - protein, 6 aa, Homo sapiens
ASGPAG

SEQ ID NO: 98 - protein, 6 aa, Homo sapiens
VVGLPG

SEQ ID NO: 99 - protein, 6 aa, Homo sapiens
VGPPGP

SEQ ID NO: 100 - skipped

SEQ ID NO: 101 - protein, 6 aa, Homo sapiens
QLSYGY

SEQ ID NO: 102 - protein, 6 aa, Homo sapiens
EKSTGG

SEQ ID NO: 103 - protein, 6 aa, Homo sapiens
PPGPQG

SEQ ID NO: 104 - protein, 6 aa, Homo sapiens
KGHRGF

SEQ ID NO: 105 - protein, 6 aa, Homo sapiens
PSGPRG

SEQ ID NO: 106 - protein, 6 aa, Homo sapiens
APGPQG

SEQ ID NO: 107 - protein, 6 aa, Homo sapiens
APGPAG

SEQ ID NO: 108 - protein, 6 aa, Homo sapiens
FPGAVG

SEQ ID NO: 109 - protein, 6 aa, Homo sapiens
SEGPQG

SEQ ID NO: 110 - protein, 6 aa, Homo sapiens
GANGAP

SEQ ID NO: 111 - protein, 6 aa, Homo sapiens
GARGLA

SEQ ID NO: 112 - protein, 6 aa, Homo sapiens
SGPQGP

SEQ ID NO: 113 - protein, 6 aa, Homo sapiens
EPGPVG

SEQ ID NO: 114 - protein, 6 aa, Homo sapiens
EPGPTG

SEQ ID NO: 115 - protein, 6 aa, Homo sapiens
RGFPGA

SEQ ID NO: 116 - protein, 6 aa, Homo sapiens
KGPAGE

SEQ ID NO: 117 - protein, 6 aa, Homo sapiens
IPGAPG

SEQ ID NO: 118 - protein, 6 aa, Homo sapiens
LPGAKG

SEQ ID NO: 119 - skipped

SEQ ID NO: 120 - protein, 6 aa, Homo sapiens
PPGARG

SEQ ID NO: 121 - protein, 6 aa, Homo sapiens
PGKAGE

SEQ ID NO: 122 - protein, 6 aa, Homo sapiens
AVGPAG

SEQ ID NO: 123 - protein, 6 aa, Homo sapiens
PAGPAG

SEQ ID NO: 124 - protein, 6 aa, Homo sapiens
AGPAGE

SEQ ID NO: 125 - protein, 6 aa, Homo sapiens
APGPDG

SEQ ID NO: 126 - protein, 6 aa, Homo sapiens
RGERGF

SEQ ID NO: 127 - protein, 6 aa, Homo sapiens
PAGPRG

SEQ ID NO: 128 - protein, 6 aa, Homo sapiens
KDGVRG

SEQ ID NO: 129 - protein, 6 aa, Homo sapiens
PAGPTG

SEQ ID NO: 130 - protein, 6 aa, Homo sapiens
TGARGA

SEQ ID NO: 131 - protein, 6 aa, Homo sapiens
PGPAGF

SEQ ID NO: 132 - protein, 6 aa, Homo sapiens
EPGDAG

SEQ ID NO: 133 - protein, 6 aa, Homo sapiens
PAGPPG

SEQ ID NO: 134 - protein, 6 aa, Homo sapiens
SAGPPG

SEQ ID NO: 135 - protein, 6 aa, Homo sapiens
DGTSGH

SEQ ID NO: 136 - protein, 6 aa, Homo sapiens
NAGPPG

SEQ ID NO: 137 - protein, 6 aa, Homo sapiens
FRGPAG

SEQ ID NO: 138 - protein, 6 aa, Homo sapiens
GEKGSP

SEQ ID NO: 139 - protein, 6 aa, Homo sapiens
GAPGTP

SEQ ID NO: 140 - protein, 6 aa, Homo sapiens
PGPQGI

SEQ ID NO: 141 - protein, 6 aa, Homo sapiens
PQGIAG

SEQ ID NO: 142 - protein, 6 aa, Homo sapiens
AIGSPG

SEQ ID NO: 143 - protein, 6 aa, Homo sapiens
QPGVMG

SEQ ID NO: 144 - protein, 6 aa, Homo sapiens
AGPPGM

SEQ ID NO: 145 - protein, 6 aa, Homo sapiens
GPSGEP

SEQ ID NO: 146 - protein, 6 aa, Homo sapiens
ERGPPG

SEQ ID NO: 147 - protein, 6 aa, Homo sapiens
RGPPGP

SEQ ID NO: 148 - protein, 6 aa, Homo sapiens
PVGPVG

SEQ ID NO: 149 - protein, 6 aa, Homo sapiens
PQGPRG

SEQ ID NO: 150 - protein, 6 aa, Homo sapiens
HRGFSG

SEQ ID NO: 151 - protein, 6 aa, Homo sapiens
EQGPSG

SEQ ID NO: 152 - protein, 6 aa, Homo sapiens
PRGPPG

SEQ ID NO: 153 - protein, 6 aa, Homo sapiens
PPGPRG

SEQ ID NO: 154 - protein, 6 aa, Homo sapiens
  MOD_RES 2: note = Hydroxyproline
  MOD_RES 5..6: note = Hydroxyproline
VGGLAG

SEQ ID NO: 155 - protein, 6 aa, Homo sapiens
GPPSAG

SEQ ID NO: 156 - protein, 6 aa, Homo sapiens
PPSAGF

SEQ ID NO: 157 - skipped

SEQ ID NO: 158 - protein, 6 aa, Homo sapiens
VKGERG

SEQ ID NO: 159 - protein, 6 aa, Homo sapiens
TPGPQG

SEQ ID NO: 160 - protein, 6 aa, Homo sapiens
QMGPRG

SEQ ID NO: 161 - protein, 6 aa, Homo sapiens
PGPPGA

SEQ ID NO: 162 - protein, 6 aa, Homo sapiens
QGIAGQ

SEQ ID NO: 163 - protein, 6 aa, Homo sapiens
PGADGQ

SEQ ID NO: 164 - protein, 6 aa, Homo sapiens
AGSPGF

SEQ ID NO: 165 - protein, 6 aa, Homo sapiens
LPGPSG

SEQ ID NO: 166 - protein, 6 aa, Homo sapiens
PPGPKG

SEQ ID NO: 167 - protein, 6 aa, Homo sapiens
PGERGA

SEQ ID NO: 168 - protein, 6 aa, Homo sapiens
IKGPAG

SEQ ID NO: 169 - protein, 6 aa, Homo sapiens
PKGPAG

SEQ ID NO: 170 - protein, 6 aa, Homo sapiens
GRNGDP

SEQ ID NO: 171 - protein, 6 aa, Homo sapiens
SPGEQG

SEQ ID NO: 172 - protein, 6 aa, Homo sapiens
GPAGRP

SEQ ID NO: 173 - protein, 6 aa, Homo sapiens
  MOD_RES 2: note = proline or hydroxyproline
PXGPIG

SEQ ID NO: 174 - protein, 6 aa, Homo sapiens
TGDAGP

SEQ ID NO: 175 - protein, 6 aa, Homo sapiens
LSGERG

SEQ ID NO: 176 - protein, 6 aa, Homo sapiens
TGPRGP

SEQ ID NO: 177 - protein, 20 aa, Homo sapiens
AGIPGAPGLMGARGPPGPAG

SEQ ID NO: 178 - protein, 19 aa, Homo sapiens
KGDPGPPGIPGRNGDPGIP

SEQ ID NO: 179 - protein, 20 aa, Homo sapiens
GLAGPPGMPGPRGSPGPQGV

SEQ ID NO: 180 - protein, 21 aa, Homo sapiens
GERGLPGPPGIKGPAGIPGFP

SEQ ID NO: 181 - protein, 22 aa, Homo sapiens
GIAGITGARGLAGPPGMPGPRG

SEQ ID NO: 182 - protein, 23 aa, Homo sapiens
GIKGHRGFPGNPGAPGSPGPAGQ

SEQ ID NO: 183 - protein, 23 aa, Homo sapiens
ARGLAGPPGMPGPRGSPGPQGVK

SEQ ID NO: 184 - protein, 25 aa, Homo sapiens
ITGARGLAGPPGMPGPRGSPGPQGV

SEQ ID NO: 185 - protein, 26 aa, Homo sapiens
ITGARGLAGPPGMPGPRGSPGPQGVK

SEQ ID NO: 186 - protein, 26 aa, Homo sapiens
GITGARGLAGPPGMPGPRGSPGPQGV

SEQ ID NO: 187 - protein, 26 aa, Homo sapiens
GVKGESGKPGANGLSGERGPPGPQGL

SEQ ID NO: 188 - protein, 26 aa, Homo sapiens
GSRGAPGPQGPRGDKGETGERGAAGI

SEQ ID NO: 189 - protein, 28 aa, Homo sapiens
PKGDAGQPGEKGSPGAQGPPGAPGPLGI

SEQ ID NO: 190 - protein, 27 aa, Homo sapiens
GITGARGLAGPPGMPGPRGSPGPQGVK

SEQ ID NO: 191 - protein, 32 aa, Homo sapiens
GLRGGAGPPGPEGGKGAAGPPGPPGAAGTPGL

SEQ ID NO: 192 - protein, 35 aa, Homo sapiens
GHAGAQGPPGPPGINGSPGGKGEMGPAGIPGAPGL

SEQ ID NO: 193 - protein, 48 aa, Homo sapiens
AGKSGDRGESGPAGPAGAPGPAGSRGAPGPQGPRGDKGETGERGAAGI

SEQ ID NO: 194 - protein, 50 aa, Homo sapiens
GLQGLPGTGGPPGENGKPGEPGPKGDAGAPGAPGGKGDAGAPGERGPPGL

SEQ ID NO: 195 - protein, 21 aa, Homo sapiens
GERGLPGPPGIKGPAGIPGFP

SEQ ID NO: 196 - protein, 24 aa, Homo sapiens
AVGGLAGYPGPAGPPGPPGPPGTS

SEQ ID NO: 197 - protein, 24 aa, Homo sapiens
KDGTSGHPGPIGPPGPRGNRGERG

SEQ ID NO: 198 - protein, 29 aa, Homo sapiens
AVGGLAGYPGPAGPPGPPGPPGTSGHPGS

SEQ ID NO: 199 - protein, 29 aa, Homo sapiens
GIAGITGARGLAGPPGMPGPRGSPGPQGV

SEQ ID NO: 200 - protein, 31 aa, Homo sapiens
APGAPGGKGDAGAPGERGPPGLAGAPGLRGG

SEQ ID NO: 201 - protein, 32 aa, Homo sapiens
AVGGLAGYPGPAGPPGPPGPPGTSGHPGSPGS

SEQ ID NO: 202 - protein, 22 aa, Homo sapiens
AIGSPGPAGPRGPVGPSGPPGK

SEQ ID NO: 203 - protein, 23 aa, Homo sapiens
GAIGSPGPAGPRGPVGPSGPPGK

SEQ ID NO: 204 - protein, 15 aa, Homo sapiens
PAGQQGAIGSPGPAG

SEQ ID NO: 205 - protein, 20 aa, Homo sapiens
GGPPGVAGPPGGSGPAGPPG

SEQ ID NO: 206 - protein, 19 aa, Homo sapiens
LAGPPGMPGPRGSPGPQGV

SEQ ID NO: 207 - protein, 19 aa, Homo sapiens
GLSGERGPPGPQGLPGLAG

SEQ ID NO: 208 - protein, 21 aa, Homo sapiens
RGLAGPPGMPGPRGSPGPQGV

SEQ ID NO: 209 - protein, 21 aa, Homo sapiens
GLAGPPGMPGPRGSPGPQGVK

SEQ ID NO: 210 - protein, 22 aa, Homo sapiens
RGLAGPPGMPGPRGSPGPQGVK

SEQ ID NO: 211 - protein, 21 aa, Homo sapiens
GPQGPPGKNGETGPQGPPGPT

SEQ ID NO: 212 - protein, 22 aa, Homo sapiens
GVKGERGSPGGPGAAGFPGARG

SEQ ID NO: 213 - protein, 22 aa, Homo sapiens
ARGLAGPPGMPGPRGSPGPQGV

SEQ ID NO: 214 - protein, 23 aa, Homo sapiens
NGLSGERGPPGPQGLPGLAGTAG

SEQ ID NO: 215 - protein, 24 aa, Homo sapiens
AVGGLAGYPGPAGPPGPPGPPGTS

SEQ ID NO: 216 - protein, 24 aa, Homo sapiens
GSPGGKGEMGPAGIPGAPGLMGAR

SEQ ID NO: 217 - protein, 24 aa, Homo sapiens
TGARGLAGPPGMPGPRGSPGPQGV

SEQ ID NO: 218 - protein, 25 aa, Homo sapiens
VKGESGKPGANGLSGERGPPGPQGL

SEQ ID NO: 219 - protein, 53 aa, Homo sapiens
GVKGERGSPGGPGAAGFPGARGLPGPPGSNGNPGPPGPSGSPGKDGPPGPAGN

SEQ ID NO: 220 - protein, 32 aa, Homo sapiens
GSPGAQGPPGAPGPLGIAGITGARGLAGPPGM

SEQ ID NO: 221 - protein, 32 aa, Homo sapiens
RGAPGEKGEGGPPGVAGPPGGSGPAGPPGPQG

SEQ ID NO: 222 - protein, 32 aa, Homo sapiens; identical to SEQ ID NO: 221

SEQ ID NO: 223 - protein, 29 aa, Homo sapiens
GIAGITGARGLAGPPGMPGPRGSPGPQGV

SEQ ID NO: 224 - protein, 14 aa, Homo sapiens
GIKGPAGIPGFPGM

SEQ ID NO: 225 - protein, 14 aa, Homo sapiens
GQPGVMGFPGPKGN

SEQ ID NO: 226 - protein, 16 aa, Homo sapiens
GIKGPAGIPGFPGMKG

SEQ ID NO: 227 - protein, 17 aa, Homo sapiens
GIKGPAGIPGFPGMKGH

SEQ ID NO: 228 - protein, 19 aa, Homo sapiens
IPGAPGLMGARGPPGPAGA

SEQ ID NO: 229 - protein, 19 aa, Homo sapiens
GERGLPGPPGIKGPAGIPG

SEQ ID NO: 230 - protein, 20 aa, Homo sapiens
GIPGAPGLMGARGPPGPAGA

SEQ ID NO: 231 - protein, 20 aa, Homo sapiens
GFRGPAGPNGIPGEKGPAGE

SEQ ID NO: 232 - protein, 20 aa, Homo sapiens
PGIPGQPGSPGSPGPPGICE

SEQ ID NO: 233 - protein, 21 aa, Homo sapiens
GERGLPGPPGIKGPAGIPGFP

SEQ ID NO: 234 - protein, 23 aa, Homo sapiens
AVGGLAGYPGPAGPPGPPGPPGT

SEQ ID NO: 235 - protein, 23 aa, Homo sapiens
GVKGERGSPGGPGAAGFPGARGL

SEQ ID NO: 236 - protein, 26 aa, Homo sapiens
GDAGAPGAPGGKGDAGAPGERGPPGL

SEQ ID NO: 237 - protein, 25 aa, Homo sapiens
QGPPGPTGPGGDKGDTGPPGPQGLQ

SEQ ID NO: 238 - protein, 25 aa, Homo sapiens
GINGSPGGKGEMGPAGIPGAPGLMG

SEQ ID NO: 239 - protein, 26 aa, Homo sapiens
QGPPGEPGQAGPSGPPGPPGAIGPSG

SEQ ID NO: 240 - protein, 26 aa, Homo sapiens
PGPPGINGSPGGKGEMGPAGIPGAPG

SEQ ID NO: 241 - protein, 33 aa, Homo sapiens
RGLPGPPGSNGNPGPPGPSGSPGKDGPPGPAGN

SEQ ID NO: 242 - protein, 32 aa, Homo sapiens
GKNGETGPQGPPGPTGPGGDKGDTGPPGPQGL

SEQ ID NO: 243 - protein, 32 aa, Homo sapiens
GLPGIAGPRGSPGERGETGPPGPAGFPGAPGQ

SEQ ID NO: 244 - protein, 35 aa, Homo sapiens
GINGSPGGKGEMGPAGIPGAPGLMGARGPPGPAGA

SEQ ID NO: 245 - protein, 36 aa, Homo sapiens
PGINGSPGGKGEMGPAGIPGAPGLMGARGPPGPAGA

SEQ ID NO: 246 - protein, 40 aa, Homo sapiens
PPGENGKPGEPGPKGDAGAPGAPGGKGDAGAPGERGPPGL

SEQ ID NO: 247 - protein, 38 aa, Homo sapiens
GLKGENGLPGENGAPGPMGPRGAPGERGRPGLPGAAGA

SEQ ID NO: 248 - protein, 41 aa, Homo sapiens
GNTGAPGSPGVSGPKGDAGQPGEKGSPGAQGPPGAPGPLGI

SEQ ID NO: 249 - protein, 41 aa, Homo sapiens
GLMGARGPPGPAGANGAPGLRGGAGEPGKNGAKGEPGPRGE

SEQ ID NO: 250 - protein, 50 aa, Homo sapiens
GLRGGAGPPGPEGGKGAAGPPGPPGAAGTPGLQGMPGERGGLGSPGPKGD

SEQ ID NO: 251 - protein, 26 aa, Homo sapiens
GQQGAIGSPGPAGPRGPVGPSGPPGK

SEQ ID NO: 252 - protein, 24 aa, Homo sapiens
KGDPGPPGIPGRNGDPGIPGQPGS

SEQ ID NO: 253 - protein, 26 aa, Homo sapiens
GLRGGAGPPGPEGGKGAAGPPGPPGA

SEQ ID NO: 254 - protein, 32 aa, Homo sapiens; identical to SEQ ID NO: 242

SEQ ID NO: 255 - protein, 23 aa, Homo sapiens
GYQGPPGEPGQAGPSGPPGPPGA

SEQ ID NO: 256 - protein, 20 aa, Homo sapiens
GVAGPPGGSGPAGPPGPQGV

SEQ ID NO: 257 - protein, 35 aa, Homo sapiens
GDKGEPGGPGADGVPGKDGPRGPTGPIGPPGPAGQ

SEQ ID NO: 258 - protein, 17 aa, Homo sapiens
QGHAGAQGPPGPPGING

SEQ ID NO: 259 - protein, 11 aa, Homo sapiens
AGERGAPGPAG

SEQ ID NO: 260 - protein, 11 aa, Homo sapiens
AGIPGFPGMKG

SEQ ID NO: 261 - protein, 12 aa, Homo sapiens
FPGMKGHRGFDG

SEQ ID NO: 262 - protein, 14 aa, Homo sapiens
GFPGARGLPGPPGS

SEQ ID NO: 263 - protein, 15 aa, Homo sapiens
AGFPGARGLPGPPGS

SEQ ID NO: 264 - protein, 15 aa, Homo sapiens
PPGPPGPPGTSGHPG

SEQ ID NO: 265 - protein, 13 aa, Homo sapiens
GFPGMKGHRGFDG

SEQ ID NO: 266 - protein, 17 aa, Homo sapiens
QPGDKGEGGAPGLPGIA

SEQ ID NO: 267 - protein, 17 aa, Homo sapiens
RGDKGETGERGAAGIKG

SEQ ID NO: 268 - protein, 17 aa, Homo sapiens
DGRNGEKGETGAPGLKG

SEQ ID NO: 269 - protein, 20 aa, Homo sapiens
AGQPGDKGEGGAPGLPGIAG

SEQ ID NO: 270 - protein, 19 aa, Homo sapiens
GGPPGENGKPGEPGPKGDA

SEQ ID NO: 271 - protein, 17 aa, Homo sapiens
AGIPGFPGMKGHRGFDG

SEQ ID NO: 272 - protein, 20 aa, Homo sapiens
RGGAGEPGKNGAKGEPGPRG

SEQ ID NO: 273 - protein, 26 aa, Homo sapiens
KGERGSPGGPGAAGFPGARGLPGPPG

SEQ ID NO: 274 - protein, 27 aa, Homo sapiens
IPGVPGAKGEDGKDGSPGEPGANGLPG

SEQ ID NO: 275 - protein, 28 aa, Homo sapiens
GAAGFPGARGLPGPPGSNGNPGPPGPSG

SEQ ID NO: 276 - protein, 26 aa, Homo sapiens
RPGPPGPSGPRGQPGVMGFPGPKGND

SEQ ID NO: 277 - protein, 29 aa, Homo sapiens
QGPPGPPGINGSPGGKGEMGPAGIPGAPG

SEQ ID NO: 278 - protein, 26 aa, Homo sapiens
AGKDGESGRPGRPGERGLPGPPGIKG

SEQ ID NO: 279 - protein, 30 aa, Homo sapiens
AGARGNDGARGSDGQPGPPGPPGTAGFPGS

SEQ ID NO: 280 - protein, 31 aa, Homo sapiens
SPGVSGPKGDAGQPGEKGSPGAQGPPGAPGP

SEQ ID NO: 281 - protein, 32 aa, Homo sapiens
RGSDGQPGPPGPPGTAGFPGSPGAKGEVGPAG

SEQ ID NO: 282 - protein, 32 aa, Homo sapiens
QGPPGPPGINGSPGGKGEMGPAGIPGAPGLMG

SEQ ID NO: 283 - protein, 33 aa, Homo sapiens
AGPPGPPGPPGTSGHPGSPGSPGYQGPPGEPGQ

SEQ ID NO: 284 - protein, 33 aa, Homo sapiens
FPGAPGQNGEPGGKGERGAPGEKGEGGPPGVAG

SEQ ID NO: 285 - protein, 33 aa, Homo sapiens
AGFPGAPGQNGEPGGKGERGAPGEKGEGGPPGV

SEQ ID NO: 286 - protein, 41 aa, Homo sapiens
AGARGNDGARGSDGQPGPPGPPGTAGFPGSPGAKGEVGPAG

SEQ ID NO: 287 - protein, 53 aa, Homo sapiens
RGAAGEPGRDGVPGGPGMRGMPGSPGGPGSDGKPGPPGSQGESGRPGPPGPSG

SEQ ID NO: 288 - protein, 12 aa, Homo sapiens
GIAGITGARGLA

SEQ ID NO: 289 - protein, 18 aa, Homo sapiens
AGPPGPPGAAGTPGLQGM

SEQ ID NO: 290 - protein, 18 aa, Homo sapiens
NGLSGERGPPGPQGLPGL

SEQ ID NO: 291 - protein, 20 aa, Homo sapiens
MGARGPPGPAGANGAPGLRG

SEQ ID NO: 292 - protein, 20 aa, Homo sapiens
NGLSGERGPPGPQGLPGLAG

SEQ ID NO: 293 - protein, 23 aa, Homo sapiens
GIAGITGARGLAGPPGMPGPRGS

SEQ ID NO: 294 - protein, 29 aa, Homo sapiens
GIAGITGARGLAGPPGMPGPRGSPGPQGV

SEQ ID NO: 295 - protein, 32 aa, Homo sapiens
RGGAGPPGPEGGKGAAGPPGPPGAAGTPGLQG

SEQ ID NO: 296 - protein, 30 aa, Homo sapiens
SGPKGDAGQPGEKGSPGAQGPPGAPGPLGI

SEQ ID NO: 297 - protein, 31 aa, Homo sapiens
GIAGITGARGLAGPPGMPGPRGSPGPQGVKG

SEQ ID NO: 298 - protein, 30 aa, Homo sapiens; identical to SEQ ID NO: 296

SEQ ID NO: 299 - protein, 31 aa, Homo sapiens; identical to SEQ ID NO: 297

SEQ ID NO: 300 - protein, 37 aa, Homo sapiens
AVGGLAGYPGPAGPPGPPGPPGTSGHPGSPGSPGYQG

SEQ ID NO: 301 - protein, 40 aa, Homo sapiens
EPGPQGHAGAQGPPGPPGINGSPGGKGEMGPAGIPGAPGL

SEQ ID NO: 302 - protein, 12 aa, Homo sapiens
IPGFPGMKGHRG

SEQ ID NO: 303 - protein, 17 aa, Homo sapiens
RGSPGGPGAAGFPGARG

SEQ ID NO: 304 - protein, 17 aa, Homo sapiens
KGPAGIPGFPGMKGHRG

SEQ ID NO: 305 - protein, 20 aa, Homo sapiens
RGLAGPPGMPGPRGSPGPQG

SEQ ID NO: 306 - protein, 20 aa, Homo sapiens
AGITGARGLAGPPGMPGPRG

SEQ ID NO: 307 - protein, 23 aa, Homo sapiens
LGIAGITGARGLAGPPGMPGPRG

SEQ ID NO: 308 - protein, 23 aa, Homo sapiens
TGARGLAGPPGMPGPRGSPGPQG

SEQ ID NO: 309 - protein, 24 aa, Homo sapiens
QGPPGPPGINGSPGGKGEMGPAGI

SEQ ID NO: 310 - protein, 24 aa, Homo sapiens
LPGPPGIKGPAGIPGFPGMKGHRG

SEQ ID NO: 311 - protein, 26 aa, Homo sapiens
AGITGARGLAGPPGMPGPRGSPGPQG

SEQ ID NO: 312 - protein, 26 aa, Homo sapiens
TGARGLAGPPGMPGPRGSPGPQGVKG

SEQ ID NO: 313 - protein, 26 aa, Homo sapiens
RGLPGPPGIKGPAGIPGFPGMKGHRG

SEQ ID NO: 314 - protein, 29 aa, Homo sapiens
GRPGLPGAAGARGNDGARGSDGQPGPPGP

SEQ ID NO: 315 - protein, 29 aa, Homo sapiens
NGAPGPMGPRGAPGERGRPGLPGAAGARG

SEQ ID NO: 316 - protein, 29 aa, Homo sapiens
AGSRGAPGPQGPRGDKGETGERGAAGIKG

SEQ ID NO: 317 - protein, 32 aa, Homo sapiens
RGLAGPPGMPGPRGSPGPQGVKGESGKPGANG

SEQ ID NO: 318 - protein, 34 aa, Homo sapiens
RGLAGPPGMPGPRGSPGPQGVKGESGKPGANGLS

SEQ ID NO: 319 - protein, 37 aa, Homo sapiens
PGPPGSNGNPGPPGPSGSPGKDGPPGPAGNTGAPGSP

SEQ ID NO: 320 - protein, 35 aa, Homo sapiens
TGARGLAGPPGMPGPRGSPGPQGVKGESGKPGANG

SEQ ID NO: 321 - protein, 38 aa, Homo sapiens
RGAPGEKGEGGPPGVAGPPGGSGPAGPPGPQGVKGERG

SEQ ID NO: 322 - protein, 40 aa, Homo sapiens
GGPPGVAGPPGGSGPAGPPGPQGVKGERGSPGGPGAAGFP

SEQ ID NO: 323 - protein, 48 aa, Homo sapiens
KSGDRGESGPAGPAGAPGPAGSRGAPGPQGPRGDKGETGERGAAGIKG

SEQ ID NO: 324 - protein, 12 aa, Homo sapiens
IPGFPGMKGHRG

SEQ ID NO: 325 - protein, 14 aa, Homo sapiens
RGLAGPPGMPGPRG

SEQ ID NO: 326 - protein, 16 aa, Homo sapiens
GPQGLQGLPGTGGPPG

SEQ ID NO: 327 - protein, 17 aa, Homo sapiens
KGPAGIPGFPGMKGHRG

SEQ ID NO: 328 - protein, 21 aa, Homo sapiens
RGLAGPPGMPGPRGSPGPQGV

SEQ ID NO: 329 - protein, 23 aa, Homo sapiens
GGPPGENGKPGEPGPKGDAGAPG

SEQ ID NO: 330 - protein, 24 aa, Homo sapiens
APGFRGPAGPNGIPGEKGPAGERG

SEQ ID NO: 331 - protein, 27 aa, Homo sapiens
EKGSPGAQGPPGAPGPLGIAGITGARG

SEQ ID NO: 332 - protein, 24 aa, Homo sapiens
LPGPPGIKGPAGIPGFPGMKGHRG

SEQ ID NO: 333 - protein, 26 aa, Homo sapiens
RGAPGFRGPAGPNGIPGEKGPAGERG

SEQ ID NO: 334 - protein, 26 aa, Homo sapiens
RGLPGPPGIKGPAGIPGFPGMKGHRG

SEQ ID NO: 335 - protein, 29 aa, Homo sapiens
RGPVGPSGPPGKDGTSGHPGPIGPPGPRG

SEQ ID NO: 336 - protein, 27 aa, Homo sapiens
APGPQGPRGDKGETGERGAAGIKGHRG

SEQ ID NO: 337 - protein, 29 aa, Homo sapiens
RGAPGPQGPRGDKGETGERGAAGIKGHRG

SEQ ID NO: 338 - protein, 32 aa, Homo sapiens
RGFPGNPGAPGSPGPAGQQGAIGSPGPAGPRG

SEQ ID NO: 339 - protein, 29 aa, Homo sapiens
LPGPPGIKGPAGIPGFPGMKGHRGFDGRN

SEQ ID NO: 340 - protein, 33 aa, Homo sapiens
DAGQPGEKGSPGAQGPPGAPGPLGIAGITGARG

SEQ ID NO: 341 - protein, 35 aa, Homo sapiens
RGPTGPIGPPGPAGQPGDKGEGGAPGLPGIAGPRG

SEQ ID NO: 342 - protein, 35 aa, Homo sapiens
KGDAGQPGEKGSPGAQGPPGAPGPLGIAGITGARG

SEQ ID NO: 343 - protein, 33 aa, Homo sapiens
RNGEKGETGAPGLKGENGLPGENGAPGPMGPRG

SEQ ID NO: 344 - protein, 35 aa, Homo sapiens
APGFRGPAGPNGIPGEKGPAGERGAPGPAGPRGAA

SEQ ID NO: 345 - protein, 35 aa, Homo sapiens
RGAPGFRGPAGPNGIPGEKGPAGERGAPGPAGPRG

SEQ ID NO: 346 - protein, 35 aa, Homo sapiens
RGSPGERGETGPPGPAGFPGAPGQNGEPGGKGERG

SEQ ID NO: 347 - protein, 38 aa, Homo sapiens
GHAGAQGPPGPPGINGSPGGKGEMGPAGIPGAPGLMGA

SEQ ID NO: 348 - protein, 38 aa, Homo sapiens
RGLAGPPGMPGPRGSPGPQGVKGESGKPGANGLSGERG

SEQ ID NO: 349 - protein, 13 aa, Homo sapiens
LGIAGITGARGLA

SEQ ID NO: 350 - protein, 12 aa, Homo sapiens
IPGFPGMKGHRG

SEQ ID NO: 351 - protein, 14 aa, Homo sapiens
RGLAGPPGMPGPRG

SEQ ID NO: 352 - protein, 20 aa, Homo sapiens
QGPPGAPGPLGIAGITGARG

SEQ ID NO: 353 - protein, 20 aa, Homo sapiens
AGITGARGLAGPPGMPGPRG

SEQ ID NO: 354 - protein, 23 aa, Homo sapiens
AGIPGAPGLMGARGPPGPAGANG

SEQ ID NO: 355 - protein, 24 aa, Homo sapiens
RGLAGPPGMPGPRGSPGPQGVKGE

SEQ ID NO: 356 - protein, 26 aa, Homo sapiens
KGSPGAQGPPGAPGPLGIAGITGARG

SEQ ID NO: 357 - protein, 24 aa, Homo sapiens
LPGPPGIKGPAGIPGFPGMKGHRG

SEQ ID NO: 358 - protein, 24 aa, Homo sapiens
KDGTSGHPGPIGPPGPRGNRGERG

SEQ ID NO: 359 - protein, 26 aa, Homo sapiens
AGITGARGLAGPPGMPGPRGSPGPQG

SEQ ID NO: 360 - protein, 27 aa, Homo sapiens
RGLAGPPGMPGPRGSPGPQGVKGESGK

SEQ ID NO: 361 - protein, 32 aa, Homo sapiens; identical to SEQ ID NO: 317

SEQ ID NO: 362 - protein, 34 aa, Homo sapiens; identical to SEQ ID NO: 318

SEQ ID NO: 363 - protein, 37 aa, Homo sapiens; identical to SEQ ID NO: 319

SEQ ID NO: 364 - protein, 38 aa, Homo sapiens; identical to SEQ ID NO: 321

SEQ ID NO: 365 - protein, 44 aa, Homo sapiens
KSGDRGESGPAGPAGAPGPAGSRGAPGPQGPRGDKGETGERGAA

SEQ ID NO: 366 - protein, 53 aa, Homo sapiens
RGAPGEKGEGGPPGVAGPPGGSGPAGPPGPQGVKGERGSPGGPGAAGFPGARG

SEQ ID NO: 367 - protein, 6 aa, Homo sapiens
AIGPSG

SEQ ID NO: 368 - protein, 10 aa, Homo sapiens
PGIPGRNGDP

SEQ ID NO: 369 - protein, 10 aa, Homo sapiens
ESCPTGPQNY

SEQ ID NO: 370 - protein, 10 aa, Homo sapiens
PKGDTGPRGP

SEQ ID NO: 371 - protein, 6 aa, Homo sapiens
GIPGAP

SEQ ID NO: 372 - skipped

SEQ ID NO: 373 - protein, 6 aa, Homo sapiens
KGESGK

SEQ ID NO: 374 - protein, 6 aa, Homo sapiens
IAGITG

SEQ ID NO: 375 - protein, 6 aa, Homo sapiens
IKGHRG

SEQ ID NO: 376 - protein, 6 aa, Homo sapiens
RGLAGP

SEQ ID NO: 377 - protein, 6 aa, Homo sapiens
TGARGL

SEQ ID NO: 378 - protein, 6 aa, Homo sapiens
ITGARG

SEQ ID NO: 379 - protein, 6 aa, Homo sapiens
VKGESG

SEQ ID NO: 380 - protein, 6 aa, Homo sapiens
KGDAGQ

SEQ ID NO: 381 - protein, 6 aa, Homo sapiens
LRGGAG

SEQ ID NO: 382 - protein, 6 aa, Homo sapiens
GKSGDR

SEQ ID NO: 383 - protein, 6 aa, Homo sapiens
LQGLPG

SEQ ID NO: 384 - protein, 6 aa, Homo sapiens
ERGLPG

SEQ ID NO: 385 - protein, 6 aa, Homo sapiens
IGSPGP

SEQ ID NO: 386 - protein, 6 aa, Homo sapiens
GAPGEK

SEQ ID NO: 387 - protein, 6 aa, Homo sapiens
GLSGER

SEQ ID NO: 388 - protein, 6 aa, Homo sapiens
GLAGPP

SEQ ID NO: 389 - protein, 6 aa, Homo sapiens
PQGPPG

SEQ ID NO: 390 - protein, 6 aa, Homo sapiens
QQGAIG

SEQ ID NO: 391 - protein, 6 aa, Homo sapiens
GPPGPT

SEQ ID NO: 392 - protein, 6 aa, Homo sapiens
INGSPG

SEQ ID NO: 393 - protein, 6 aa, Homo sapiens
GPPGEP

SEQ ID NO: 394 - protein, 6 aa, Homo sapiens
GLPGPP

SEQ ID NO: 395 - protein, 6 aa, Homo sapiens
KNGETG

SEQ ID NO: 396 - protein, 6 aa, Homo sapiens
LPGIAG

SEQ ID NO: 397 - protein, 6 aa, Homo sapiens
GINGSP

SEQ ID NO: 398 - protein, 6 aa, Homo sapiens
GINGSP

SEQ ID NO: 399 - protein, 6 aa, Homo sapiens
LKGENG

SEQ ID NO: 400 - protein, 6 aa, Homo sapiens
LMGARG

SEQ ID NO: 401 - protein, 6 aa, Homo sapiens
YQGPPG

SEQ ID NO: 402 - protein, 6 aa, Homo sapiens
GERGAP

SEQ ID NO: 403 - protein, 6 aa, Homo sapiens
DKGEPG

SEQ ID NO: 404 - protein, 6 aa, Homo sapiens
GHAGAQ

SEQ ID NO: 405 - protein, 6 aa, Homo sapiens
GSDGQP

SEQ ID NO: 406 - protein, 6 aa, Homo sapiens
PGMKGH

SEQ ID NO: 407 - protein, 6 aa, Homo sapiens
FPGARG

SEQ ID NO: 408 - protein, 6 aa, Homo sapiens
GFPGAR

SEQ ID NO: 409 - protein, 6 aa, Homo sapiens
FPGMKG

SEQ ID NO: 410 - protein, 6 aa, Homo sapiens
PGDKGE

SEQ ID NO: 411 - protein, 6 aa, Homo sapiens
GDKGET

SEQ ID NO: 412 - protein, 6 aa, Homo sapiens
GQPGDK

SEQ ID NO: 413 - protein, 6 aa, Homo sapiens
GPPGEN

SEQ ID NO: 414 - protein, 6 aa, Homo sapiens
GIPGFP

SEQ ID NO: 415 - protein, 6 aa, Homo sapiens
GERGSP

SEQ ID NO: 416 - protein, 6 aa, Homo sapiens
PGVPGA

SEQ ID NO: 417 - protein, 6 aa, Homo sapiens
AAGFPG

SEQ ID NO: 418 - protein, 6 aa, Homo sapiens
GKDGES

SEQ ID NO: 419 - protein, 6 aa, Homo sapiens
GARGND

SEQ ID NO: 420 - protein, 6 aa, Homo sapiens
GFPGAP

SEQ ID NO: 421 - protein, 6 aa, Homo sapiens
GAAGEP

SEQ ID NO: 422 - protein, 6 aa, Homo sapiens
GARGPP

SEQ ID NO: 423 - protein, 6 aa, Homo sapiens
GPPGSN

SEQ ID NO: 424 - protein, 6 aa, Homo sapiens
GPKGDA

SEQ ID NO: 425 - protein, 6 aa, Homo sapiens
GGAGPP

SEQ ID NO: 426 - protein, 6 aa, Homo sapiens
PGPQGH

SEQ ID NO: 427 - protein, 6 aa, Homo sapiens
PGFPGM

SEQ ID NO: 428 - protein, 6 aa, Homo sapiens
GSPGGP

SEQ ID NO: 429 - protein, 6 aa, Homo sapiens
SGDRGE

SEQ ID NO: 430 - protein, 6 aa, Homo sapiens
GITGAR

SEQ ID NO: 431 - protein, 6 aa, Homo sapiens
GIAGIT

SEQ ID NO: 432 - protein, 6 aa, Homo sapiens
PGPPGI

SEQ ID NO: 433 - protein, 6 aa, Homo sapiens
ESCPTG

SEQ ID NO: 434 - protein, 6 aa, Homo sapiens
HAGAQG

SEQ ID NO: 435 - protein, 6 aa, Homo sapiens
GAPGFR

SEQ ID NO: 436 - protein, 6 aa, Homo sapiens
RPGLPG

SEQ ID NO: 437 - protein, 6 aa, Homo sapiens
NTGAPG

SEQ ID NO: 438 - protein, 6 aa, Homo sapiens
GAPGPM

SEQ ID NO: 439 - protein, 6 aa, Homo sapiens
GSPGER

SEQ ID NO: 440 - protein, 6 aa, Homo sapiens
PQGLQG

SEQ ID NO: 441 - protein, 6 aa, Homo sapiens
GPAGIP

SEQ ID NO: 442 - protein, 6 aa, Homo sapiens
DRGPQG

SEQ ID NO: 443 - protein, 6 aa, Homo sapiens
PGFRGP

SEQ ID NO: 444 - protein, 6 aa, Homo sapiens
KGSPGA

SEQ ID NO: 445 - protein, 6 aa, Homo sapiens
GAPGPQ

SEQ ID NO: 446 - protein, 6 aa, Homo sapiens
GFPGNP

SEQ ID NO: 447 - protein, 6 aa, Homo sapiens
GPVGPS

SEQ ID NO: 448 - protein, 6 aa, Homo sapiens
GPTGPI

SEQ ID NO: 449 - protein, 6 aa, Homo sapiens
GDAGQP

SEQ ID NO: 450 - protein, 6 aa, Homo sapiens
NGEKGE

SEQ ID NO: 451 - protein, 6 aa, Homo sapiens
SRGAPG

SEQ ID NO: 452 - protein, 6 aa, Homo sapiens
VAGPPG

SEQ ID NO: 453 - protein, 6 aa, Homo sapiens
PGPQGP

SEQ ID NO: 454 - protein, 6 aa, Homo sapiens
AGQPGE

SEQ ID NO: 455 - protein, 6 aa, Homo sapiens
PGAPGG

SEQ ID NO: 456 - protein, 6 aa, Homo sapiens
PGAPGQ

SEQ ID NO: 457 - protein, 6 aa, Homo sapiens
AGQQGA

SEQ ID NO: 458 - skipped

SEQ ID NO: 459 - protein, 6 aa, Homo sapiens
SPGGKG

SEQ ID NO: 460 - protein, 6 aa, Homo sapiens
GRNGEK

SEQ ID NO: 461 - protein, 6 aa, Homo sapiens
GPPGAP

SEQ ID NO: 462 - protein, 6 aa, Homo sapiens
GSRGAP

SEQ ID NO: 463 - protein, 6 aa, Homo sapiens
GGAGEP

SEQ ID NO: 464 - protein, 6 aa, Homo sapiens
GSPGAQ

SEQ ID NO: 465 - protein, 6 aa, Homo sapiens
SPGAQG

SEQ ID NO: 466 - protein, 6 aa, Homo sapiens
PGVSGP

SEQ ID NO: 467 - protein, 6 aa, Homo sapiens
PGAPGL

SEQ ID NO: 468 - protein, 6 aa, Homo sapiens
GIPGQP

SEQ ID NO: 469 - protein, 6 aa, Homo sapiens
DAGAPG

SEQ ID NO: 470 - protein, 6 aa, Homo sapiens
GPPGIN

SEQ ID NO: 471 - protein, 6 aa, Homo sapiens
NGDPGI

SEQ ID NO: 472 - protein, 6 aa, Homo sapiens
SPGPQG

SEQ ID NO: 473 - protein, 6 aa, Homo sapiens
GMPGPR

SEQ ID NO: 474 - protein, 6 aa, Homo sapiens
SPGPAG

SEQ ID NO: 475 - protein, 6 aa, Homo sapiens
PGPQGV

SEQ ID NO: 476 - protein, 6 aa, Homo sapiens
ERGAAG

SEQ ID NO: 477 - protein, 6 aa, Homo sapiens
PGPLGI

SEQ ID NO: 478 - protein, 6 aa, Homo sapiens
AAGTPG

SEQ ID NO: 479 - protein, 6 aa, Homo sapiens
PGPPGT

SEQ ID NO: 480 - protein, 6 aa, Homo sapiens
GNRGER

SEQ ID NO: 481 - protein, 6 aa, Homo sapiens
APGLRG

SEQ ID NO: 482 - protein, 6 aa, Homo sapiens
HPGSPG

SEQ ID NO: 483 - protein, 6 aa, Homo sapiens
PSGPPG

SEQ ID NO: 484 - protein, 6 aa, Homo sapiens
GSPGPA

SEQ ID NO: 485 - protein, 6 aa, Homo sapiens
GPAGPP

SEQ ID NO: 486 - protein, 6 aa, Homo sapiens
GLPGLA

SEQ ID NO: 487 - protein, 6 aa, Homo sapiens
QGPPGP

SEQ ID NO: 488 - protein, 6 aa, Homo sapiens
GLAGTA

SEQ ID NO: 489 - protein, 6 aa, Homo sapiens
PGLMGA

SEQ ID NO: 490 - protein, 6 aa, Homo sapiens
GPPGPQ

SEQ ID NO: 491 - protein, 6 aa, Homo sapiens
  MOD_RES 2: note = proline or hydroxyproline
  MOD_RES 4: note = proline or hydroxyproline
FXGXKG

SEQ ID NO: 492 - protein, 6 aa, Homo sapiens
IPGFPG

SEQ ID NO: 493 - protein, 6 aa, Homo sapiens
GFPGMK

SEQ ID NO: 494 - protein, 6 aa, Homo sapiens
FPGAPG

SEQ ID NO: 495 - protein, 6 aa, Homo sapiens
GAIGPS

SEQ ID NO: 496 - protein, 6 aa, Homo sapiens
AGIPGF

SEQ ID NO: 497 - protein, 6 aa, Homo sapiens
PGPQGL

SEQ ID NO: 498 - protein, 6 aa, Homo sapiens
GAPGLM

SEQ ID NO: 499 - protein, 6 aa, Homo sapiens
SPGPKG

SEQ ID NO: 500 - protein, 6 aa, Homo sapiens
GEPGPR

SEQ ID NO: 501 - protein, 6 aa, Homo sapiens
IPGQPG

SEQ ID NO: 502 - protein, 6 aa, Homo sapiens
TGAPGS

SEQ ID NO: 503 - protein, 6 aa, Homo sapiens
GHRGFD

SEQ ID NO: 504 - protein, 6 aa, Homo sapiens
PGLPGI

SEQ ID NO: 505 - protein, 6 aa, Homo sapiens
GAAGIK

SEQ ID NO: 506 - protein, 6 aa, Homo sapiens
PGPKGD

SEQ ID NO: 507 - protein, 6 aa, Homo sapiens
GLPGIA

SEQ ID NO: 508 - protein, 6 aa, Homo sapiens
PQGLPG

SEQ ID NO: 509 - protein, 6 aa, Homo sapiens
GAPGLR

SEQ ID NO: 510 - protein, 6 aa, Homo sapiens
GANGLP

SEQ ID NO: 511 - protein, 6 aa, Homo sapiens
GPPGPS

SEQ ID NO: 512 - protein, 6 aa, Homo sapiens
GPPGIK

SEQ ID NO: 513 - protein, 6 aa, Homo sapiens
TAGFPG

SEQ ID NO: 514 - protein, 6 aa, Homo sapiens
GEVGPA

SEQ ID NO: 515 - protein, 6 aa, Homo sapiens
EKGPAG

SEQ ID NO: 516 - protein, 6 aa, Homo sapiens
  MOD_RES 2: note = proline or hydroxyproline
EXGPRG

SEQ ID NO: 517 - protein, 6 aa, Homo sapiens
PPGAPG

SEQ ID NO: 518 - protein, 6 aa, Homo sapiens
TSGHPG

SEQ ID NO: 519 - protein, 6 aa, Homo sapiens
GAPGPA

SEQ ID NO: 520 - protein, 6 aa, Homo sapiens
TPGLQG

SEQ ID NO: 521 - protein, 6 aa, Homo sapiens
GTPGLQ

SEQ ID NO: 522 - protein, 6 aa, Homo sapiens
GTSGHP

SEQ ID NO: 523 - protein, 6 aa, Homo sapiens
MPGPRG

SEQ ID NO: 524 - protein, 6 aa, Homo sapiens
GPQGVK

SEQ ID NO: 525 - protein, 6 aa, Homo sapiens
GAPGLK

SEQ ID NO: 526 - protein, 6 aa, Homo sapiens
GSPGYQ

SEQ ID NO: 527 - protein, 6 aa, Homo sapiens
  MOD_RES 1: note = proline or hydroxyproline
  MOD_RES 4: note = lysine or hydroxylysine
XGPXGN

SEQ ID NO: 528 - protein, 6 aa, Homo sapiens
GAAGAR

SEQ ID NO: 529 - protein, 6 aa, Homo sapiens
PGANGL

SEQ ID NO: 530 - protein, 6 aa, Homo sapiens
GTGGPP

SEQ ID NO: 531 - protein, 6 aa, Homo sapiens
GMKGHR

SEQ ID NO: 532 - protein, 6 aa, Homo sapiens
EGGPPG

SEQ ID NO: 533 - protein, 6 aa, Homo sapiens
GSPGPQ

SEQ ID NO: 534 - protein, 6 aa, Homo sapiens
EMGPAG

SEQ ID NO: 535 - protein, 6 aa, Homo sapiens
GIAGPR

SEQ ID NO: 536 - protein, 6 aa, Homo sapiens
QPGPPG

SEQ ID NO: 537 - protein, 6 aa, Homo sapiens
GKPGAN

SEQ ID NO: 538 - protein, 6 aa, Homo sapiens
GVKGER

SEQ ID NO: 539 - protein, 6 aa, Homo sapiens
PGAAGF

SEQ ID NO: 540 - protein, 6 aa, Homo sapiens
TGERGA

SEQ ID NO: 541 - protein, 6 aa, Homo sapiens
PQGVKG

SEQ ID NO: 542 - protein, 6 aa, Homo sapiens
GDAGAP

SEQ ID NO: 543 - protein, 6 aa, Homo sapiens
GPAGER

SEQ ID NO: 544 - protein, 6 aa, Homo sapiens
GPPGPR

SEQ ID NO: 545 - protein, 6 aa, Homo sapiens
GPAGPR

SEQ ID NO: 546 - protein, 6 aa, Homo sapiens
RGFDGR

SEQ ID NO: 547 - protein, 6 aa, Homo sapiens
AGPRGA

SEQ ID NO: 548 - protein, 6 aa, Homo sapiens
GGKGER

SEQ ID NO: 549 - protein, 6 aa, Homo sapiens
APGLMG

SEQ ID NO: 550 - protein, 6 aa, Homo sapiens
GPAGAN

SEQ ID NO: 551 - protein, 12 aa, Homo sapiens
DIDGYRGPPGPQ

SEQ ID NO: 552 - protein, 15 aa, Homo sapiens
SMGPPGTPSVDHGFL

SEQ ID NO: 553 - protein, 20 aa, Homo sapiens
PDGLPGSMGPPGTPSVDHGF

SEQ ID NO: 554 - protein, 21 aa, Homo sapiens
PDGLPGSMGPPGTPSVDHGFL

SEQ ID NO: 555 - protein, 22 aa, Homo sapiens
PDGLPGSMGPPGTPSVDHGFLV

SEQ ID NO: 556 - protein, 23 aa, Homo sapiens
PSGRDGLPGPPGSPGPPGQPGYT

SEQ ID NO: 557 - protein, 25 aa, Homo sapiens
PSGRDGLPGPPGSPGPPGQPGYTNG

SEQ ID NO: 558 - protein, 26 aa, Homo sapiens
PSGRDGLPGPPGSPGPPGQPGYTNGI

SEQ ID NO: 559 - protein, 26 aa, Homo sapiens
IPGSKGEQGFMGPPGPQGQPGLPGSP

SEQ ID NO: 560 - protein, 27 aa, Homo sapiens
PRGFPGPPGPDGLPGSMGPPGTPSVDH

SEQ ID NO: 561 - protein, 16 aa, Homo sapiens
EPGPPGLPGSVGSPGV

SEQ ID NO: 562 - protein, 14 aa, Homo sapiens
IDGYRGPPGPQGPP

SEQ ID NO: 563 - protein, 19 aa, Homo sapiens
PRGFPGPPGPDGLPGSMGP

SEQ ID NO: 564 - protein, 20 aa, Homo sapiens
DGLPGSMGPPGTPSVDHGFL

SEQ ID NO: 565 - protein, 21 aa, Homo sapiens
DGLPGSMGPPGTPSVDHGFLV

SEQ ID NO: 566 - protein, 29 aa, Homo sapiens
PGLPGQQGAPGIPGFPGSKGEMGVMGTPG

SEQ ID NO: 567 - protein, 31 aa, Homo sapiens
IGIPGMPGSPGLKGSPGSVGYPGSPGLPGEK

SEQ ID NO: 568 - protein, 37 aa, Homo sapiens
PGPPGPPGEKGQMGLSFQGPKGDKGDQGVSGPPGVPG

SEQ ID NO: 569 - protein, 39 aa, Homo sapiens
PGIGPPGARGPPGGQGPPGLSGPPGIKGEKGFPGFPGLD

SEQ ID NO: 570 - protein, 15 aa, Homo sapiens
EPGLPGIPGVSGPKG

SEQ ID NO: 571 - protein, 19 aa, Homo sapiens
GEKGQKGDTGPPGPPGLVI

SEQ ID NO: 572 - protein, 38 aa, Homo sapiens
LPGIGVQGPPGPPGIPGPIGQPGLHGIPGEKGDPGPPG

SEQ ID NO: 573 - protein, 14 aa, Homo sapiens
GSPGIPGHQGEMGP

SEQ ID NO: 574 - protein, 14 aa, Homo sapiens
EPGMQGEPGPPGPP

SEQ ID NO: 575 - protein, 18 aa, Homo sapiens
GPPGRLGAPGTPGLPGPR

SEQ ID NO: 576 - protein, 14 aa, Homo sapiens
PPGPKGFPGIPGPP

SEQ ID NO: 577 - protein, 14 aa, Homo sapiens
AKGQPGLPGFPGTP

SEQ ID NO: 578 - protein, 17 aa, Homo sapiens
DRGPPGPPGIRGPPGPP

SEQ ID NO: 579 - protein, 19 aa, Homo sapiens
PGPPGEKGKPGQDGIPGPA

SEQ ID NO: 580 - protein, 26 aa, Homo sapiens
LLGSKGEKGEPGLPGIPGVSGPKGYQ

SEQ ID NO: 581 - protein, 19 aa, Homo sapiens
DGLPGSMGPPGTPSVDHGF

SEQ ID NO: 582 - protein, 22 aa, Homo sapiens
TGPLGEKGERGYPGTPGPRGEP

SEQ ID NO: 583 - protein, 43 aa, Homo sapiens
GLQGIRGEPGPPGLPGSVGSPGVPGIGPPGARGPPGGQGPPGL

SEQ ID NO: 584 - protein, 28 aa, Homo sapiens
DPGLKGDKGDVGLPGKPGSMDKVDMGSM

SEQ ID NO: 585 - protein, 17 aa, Homo sapiens
LPGPMGPPGLPGIDGVK

SEQ ID NO: 586 - protein, 28 aa, Homo sapiens
GIRGEPGPPGLPGSVGSPGVPGIGPPGA

SEQ ID NO: 587 - protein, 28 aa, Homo sapiens
GFPGPPGPDGLPGSMGPPGTPSVDHGFL

SEQ ID NO: 588 - protein, 31 aa, Homo sapiens
GLQGIRGEPGPPGLPGSVGSPGVPGIGPPGA

SEQ ID NO: 589 - protein, 40 aa, Homo sapiens
GIRGEPGPPGLPGSVGSPGVPGIGPPGARGPPGGQGPPGL

SEQ ID NO: 590 - protein, 17 aa, Homo sapiens
EDGVIGMMGFPGAIGPP

SEQ ID NO: 591 - protein, 34 aa, Homo sapiens
YPGNPGILGPPGEDGVIGMMGFPGAIGPPGPPGN

SEQ ID NO: 592 - protein, 16 aa, Homo sapiens
IPPSDEICEPGPPGPP

SEQ ID NO: 593 - protein, 26 aa, Homo sapiens
LPGLPGPKGEPGLPGYPGNPGIKGSV

SEQ ID NO: 594 - protein, 19 aa, Homo sapiens
GIKGDKGSMGHPGPKGPPG

SEQ ID NO: 595 - protein, 22 aa, Homo sapiens
TPGSPGCAGSPGLPGSPGPPGP

SEQ ID NO: 596 - protein, 46 aa, Homo sapiens
PGAPGPQGLPGPPGFPGPVGPPGPPGFFGFPGAMGPRGPKGHMGER

SEQ ID NO: 597 - protein, 11 aa, Homo sapiens
GLPGFAGNPGP

SEQ ID NO: 598 - protein, 17 aa, Homo sapiens
GAEGLPGSPGFPGPQGD

SEQ ID NO: 599 - protein, 17 aa, Homo sapiens
MGPPGVPGFQGPKGLPG

SEQ ID NO: 600 - protein, 17 aa, Homo sapiens
DIDGYRGPPGPQGPPGE

SEQ ID NO: 601 - protein, 18 aa, Homo sapiens
GDQGDQGVPGAKGLPGPP

SEQ ID NO: 602 - protein, 18 aa, Homo sapiens
GDRGPQGQPGLPGLPGPM

SEQ ID NO: 603 - protein, 27 aa, Homo sapiens
EKGSIGIPGMPGSPGLKGSPGSVGYPG

SEQ ID NO: 604 - protein, 49 aa, Homo sapiens
GLQGIRGEPGPPGLPGSVGSPGVPGIGPPGARGPPGGQGPPGLSGPPGI

SEQ ID NO: 605 - protein, 19 aa, Homo sapiens
PGPPGLMGPPGPPGLPGPK

SEQ ID NO: 606 - protein, 23 aa, Homo sapiens
GERGSPGIPGAPGPIGPPGSPGL

SEQ ID NO: 607 - protein, 44 aa, Homo sapiens
PGIPGAPGAPGFPGSKGEPGDILTFPGMKGDKGELGSPGAPGLP

SEQ ID NO: 608 - protein, 18 aa, Homo sapiens
CDGGVPNTGPPGEPGPPG

SEQ ID NO: 609 - protein, 6 aa, Homo sapiens
IDGYRG

SEQ ID NO: 610 - protein, 6 aa, Homo sapiens
MGPPGT

SEQ ID NO: 611 - protein, 6 aa, Homo sapiens
DGLPGS

SEQ ID NO: 612 - protein, 6 aa, Homo sapiens
PGSKGE

SEQ ID NO: 613 - protein, 6 aa, Homo sapiens
RGFPGP

SEQ ID NO: 614 - protein, 6 aa, Homo sapiens
PGPPGL

SEQ ID NO: 615 - protein, 6 aa, Homo sapiens
GLPGSM

SEQ ID NO: 616 - protein, 6 aa, Homo sapiens
GLPGQQ

SEQ ID NO: 617 - protein, 6 aa, Homo sapiens
LGSKGE

SEQ ID NO: 618 - protein, 6 aa, Homo sapiens
PGIGVQ

SEQ ID NO: 619 - protein, 6 aa, Homo sapiens
SPGIPG

SEQ ID NO: 620 - protein, 6 aa, Homo sapiens
PGMQGE

SEQ ID NO: 621 - protein, 6 aa, Homo sapiens
PGPKGF

SEQ ID NO: 622 - protein, 6 aa, Homo sapiens
KGQPGL

SEQ ID NO: 623 - protein, 6 aa, Homo sapiens
PPSDEI

SEQ ID NO: 624 - protein, 6 aa, Homo sapiens
PGLKGD

SEQ ID NO: 625 - protein, 6 aa, Homo sapiens
GPLGEK

SEQ ID NO: 626 - protein, 6 aa, Homo sapiens
IRGEPG

SEQ ID NO: 627 - protein, 6 aa, Homo sapiens
FPGPPG

SEQ ID NO: 628 - protein, 6 aa, Homo sapiens
LQGIRG

SEQ ID NO: 629 - protein, 6 aa, Homo sapiens
DGVIGM

SEQ ID NO: 630 - protein, 6 aa, Homo sapiens
PGNPGI

SEQ ID NO: 631 - protein, 6 aa, Homo sapiens
IKGDKG

SEQ ID NO: 632 - protein, 6 aa, Homo sapiens
PGSPGC

SEQ ID NO: 633 - protein, 6 aa, Homo sapiens
GPPGVP

SEQ ID NO: 634 - protein, 6 aa, Homo sapiens
DQGDQG

SEQ ID NO: 635 - protein, 6 aa, Homo sapiens
KGSIGI

SEQ ID NO: 636 - protein, 6 aa, Homo sapiens
PPGRLG

SEQ ID NO: 637 - protein, 6 aa, Homo sapiens
EKGQKG

SEQ ID NO: 638 - protein, 6 aa, Homo sapiens
DGGVPN

SEQ ID NO: 639 - protein, 6 aa, Homo sapiens
SGRDGL

SEQ ID NO: 640 - protein, 6 aa, Homo sapiens
  MOD_RES 2..3: note = Proline or hydroxyproline
GXXGEK

SEQ ID NO: 641 - protein, 6 aa, Homo sapiens
AEGLPG

SEQ ID NO: 642 - protein, 6 aa, Homo sapiens
DGYRGP

SEQ ID NO: 643 - protein, 6 aa, Homo sapiens
GPPGLM

SEQ ID NO: 644 - protein, 6 aa, Homo sapiens
LPGFAG

SEQ ID NO: 645 - protein, 6 aa, Homo sapiens
GIPGMP

SEQ ID NO: 646 - protein, 6 aa, Homo sapiens
SVDHGF

SEQ ID NO: 647 - protein, 6 aa, Homo sapiens
PSVDHG

SEQ ID NO: 648 - protein, 6 aa, Homo sapiens
VDHGFL

SEQ ID NO: 649 - protein, 6 aa, Homo sapiens
PGQPGY

SEQ ID NO: 650 - protein, 6 aa, Homo sapiens
QPGYTN

SEQ ID NO: 651 - protein, 6 aa, Homo sapiens
PGLPGS

SEQ ID NO: 652 - protein, 6 aa, Homo sapiens
GTPSVD

SEQ ID NO: 653 - protein, 6 aa, Homo sapiens
SVGSPG

SEQ ID NO: 654 - protein, 6 aa, Homo sapiens
LPGSMG

SEQ ID NO: 655 - protein, 6 aa, Homo sapiens
PGFPGL

SEQ ID NO: 656 - protein, 6 aa, Homo sapiens
PGLPGE

SEQ ID NO: 657 - protein, 6 aa, Homo sapiens
HQGEMG

SEQ ID NO: 658 - protein, 6 aa, Homo sapiens
GPPGLV

SEQ ID NO: 659 - protein, 6 aa, Homo sapiens
PGIPGP

SEQ ID NO: 660 - protein, 6 aa, Homo sapiens
PGFPGT

SEQ ID NO: 661 - protein, 6 aa, Homo sapiens
DGIPGP

SEQ ID NO: 662 - protein, 6 aa, Homo sapiens
DGIPGP

SEQ ID NO: 663 - protein, 6 aa, Homo sapiens
PGPRGE

SEQ ID NO: 664 - protein, 6 aa, Homo sapiens
  MOD_RES 5: note = Proline or hydroxyproline
GQGPXG

SEQ ID NO: 665 - protein, 6 aa, Homo sapiens
KVDMGS

SEQ ID NO: 666 - protein, 6 aa, Homo sapiens
PGIDGV

SEQ ID NO: 667 - protein, 6 aa, Homo sapiens
KGHMGE

SEQ ID NO: 668 - protein, 6 aa, Homo sapiens
PGAIGP

SEQ ID NO: 669 - protein, 6 aa, Homo sapiens
KGLPGP

SEQ ID NO: 670 - protein, 6 aa, Homo sapiens
GPKGLP

SEQ ID NO: 671 - protein, 6 aa, Homo sapiens
GPKGPP

SEQ ID NO: 672 - protein, 6 aa, Homo sapiens
SPGPPG

SEQ ID NO: 673 - protein, 6 aa, Homo sapiens
GSVGYP

SEQ ID NO: 674 - protein, 6 aa, Homo sapiens
PPGSPG

SEQ ID NO: 675 - protein, 6 aa, Homo sapiens
GEPGPP

SEQ ID NO: 676 - protein, 6 aa, Homo sapiens
AGNPGP

SEQ ID NO: 677 - protein, 6 aa, Homo sapiens
PGIKGS

SEQ ID NO: 678 - protein, 6 aa, Homo sapiens
PGYTNG

SEQ ID NO: 679 - protein, 6 aa, Homo sapiens
FPGPQG

SEQ ID NO: 680 - protein, 6 aa, Homo sapiens
LSGPPG

SEQ ID NO: 681 - protein, 6 aa, Homo sapiens
GVMGTP

SEQ ID NO: 682 - protein, 6 aa, Homo sapiens
GVSGPK

SEQ ID NO: 683 - protein, 15 aa, Homo sapiens
  MOD_RES 4: note = Proline or hydroxyproline
  MOD_RES 6: note = Proline or hydroxyproline
  MOD_RES 9: note = Proline or hydroxyproline
KGDXGXPGXIGSLGH

SEQ ID NO: 684 - protein, 14 aa, Homo sapiens
GLRGIPGPVGEPGL

SEQ ID NO: 685 - protein, 17 aa, Homo sapiens
VIGPPGLQGLPGPPGEK

SEQ ID NO: 686 - protein, 17 aa, Homo sapiens
  MOD_RES 6: note = Proline or hydroxyproline
  MOD_RES 15: note = Proline or hydroxyproline
GKDGIXGPLGPLGPXGA

SEQ ID NO: 687 - protein, 16 aa, Homo sapiens
GLRGIPGPVGEPGLLG

SEQ ID NO: 688 - protein, 17 aa, Homo sapiens
GVLGPQGKTGEVGPLGE

SEQ ID NO: 689 - protein, 18 aa, Homo sapiens
KDGIPGPLGPLGPPGAAG

SEQ ID NO: 690 - protein, 17 aa, Homo sapiens
  MOD_RES 12: note = proline or hydroxyproline
GEDGERGAEGPXGPTGQ

SEQ ID NO: 691 - protein, 17 aa, Homo sapiens
  MOD_RES 6: note = Proline or hydroxyproline
  MOD_RES 9: note = Proline or hydroxyproline
  MOD_RES 11: note = Proline or hydroxyproline
  MOD_RES 15: note = Proline or hydroxyproline
GLQGPXGFXGXKGPXGH

SEQ ID NO: 692 - protein, 19 aa, Homo sapiens
PIGSLGHPGPPGVAGPLGQ

SEQ ID NO: 693 - protein, 16 aa, Homo sapiens
GIRGPPGTVIMMPFQF

SEQ ID NO: 694 - protein, 19 aa, Homo sapiens
  MOD_RES 6: note = proline or hydroxyproline
  MOD_RES 11: note = proline or hydroxyproline
  MOD_RES 15: note = proline or hydroxyproline
GQMGPXGPLGXSGLXGLKG

SEQ ID NO: 695 - protein, 20 aa, Homo sapiens
GLLGAPGQMGPPGPLGPSGL

SEQ ID NO: 696 - protein, 20 aa, Homo sapiens
  MOD_RES 6: note = proline or hydroxyproline
  MOD_RES 12: note = proline or hydroxyproline
  MOD_RES 18: note = proline or hydroxyproline
GLRGIXGPVGEXGLLGAXGQ

SEQ ID NO: 697 - protein, 20 aa, Homo sapiens
  MOD_RES 9: note = proline or hydroxyproline
  MOD_RES 15: note = proline or hydroxyproline
GLLGPRGSXGPTGRXGVTGI

SEQ ID NO: 698 - protein, 17 aa, Homo sapiens
GIRGPPGTVIMMPFQFA

SEQ ID NO: 699 - protein, 21 aa, Homo sapiens
GKDGIPGPLGPLGPPGAAGPS

SEQ ID NO: 700 - protein, 23 aa, Homo sapiens
  MOD_RES 8: note = proline or hydroxyproline
  MOD_RES 15: note = proline or hydroxyproline
GKDGIPGXLGPLGPXGAAGPSGE

SEQ ID NO: 701 - protein, 24 aa, Homo sapiens
  MOD_RES 13: note = lysine or hydroxylysine
  MOD_RES 19: note = proline or hydroxyproline
QGLPGLEGREGAXGELGPXGPLGK

SEQ ID NO: 702 - protein, 30 aa, Homo sapiens
  MOD_RES 7: note = lysine or hydroxylysine
  MOD_RES 16: note = proline or hydroxyproline
  MOD_RES 24: note = proline or hydroxyproline
LGPIGEXGKSGKTGQXGLEGERGXPGSRGE

SEQ ID NO: 703 - protein, 32 aa, Homo sapiens
  MOD_RES 8: note = proline or hydroxyproline
  MOD_RES 12: note = proline or hydroxyproline
  MOD_RES 18: note = proline or hydroxyproline
  MOD_RES 21: note = methionine or oxidised methionine
  MOD_RES 23: note = proline or hydroxyproline
GLRGIPGXVGEXGLLGAXGQXGXPGPLGPSGL

SEQ ID NO: 704 - protein, 35 aa, Homo sapiens
  MOD_RES 6: note = proline or hydroxyproline
  MOD_RES 21: note = proline or hydroxyproline
GANGSXGERGPLGPAGGIGLXGQSGSEGPVGPAGK

SEQ ID NO: 705 - protein, 38 aa, Homo sapiens
  MOD_RES 6: note = proline or hydroxyproline
  MOD_RES 11..12: note = proline or hydroxyproline
  MOD_RES 15: note = proline or hydroxyproline
  MOD_RES 18: note = proline or hydroxyproline
  MOD_RES 21: note = proline or hydroxyproline
  MOD_RES 26: note = proline or hydroxyproline
GLIGTXGEKGXXGNXGIXGLXGSDGXLGHPGHEGPTGE

SEQ ID NO: 706 - protein, 11 aa, Homo sapiens
  MOD_RES 3: note = proline or hydroxyproline
  MOD_RES 6: note = proline or hydroxyproline
GLXGEXGPRGL

SEQ ID NO: 707 - protein, 12 aa, Homo sapiens
  MOD_RES 10: note = methionine or oxidised methionine
LALRGPAGPXGL

SEQ ID NO: 708 - protein, 13 aa, Homo sapiens
  MOD_RES 11: note = methionine or oxidised methionine
RLALRGPAGPXGL

SEQ ID NO: 709 - protein, 17 aa, Homo sapiens
  MOD_RES 6: note = proline or hydroxyproline
  MOD_RES 12: note = proline or hydroxyproline
GLTGRXGPVGPXGSGGL

SEQ ID NO: 710 - protein, 17 aa, Homo sapiens
  MOD_RES 6: note = lysine or hydroxylysine
  MOD_RES 11..12: note = proline or hydroxyproline
  MOD_RES 14: note = proline or hydroxyproline
GLLGPXGPPGXXGXPGV

SEQ ID NO: 711 - protein, 17 aa, Homo sapiens
  MOD_RES 3: note = proline or hydroxyproline
  MOD_RES 6: note = proline or hydroxyproline
  MOD_RES 14: note = proline or hydroxyproline
GIXGRXGPQGPPGXAGE

SEQ ID NO: 712 - protein, 17 aa, Homo sapiens
  MOD_RES 3: note = proline or hydroxyproline
  MOD_RES 6: note = proline or hydroxyproline
  MOD_RES 13: note = proline or hydroxyproline
  MOD_RES 16: note = proline or hydroxyproline
PGXDGXPGPMGPXGLXG

SEQ ID NO: 713 - protein, 17 aa, Homo sapiens
  MOD_RES 3: note = proline or hydroxyproline
  MOD_RES 12: note = proline or hydroxyproline
GQXGPSGADGEXGPRGQ

SEQ ID NO: 714 - protein, 17 aa, Homo sapiens
  MOD_RES 12: note = proline or hydroxyproline
  MOD_RES 15: note = proline or hydroxyproline
GETGFQGKTGPXGPXGV

SEQ ID NO: 715 - protein, 16 aa, Homo sapiens
  MOD_RES 6: note = proline or hydroxyproline
  MOD_RES 12: note = proline or hydroxyproline
GLRGFXGDRGLXGPVG

SEQ ID NO: 716 - protein, 17 aa, Homo sapiens
  MOD_RES 6: note = proline or hydroxyproline
  MOD_RES 12: note = proline or hydroxyproline
GLRGFXGDRGLXGPVGA

SEQ ID NO: 717 - protein, 20 aa, Homo sapiens
  MOD_RES 12: note = proline or hydroxyproline
  MOD_RES 15: note = proline or hydroxyproline
GKTGPIGPQGAXGKXGPDGL

SEQ ID NO: 718 - protein, 20 aa, Homo sapiens
  MOD_RES 2..3: note = proline or hydroxyproline
  MOD_RES 6: note = proline or hydroxyproline
  MOD_RES 9: note = proline or hydroxyproline
  MOD_RES 17..18: note = proline or hydroxyproline
GXXGRXGLPGADGLPGXXGT

SEQ ID NO: 719 - protein, 21 aa, Homo sapiens
  MOD_RES 3: note = lysine or hydroxylysine
  MOD_RES 12: note = proline or hydroxyproline
GLXGNEGPPGPXGPAGSPGER

SEQ ID NO: 720 - protein, 20 aa, Homo sapiens
  MOD_RES 6: note = proline or hydroxyproline
  MOD_RES 12: note = proline or hydroxyproline
GLRGFXGDRGLXGPVGALGL

SEQ ID NO: 721 - protein, 20 aa, Homo sapiens
  MOD_RES 6: note = proline or hydroxyproline
  MOD_RES 9: note = proline or hydroxyproline
  MOD_RES 12: note = proline or hydroxyproline
  MOD_RES 18: note = proline or hydroxyproline
GERGHXGPXGPXGEQGLXGL

SEQ ID NO: 722 - protein, 21 aa, Homo sapiens
  MOD_RES 4: note = proline or hydroxyproline
  MOD_RES 10: note = lysine or hydroxylysine
  MOD_RES 16: note = proline or hydroxyproline
IGPXGEQGEXGDRGLXGPQGS

SEQ ID NO: 723 - protein, 24 aa, Homo sapiens
  MOD_RES 9: note = proline or hydroxyproline
  MOD_RES 11..12: note = proline or hydroxyproline
  MOD_RES 14: note = proline or hydroxyproline
GEAGHPGPXGXXGXPGEVIQPLPI

SEQ ID NO: 724 - protein, 26 aa, Homo sapiens
  MOD_RES 2: note = proline or hydroxyproline
  MOD_RES 5: note = lysine or hydroxylysine
  MOD_RES 22: note = proline or hydroxyproline
  MOD_RES 25: note = proline or hydroxyproline
KXGPXGNSGGDGPAGPPGERGXNGXQ

SEQ ID NO: 725 - protein, 26 aa, Homo sapiens
  MOD_RES 6: note = proline or hydroxyproline
  MOD_RES 9: note = proline or hydroxyproline
  MOD_RES 18: note = methionine or oxidised methionine
  MOD_RES 21: note = proline or hydroxyproline
  MOD_RES 24: note = proline or hydroxyproline
GEQGLXGSXGPDGPPGPXGPXGLXGL

SEQ ID NO: 726 - protein, 27 aa, Homo sapiens
  MOD_RES 3..4: note = proline or hydroxyproline
  MOD_RES 12: note = proline or hydroxyproline
  MOD_RES 24: note = proline or hydroxyproline
EGXXGEKGGQGXPGPQGPIGYPGXRGV

SEQ ID NO: 727 - protein, 26 aa, Homo sapiens
  MOD_RES 3: note = proline or hydroxyproline
  MOD_RES 5: note = proline or hydroxyproline
  MOD_RES 8: note = proline or hydroxyproline
  MOD_RES 12: note = proline or hydroxyproline
  MOD_RES 18: note = proline or hydroxyproline
  MOD_RES 21: note = proline or hydroxyproline
GFXGXKGXPGPXGKDGLXGHXGQRGE

SEQ ID NO: 728 - protein, 11 aa, Homo sapiens
LPFRFGGGGDA

SEQ ID NO: 729 - protein, 11 aa, Homo sapiens
GSKGPMVSAQE

SEQ ID NO: 730 - protein, 11 aa, Homo sapiens
QESQAQAILQQ

SEQ ID NO: 731 - protein, 14 aa, Homo sapiens
  MOD_RES 6: note = proline or hydroxyproline
  MOD_RES 9: note = lysine or hydroxylysine
GAIGPXGEXGPLGK

SEQ ID NO: 732 - protein, 15 aa, Homo sapiens
  MOD_RES 3: note = proline or hydroxyproline
  MOD_RES 13: note = proline or hydroxyproline
GGXNGDPGPLGPXGE

SEQ ID NO: 733 - protein, 14 aa, Homo sapiens
  MOD_RES 2: note = proline or hydroxyproline
  MOD_RES 4..5: note = proline or hydroxyproline
  MOD_RES 11: note = proline or hydroxyproline
PXGXXGEQGLXGLA

SEQ ID NO: 734 - protein, 17 aa, Homo sapiens
  MOD_RES 11..12: note = proline or hydroxyproline
  MOD_RES 14: note = proline or hydroxyproline
GLLGPKGPPGXXGXPGV

SEQ ID NO: 735 - protein, 17 aa, Homo sapiens
  MOD_RES 6: note = proline or hydroxyproline
  MOD_RES 12: note = proline or hydroxyproline
GQQGNXGAQGLXGPQGA

SEQ ID NO: 736 - protein, 17 aa, Homo sapiens
  MOD_RES 2: note = lysine or hydroxylysine
  MOD_RES 5: note = proline or hydroxyproline
  MOD_RES 15: note = proline or hydroxyproline
GXEGXPGEKGGQGPXGP

SEQ ID NO: 737 - protein, 17 aa, Homo sapiens
  MOD_RES 12: note = proline or hydroxyproline
  MOD_RES 15: note = proline or hydroxyproline
GETGFQGKTGPXGPXGV

SEQ ID NO: 738 - protein, 17 aa, Homo sapiens
  MOD_RES 3: note = lysine or hydroxylysine
  MOD_RES 6: note = proline or hydroxyproline
  MOD_RES 15: note = proline or hydroxyproline
GEXGHXGLIGLIGPXGE

SEQ ID NO: 739 - protein, 20 aa, Homo sapiens
  MOD_RES 12: note = proline or hydroxyproline
  MOD_RES 15: note = proline or hydroxyproline
GKTGPIGPQGAXGKXGPDGL

SEQ ID NO: 740 - protein, 20 aa, Homo sapiens
  MOD_RES 3: note = proline or hydroxyproline
  MOD_RES 6: note = proline or hydroxyproline
  MOD_RES 12..13: note = proline or hydroxyproline
  MOD_RES 16: note = proline or hydroxyproline
PGXDGXPGPMGXXGLXGLKG

SEQ ID NO: 741 - protein, 26 aa, Homo sapiens
  MOD_RES 15: note = proline or hydroxyproline
  MOD_RES 17: note = proline or hydroxyproline
  MOD_RES 20..21: note = proline or hydroxyproline
GERGPNGPQGPTGFXGXKGXXGPPGK

SEQ ID NO: 742 - protein, 26 aa, Homo sapiens
  MOD_RES 7..8: note = proline or hydroxyproline
LIGLIGXXGEQGEKGDRGLPGPQGSS

SEQ ID NO: 743 - protein, 31 aa, Homo sapiens
  MOD_RES 4: note = proline or hydroxyproline
  MOD_RES 6..7: note = proline or hydroxyproline
IGPXGXXGLPGPPGPKGAKGSSGPTGPKGEA

SEQ ID NO: 744 - protein, 30 aa, Homo sapiens
  MOD_RES 4..5: note = proline or hydroxyproline
  MOD_RES 8: note = lysine or hydroxylysine
  MOD_RES 14: note = proline or hydroxyproline
PLGXXGEXGKLGVXGLPGYPGRQGPKGSIG

SEQ ID NO: 745 - protein, 33 aa, Homo sapiens
  MOD_RES 13: note = proline or hydroxyproline
  MOD_RES 19: note = lysine or hydroxylysine
  MOD_RES 25: note = proline or hydroxyproline
  MOD_RES 28: note = proline or hydroxyproline
QGPKGSIGFPGFXGANGEXGGRGTXGKXGPRGQ

SEQ ID NO: 746 - protein, 15 aa, Homo sapiens
  MOD_RES 10: note = proline or hydroxyproline
PGPKGDPGPXGPIGS

SEQ ID NO: 747 - protein, 14 aa, Homo sapiens
  MOD_RES 2: note = proline or hydroxyproline
  MOD_RES 5: note = proline or hydroxyproline
  MOD_RES 11: note = proline or hydroxyproline
AXGIXGEKGLXGLQ

SEQ ID NO: 748 - protein, 16 aa, Homo sapiens
  MOD_RES 3..4: note = proline or hydroxyproline
  MOD_RES 6: note = proline or hydroxyproline
  MOD_RES 10: note = proline or hydroxyproline
  MOD_RES 12: note = proline or hydroxyproline
  MOD_RES 15: note = proline or hydroxyproline
QGXXGXKGDXGXPGXI

SEQ ID NO: 749 - protein, 17 aa, Homo sapiens
  MOD_RES 6: note = proline or hydroxyproline
  MOD_RES 9: note = proline or hydroxyproline
GSLGHXGPXGVAGPLGQ

SEQ ID NO: 750 - protein, 17 aa, Homo sapiens
  MOD_RES 12: note = proline or hydroxyproline
GELGFQGQTGPXGPAGV

SEQ ID NO: 751 - protein, 17 aa, Homo sapiens
  MOD_RES 3: note = lysine or hydroxylysine
  MOD_RES 15: note = proline or hydroxyproline
GEXGHIGLIGLIGPXGE

SEQ ID NO: 752 - protein, 20 aa, Homo sapiens
  MOD_RES 2: note = proline or hydroxyproline
  MOD_RES 12: note = proline or hydroxyproline
GXVGEPGLLGAXGQMGPPGP

SEQ ID NO: 753 - protein, 26 aa, Homo sapiens
  MOD_RES 11: note = proline or hydroxyproline
  MOD_RES 14: note = lysine or hydroxylysine
  MOD_RES 18: note = proline or hydroxyproline
GSRGERGPPGXTGXDGIXGPLGPLGP

SEQ ID NO: 754 - protein, 26 aa, Homo sapiens
  MOD_RES 5: note = lysine or hydroxylysine
  MOD_RES 12: note = proline or hydroxyproline
  MOD_RES 21: note = proline or hydroxyproline
GEKGXSGKTGQXGLEGERGPXGSRGE

SEQ ID NO: 755 - protein, 10 aa, Homo sapiens
  MOD_RES 2: note = proline or hydroxyproline
  MOD_RES 5: note = proline or hydroxyproline
LXGEXGPRGL

SEQ ID NO: 756 - protein, 11 aa, Homo sapiens
  MOD_RES 9: note = methionine or oxidised methionine
ALRGPAGPXGL

SEQ ID NO: 757 - protein, 35 aa, Homo sapiens
  MOD_RES 8..9: note = proline or hydroxyproline
  MOD_RES 14: note = proline or hydroxyproline
  MOD_RES 18: note = proline or hydroxyproline
  MOD_RES 21: note = proline or hydroxyproline
  MOD_RES 23: note = methionine or oxidised methionine
  MOD_RES 24: note = proline or hydroxyproline
  MOD_RES 29..30: note = proline or hydroxyproline
  MOD_RES 33: note = proline or hydroxyproline
GPQGAIGXXGEKGXLGKXGLXGXXGADGXXGHXGK

SEQ ID NO: 758 - protein, 36 aa, Homo sapiens
  MOD_RES 15..16: note = proline or hydroxyproline
  MOD_RES 22: note = lysine or hydroxylysine
  MOD_RES 25: note = proline or hydroxyproline
AGPMGLTGRPGPVGXXGSGGLXGEXGDVGPQGPRGV

SEQ ID NO: 759 - protein, 35 aa, Homo sapiens
  MOD_RES 8: note = proline or hydroxyproline
  MOD_RES 12: note = proline or hydroxyproline
  MOD_RES 18: note = proline or hydroxyproline
  MOD_RES 21: note = methionine or oxidised methionine
  MOD_RES 23..24: note = proline or hydroxyproline
GLRGIPGXVGEXGLLGAXGQXGXXGPLGPSGLPGL

SEQ ID NO: 760 - protein, 6 aa, Homo sapiens
  MOD_RES 5: note = proline or hydroxyproline
LRGIXG

SEQ ID NO: 761 - protein, 6 aa, Homo sapiens
IGPPGI

SEQ ID NO: 762 - protein, 6 aa, Homo sapiens
IGSLGH

SEQ ID NO: 763 - protein, 6 aa, Homo sapiens
IRGPPG

SEQ ID NO: 764 - protein, 6 aa, Homo sapiens
  MOD_RES 5: note = proline or hydroxyproline
ANGSXG

SEQ ID NO: 765 - protein, 6 aa, Homo sapiens
  MOD_RES 5: note = proline or hydroxyproline
LIGTXG

SEQ ID NO: 766 - protein, 6 aa, Homo sapiens
  MOD_RES 2: note = proline or hydroxyproline
  MOD_RES 5: note = proline or hydroxyproline
LXGEXG

SEQ ID NO: 767 - protein, 6 aa, Homo sapiens
  MOD_RES 2: note = proline or hydroxyproline
  MOD_RES 5: note = proline or hydroxyproline
IXGRXG

SEQ ID NO: 768 - protein, 6 aa, Homo sapiens
  MOD_RES 2: note = proline or hydroxyproline
  MOD_RES 5: note = proline or hydroxyproline
GXDGXP

SEQ ID NO: 769 - protein, 6 aa, Homo sapiens
  MOD_RES 2: note = proline or hydroxyproline
QXGPSG

SEQ ID NO: 770 - protein, 6 aa, Homo sapiens
  MOD_RES 2: note = lysine or hydroxylysine
LXGNEG

SEQ ID NO: 771 - protein, 6 aa, Homo sapiens
  MOD_RES 5: note = proline or hydroxyproline
ERGHXG

SEQ ID NO: 772 - protein, 6 aa, Homo sapiens
  MOD_RES 3: note = proline or hydroxyproline
GPXGEQ

SEQ ID NO: 773 - protein, 6 aa, Homo sapiens
PFRFGG

SEQ ID NO: 774 - protein, 6 aa, Homo sapiens
ESQAQA

SEQ ID NO: 775 - protein, 6 aa, Homo sapiens
  MOD_RES 5: note = lysine or hydroxylysine
LLGPXG

SEQ ID NO: 776 - protein, 6 aa, Homo sapiens
  MOD_RES 5: note = proline or hydroxyproline
QQGNXG

SEQ ID NO: 777 - protein, 6 aa, Homo sapiens
  MOD_RES 1: note = lysine or hydroxylysine
  MOD_RES 4: note = proline or hydroxyproline
XEGXPG

SEQ ID NO: 778 - protein, 6 aa, Homo sapiens
  MOD_RES 6: note = proline or hydroxyproline
IGLIGX

SEQ ID NO: 779 - protein, 6 aa, Homo sapiens
  MOD_RES 3..4: note = proline or hydroxyproline
LGXXGE

SEQ ID NO: 780 - skipped

SEQ ID NO: 781 - protein, 6 aa, Homo sapiens
  MOD_RES 5: note = proline or hydroxyproline
SLGHXG

SEQ ID NO: 782 - protein, 6 aa, Homo sapiens
  MOD_RES 5: note = proline or hydroxyproline
KDGIXG

SEQ ID NO: 783 - protein, 6 aa, Homo sapiens
  MOD_RES 5: note = proline or hydroxyproline
PVGEPG

SEQ ID NO: 784 - protein, 6 aa, Homo sapiens
  MOD_RES 1: note = proline or hydroxyproline
  MOD_RES 4: note = proline or hydroxyproline
XGEXGP

SEQ ID NO: 785 - protein, 6 aa, Homo sapiens
  MOD_RES 5: note = proline or hydroxyproline
LLGAXG

SEQ ID NO: 786 - protein, 6 aa, Homo sapiens
GLPGLE

SEQ ID NO: 787 - protein, 6 aa, Homo sapiens
GIPGEK

SEQ ID NO: 788 - protein, 6 aa, Homo sapiens
LALRGP

SEQ ID NO: 789 - protein, 6 aa, Homo sapiens
  MOD_RES 5: note = proline or hydroxyproline
LTGRXG

SEQ ID NO: 790 - protein, 6 aa, Homo sapiens
  MOD_RES 5: note = proline or hydroxyproline
LRGFXG

SEQ ID NO: 791 - protein, 6 aa, Homo sapiens
KTGPIG

SEQ ID NO: 792 - skipped

SEQ ID NO: 793 - protein, 6 aa, Homo sapiens
  MOD_RES 5: note = proline or hydroxyproline
EQGLXG

SEQ ID NO: 794 - protein, 6 aa, Homo sapiens
  MOD_RES 6: note = proline or hydroxyproline
AIGGPX

SEQ ID NO: 795 - protein, 6 aa, Homo sapiens
  MOD_RES 2: note = proline or hydroxyproline
GXNGDP

SEQ ID NO: 796 - skipped

SEQ ID NO: 797 - protein, 6 aa, Homo sapiens
LLGPRG

SEQ ID NO: 798 - protein, 6 aa, Homo sapiens
ERGPNG

SEQ ID NO: 799 - protein, 6 aa, Homo sapiens
GPKGDP

SEQ ID NO: 800 - protein, 6 aa, Homo sapiens
  MOD_RES 1: note = proline or hydroxyproline
  MOD_RES 4: note = proline or hydroxyproline
XGIXGE

SEQ ID NO: 801 - protein, 6 aa, Homo sapiens
  MOD_RES 2: note = lysine or hydroxylysine
EXGHIG

SEQ ID NO: 802 - protein, 6 aa, Homo sapiens
  MOD_RES 5: note = proline or hydroxyproline
QMGPXG

SEQ ID NO: 803 - protein, 6 aa, Homo sapiens
SRGERG

SEQ ID NO: 804 - protein, 6 aa, Homo sapiens
  MOD_RES 4: note = lysine or hydroxylysine
EKGXSG

SEQ ID NO: 805 - protein, 6 aa, Homo sapiens
  MOD_RES 6: note = lysine or hydroxylysine
GPIGEX

SEQ ID NO: 806 - protein, 6 aa, Homo sapiens
PQGAIG

SEQ ID NO: 807 - protein, 6 aa, Homo sapiens
GPMGLT

SEQ ID NO: 808 - protein, 6 aa, Homo sapiens
ETGFQG

SEQ ID NO: 809 - protein, 6 aa, Homo sapiens
GSKGPM

SEQ ID NO: 810 - protein, 6 aa, Homo sapiens
ALRGPA

SEQ ID NO: 811 - protein, 6 aa, Homo sapiens
EAGHPG

SEQ ID NO: 812 - protein, 6 aa, Homo sapiens
  MOD_RES 2: note = lysine or hydroxylysine
  MOD_RES 5: note = proline or hydroxyproline
EXGHXG

SEQ ID NO: 813 - protein, 5 aa, Homo sapiens
KDGIP

SEQ ID NO: 814 - protein, 6 aa, Homo sapiens
VLGPQG

SEQ ID NO: 815 - protein, 6 aa, Homo sapiens
EDGERG

SEQ ID NO: 816 - protein, 6 aa, Homo sapiens
GPKGSI

SEQ ID NO: 817 - protein, 6 aa, Homo sapiens
ELGFQG

SEQ ID NO: 818 - protein, 6 aa, Homo sapiens
LRGPAG

SEQ ID NO: 819 - protein, 6 aa, Homo sapiens
PIGSLG

SEQ ID NO: 820 - protein, 6 aa, Homo sapiens
  MOD_RES 2: note = proline or hydroxyproline
PXGPTG

SEQ ID NO: 821 - protein, 6 aa, Homo sapiens
  MOD_RES 1: note = proline or hydroxyproline
  MOD_RES 5: note = proline or hydroxyproline
XKGPXG

SEQ ID NO: 822 - protein, 6 aa, Homo sapiens
VAGPLG

SEQ ID NO: 823 - protein, 6 aa, Homo sapiens
  MOD_RES 2: note = proline or hydroxyproline
RXGVTG

SEQ ID NO: 824 - protein, 6 aa, Homo sapiens
MMPFQF

SEQ ID NO: 825 - protein, 6 aa, Homo sapiens
PGAAGP

SEQ ID NO: 826 - protein, 6 aa, Homo sapiens
PVGPAG

SEQ ID NO: 827 - protein, 6 aa, Homo sapiens
HEGPTG

SEQ ID NO: 828 - protein, 6 aa, Homo sapiens
  MOD_RES 3: note = proline or hydroxyproline
  MOD_RES 6: note = proline or hydroxyproline
GPXGLX

SEQ ID NO: 829 - protein, 6 aa, Homo sapiens
AGSPGE

SEQ ID NO: 830 - protein, 6 aa, Homo sapiens
PVGALG

SEQ ID NO: 831 - protein, 6 aa, Homo sapiens
  MOD_RES 4: note = proline or hydroxyproline
YPGXRG

SEQ ID NO: 832 - protein, 6 aa, Homo sapiens
  MOD_RES 2: note = proline or hydroxyproline
HXGQRG

SEQ ID NO: 833 - protein, 6 aa, Homo sapiens
GGGGDA

SEQ ID NO: 834 - protein, 6 aa, Homo sapiens
  MOD_RES 5: note = proline or hydroxyproline
LIGPXG

SEQ ID NO: 835 - protein, 6 aa, Homo sapiens
  MOD_RES 3: note = proline or hydroxyproline
GLXGLK

SEQ ID NO: 836 - protein, 6 aa, Homo sapiens
  MOD_RES 4: note = proline or hydroxyproline
KGLXGL

SEQ ID NO: 837 - protein, 6 aa, Homo sapiens
QQARLA

SEQ ID NO: 838 - skipped

SEQ ID NO: 839 - protein, 6 aa, Homo sapiens
  MOD_RES 5: note = proline or hydroxyproline
PLGPXG

SEQ ID NO: 840 - protein, 6 aa, Homo sapiens
GEPGLL

SEQ ID NO: 841 - protein, 6 aa, Homo sapiens
EVGPLG

SEQ ID NO: 842 - protein, 6 aa, Homo sapiens
IMMPFQ

SEQ ID NO: 843 - protein, 6 aa, Homo sapiens
PLGPSG

SEQ ID NO: 844 - protein, 6 aa, Homo sapiens
AAGPSG

SEQ ID NO: 845 - protein, 6 aa, Homo sapiens
  MOD_RES 2: note = proline or hydroxyproline
PXGPLG

SEQ ID NO: 846 - protein, 6 aa, Homo sapiens
  MOD_RES 1: note = proline or hydroxyproline
  MOD_RES 2: note = proline or hydroxyproline
XXGSRG

SEQ ID NO: 847 - protein, 6 aa, Homo sapiens
  MOD_RES 5: note = methionine or oxidised methionine
PAGPXG

SEQ ID NO: 848 - protein, 6 aa, Homo sapiens
  MOD_RES 2: note = proline or hydroxyproline
PXGSGG

SEQ ID NO: 849 - protein, 6 aa, Homo sapiens
  MOD_RES 3: note = proline or hydroxyproline
GLXGPV

SEQ ID NO: 850 - protein, 6 aa, Homo sapiens
  MOD_RES 2: note = proline or hydroxyproline
LXGPVG

SEQ ID NO: 851 - protein, 6 aa, Homo sapiens
  MOD_RES 2: note = proline or hydroxyproline
KXGPDG

SEQ ID NO: 852 - protein, 6 aa, Homo sapiens
  MOD_RES 2: note = proline or hydroxyproline
LXGPQG

SEQ ID NO: 853 - protein, 6 aa, Homo sapiens
VIQPLP

SEQ ID NO: 854 - protein, 6 aa, Homo sapiens
RGPNGP

SEQ ID NO: 855 - protein, 6 aa, Homo sapiens
PGPQGS

SEQ ID NO: 856 - protein, 6 aa, Homo sapiens
  MOD_RES 2: note = Lysine or hydroxylysine
EXGPLG

SEQ ID NO: 857 - protein, 6 aa, Homo sapiens
GPPGAA

SEQ ID NO: 858 - protein, 6 aa, Homo sapiens
TGPKGE

SEQ ID NO: 859 - protein, 6 aa, Homo sapiens
  MOD_RES 4: note = proline or hydroxyproline
QGLXGL

SEQ ID NO: 860 - protein, 6 aa, Homo sapiens
PSGLPG

SEQ ID NO: 861 - protein, 6 aa, Homo sapiens
  MOD_RES 2: note = proline or hydroxyproline
  MOD_RES 5: note = proline or hydroxyproline
PXGLXG

SEQ ID NO: 862 - protein, 6 aa, Homo sapiens
  MOD_RES 2: note = proline or hydroxyproline
KXGPRG

SEQ ID NO: 863 - protein, 6 aa, Homo sapiens
PLGPLG

SEQ ID NO: 864 - protein, 14 aa, Homo sapiens
GYRGPEGPQGPPGH

SEQ ID NO: 865 - protein, 16 aa, Homo sapiens
GPIGPKGYRGDEGPPG

SEQ ID NO: 866 - protein, 12 aa, Homo sapiens
IGIGIGNADITE

SEQ ID NO: 867 - protein, 14 aa, Homo sapiens
GAQGPAGPAGPPGL

SEQ ID NO: 868 - protein, 14 aa, Homo sapiens
GLIGEQGISGPRGS

SEQ ID NO: 869 - protein, 15 aa, Homo sapiens
PPGLIGEQGISGPRG

SEQ ID NO: 870 - protein, 16 aa, Homo sapiens
EPGEPGPKGGIGNRGP

SEQ ID NO: 871 - protein, 26 aa, Homo sapiens
GISGPRGSGGAAGAPGERGRTGPLGR

SEQ ID NO: 872 - protein, 14 aa, Homo sapiens
PGPAGPPGDPGLMG

SEQ ID NO: 873 - protein, 28 aa, Homo sapiens
VAAKPAAVRPPAAAAAKPVATKPEVPRP

SEQ ID NO: 874 - protein, 14 aa, Homo sapiens
GEPGLNGTTGPKGI

SEQ ID NO: 875 - protein, 17 aa, Homo sapiens
IGPKGIPGEDGYRGYPG

SEQ ID NO: 876 - protein, 26 aa, Homo sapiens
VAVVQHAPSESVDNASMPPVKVEFSL

SEQ ID NO: 877 - protein, 10 aa, Homo sapiens
LGPMGVPGRD

SEQ ID NO: 878 - protein, 28 aa, Homo sapiens
GEPGPPGEKGEAGDEGNPGPDGAPGERG

SEQ ID NO: 879 - protein, 28 aa, Homo sapiens
RGPIGSIGPKGIPGEDGYRGYPGDEGGP

SEQ ID NO: 880 - protein, 11 aa, Homo sapiens
PPPPQPARSAS

SEQ ID NO: 881 - protein, 12 aa, Homo sapiens
FGPSAATPAPPG

SEQ ID NO: 882 - protein, 29 aa, Homo sapiens
GPKGETGDLGPMGVPGRDGVPGGPGETGK

SEQ ID NO: 883 - protein, 6 aa, Homo sapiens
YRGPEG

SEQ ID NO: 884 - protein, 16 aa, Homo sapiens
SSGIENGAFQGMKKLS

SEQ ID NO: 885 - protein, 6 aa, Homo sapiens
GIGIGN

SEQ ID NO: 886 - protein, 6 aa, Homo sapiens
ISGPRG

SEQ ID NO: 887 - protein, 6 aa, Homo sapiens
PGPAGP

SEQ ID NO: 888 - protein, 6 aa, Homo sapiens
VAAKPA

SEQ ID NO: 889 - protein, 6 aa, Homo sapiens
RGPIGS

SEQ ID NO: 890 - protein, 6 aa, Homo sapiens
PPPPQP

SEQ ID NO: 891 - protein, 6 aa, Homo sapiens
AQGPAG

SEQ ID NO: 892 - protein, 6 aa, Homo sapiens
LIGEQG

SEQ ID NO: 893 - protein, 6 aa, Homo sapiens
PGLIGE

SEQ ID NO: 894 - protein, 6 aa, Homo sapiens
GEPGLN

SEQ ID NO: 895 - protein, 6 aa, Homo sapiens
IGPKGI

SEQ ID NO: 896 - protein, 6 aa, Homo sapiens
VAVVQH

SEQ ID NO: 897 - protein, 6 aa, Homo sapiens
FGPSAA

SEQ ID NO: 898 - protein, 6 aa, Homo sapiens
GPKGET

SEQ ID NO: 899 - protein, 6 aa, Homo sapiens
LGPMGV

SEQ ID NO: 900 - protein, 6 aa, Homo sapiens
GDEGPP

SEQ ID NO: 901 - protein, 6 aa, Homo sapiens
GNADIT

SEQ ID NO: 902 - protein, 6 aa, Homo sapiens
DPGLMG

SEQ ID NO: 903 - protein, 6 aa, Homo sapiens
PEVPRP

SEQ ID NO: 904 - protein, 6 aa, Homo sapiens
TGPKGI

SEQ ID NO: 905 - protein, 6 aa, Homo sapiens
GDEGGP

SEQ ID NO: 906 - protein, 6 aa, Homo sapiens
PARSAS

SEQ ID NO: 907 - protein, 6 aa, Homo sapiens
GISGPR

SEQ ID NO: 908 - protein, 6 aa, Homo sapiens
GIGNRG

SEQ ID NO: 909 - protein, 6 aa, Homo sapiens
YRGYPG

SEQ ID NO: 910 - protein, 6 aa, Homo sapiens
KVEFSL

SEQ ID NO: 911 - protein, 6 aa, Homo sapiens
GVPGRD

SEQ ID NO: 912 - protein, 6 aa, Homo sapiens
PGETGK

SEQ ID NO: 913 - protein, 6 aa, Homo sapiens
RTGPLG

SEQ ID NO: 914 - protein, 6 aa, Homo sapiens
APGERG

SEQ ID NO: 915 - protein, 6 aa, Homo sapiens
TPAPPG

SEQ ID NO: 916 - protein, 22 aa, Homo sapiens
SVPKEISPDTTLLDLQNNDISE

SEQ ID NO: 917 - protein, 23 aa, Homo sapiens
KSVPKEISPDTTLLDLQNNDISE

SEQ ID NO: 918 - protein, 23 aa, Homo sapiens
NSGFEPGAFDGLKLNYLRISEAK

SEQ ID NO: 919 - protein, 24 aa, Homo sapiens
LKSVPKEISPDTTLLDLQNNDISE

SEQ ID NO: 920 - protein, 18 aa, Homo sapiens
LRISEAKLTGIPKDLPET

SEQ ID NO: 921 - protein, 26 aa, Homo sapiens
LTGIPKDLPETLNELHLDHNKIQAIE

SEQ ID NO: 922 - protein, 20 aa, Homo sapiens
RISEAKLTGIPKDLPETLNE

SEQ ID NO: 923 - protein, 12 aa, Homo sapiens
AIELEDLLRYSK

SEQ ID NO: 924 - protein, 10 aa, Homo sapiens
AIELEDLLRY

SEQ ID NO: 925 - protein, 17 aa, Homo sapiens
EAKLTGIPKDLPETLNE

SEQ ID NO: 926 - protein, 24 aa, Homo sapiens
LKAVPKEISPDTTLLDLQNNDISE

SEQ ID NO: 927 - protein, 16 aa, Homo sapiens
LLDLQNNDISELRKDD

SEQ ID NO: 928 - protein, 10 aa, Homo sapiens
IELEDLLRYS

SEQ ID NO: 929 - protein, 13 aa, Homo sapiens
NSGFEPGAFDGLK

SEQ ID NO: 930 - protein, 11 aa, Homo sapiens
IVIELGTNPLK

SEQ ID NO: 931 - protein, 14 aa, Homo sapiens
DEASGIGPEVPDDR

SEQ ID NO: 932 - protein, 15 aa, Homo sapiens
LHLDGNKISRVDAAS

SEQ ID NO: 933 - protein, 16 aa, Homo sapiens
VNNKISKVSPGAFTPL

SEQ ID NO: 934 - protein, 24 aa, Homo sapiens
LILVNNKISKVSPGAFTPLVKLER

SEQ ID NO: 935 - protein, 15 aa, Homo sapiens
SNPVQYWEIQPSTFR

SEQ ID NO: 936 - protein, 11 aa, Homo sapiens
KITEIKDGDFK

SEQ ID NO: 937 - protein, 15 aa, Homo sapiens
GLPPSLTELHLDGNK

SEQ ID NO: 938 - protein, 10 aa, Homo sapiens
LLASDAGLYR

SEQ ID NO: 939 - protein, 12 aa, Homo sapiens
LATVGELQAAWR

SEQ ID NO: 940 - protein, 13 aa, Homo sapiens
ETTVLVAQNGNIK

SEQ ID NO: 941 - protein, 11 aa, Homo sapiens
SLEDLQLTHNK

SEQ ID NO: 942 - protein, 11 aa, Homo sapiens
LKEDAVSAAFK

SEQ ID NO: 943 - protein, 14 aa, Homo sapiens
SIEYSPQLEDAGSR

SEQ ID NO: 944 - protein, 10 aa, Homo sapiens
LEGDTLIIPR

SEQ ID NO: 945 - protein, 14 aa, Homo sapiens
VSEAVVEKLEPEYR

SEQ ID NO: 946 - protein, 16 aa, Homo sapiens
SSGIENGAFQGMKKLS

SEQ ID NO: 947 - protein, 15 aa, Homo sapiens
EVSEAVVEKLEPEYR

SEQ ID NO: 948 - protein, 17 aa, Homo sapiens
SIEYSPQLEDASAKEFR

SEQ ID NO: 949 - protein, 6 aa, Homo sapiens
SVPKEI

SEQ ID NO: 950 - protein, 6 aa, Homo sapiens
GLKLNY

SEQ ID NO: 951 - protein, 6 aa, Homo sapiens
RISEAK

SEQ ID NO: 952 - protein, 6 aa, Homo sapiens
NSGFEP

SEQ ID NO: 953 - protein, 6 aa, Homo sapiens
LKSVPK

SEQ ID NO: 954 - protein, 6 aa, Homo sapiens
AIELED

SEQ ID NO: 955 - protein, 6 aa, Homo sapiens
QCSDLG

SEQ ID NO: 956 - protein, 6 aa, Homo sapiens
EAKLTG

SEQ ID NO: 957 - protein, 6 aa, Homo sapiens
IELEDL

SEQ ID NO: 958 - protein, 6 aa, Homo sapiens
LRISEA

SEQ ID NO: 959 - protein, 6 aa, Homo sapiens
LTGIPK

SEQ ID NO: 960 - protein, 6 aa, Homo sapiens
LKAVPK

SEQ ID NO: 961 - protein, 6 aa, Homo sapiens
LLDLQN

SEQ ID NO: 962 - protein, 6 aa, Homo sapiens
IVIELG

SEQ ID NO: 963 - protein, 6 aa, Homo sapiens
DEASGI

SEQ ID NO: 964 - protein, 6 aa, Homo sapiens
VNNKIS

SEQ ID NO: 965 - protein, 6 aa, Homo sapiens
NGLNQM

SEQ ID NO: 966 - protein, 6 aa, Homo sapiens
LHLDGN

SEQ ID NO: 967 - protein, 6 aa, Homo sapiens
LILVNN

SEQ ID NO: 968 - protein, 6 aa, Homo sapiens
SSGIEN

SEQ ID NO: 969 - protein, 6 aa, Homo sapiens
KITEIK

SEQ ID NO: 970 - protein, 6 aa, Homo sapiens
GLPPSL

SEQ ID NO: 971 - protein, 6 aa, Homo sapiens
SNPVQY

SEQ ID NO: 972 - protein, 6 aa, Homo sapiens
LLASDA

SEQ ID NO: 973 - protein, 6 aa, Homo sapiens
LATVGE

SEQ ID NO: 974 - protein, 6 aa, Homo sapiens
ETTVLV

SEQ ID NO: 975 - protein, 6 aa, Homo sapiens
ENQDAR

SEQ ID NO: 976 - protein, 6 aa, Homo sapiens
NGFDQC

SEQ ID NO: 977 - protein, 6 aa, Homo sapiens
SLTVVK

SEQ ID NO: 978 - protein, 6 aa, Homo sapiens
SLEDLQ

SEQ ID NO: 979 - protein, 6 aa, Homo sapiens
LKEDAV

SEQ ID NO: 980 - protein, 6 aa, Homo sapiens
HLQHNR

SEQ ID NO: 981 - protein, 6 aa, Homo sapiens
SIEYSP

SEQ ID NO: 982 - protein, 6 aa, Homo sapiens
LVNFTR

SEQ ID NO: 983 - protein, 6 aa, Homo sapiens
VSEAVV

SEQ ID NO: 984 - protein, 6 aa, Homo sapiens
EVSEAV

SEQ ID NO: 985 - protein, 6 aa, Homo sapiens
LQHNRL

SEQ ID NO: 986 - protein, 6 aa, Homo sapiens
NNDISE

SEQ ID NO: 987 - protein, 6 aa, Homo sapiens
YWEVQP

SEQ ID NO: 988 - protein, 6 aa, Homo sapiens
EDLLRY

SEQ ID NO: 989 - protein, 6 aa, Homo sapiens
KIQAIE

SEQ ID NO: 990 - protein, 6 aa, Homo sapiens
PETLNE

SEQ ID NO: 991 - protein, 6 aa, Homo sapiens
LRKDDF

SEQ ID NO: 992 - protein, 6 aa, Homo sapiens
LLRYSK

SEQ ID NO: 993 - protein, 6 aa, Homo sapiens
ELRKDD

SEQ ID NO: 994 - protein, 6 aa, Homo sapiens
KDLPET

SEQ ID NO: 995 - protein, 6 aa, Homo sapiens
DLLRYS

SEQ ID NO: 996 - protein, 6 aa, Homo sapiens
AFDGLK

SEQ ID NO: 997 - protein, 6 aa, Homo sapiens
LNELHL

SEQ ID NO: 998 - protein, 6 aa, Homo sapiens
GTNPLK

SEQ ID NO: 999 - protein, 6 aa, Homo sapiens
EVPDDR

SEQ ID NO: 1000 - protein, 6 aa, Homo sapiens
GAFTPL

SEQ ID NO: 1001 - protein, 6 aa, Homo sapiens
RVDAAS

SEQ ID NO: 1002 - protein, 6 aa, Homo sapiens
LVKLER

SEQ ID NO: 1003 - protein, 6 aa, Homo sapiens
GMKKLS

SEQ ID NO: 1004 - protein, 6 aa, Homo sapiens
KDGDFK

SEQ ID NO: 1005 - protein, 6 aa, Homo sapiens
HLDGNK

SEQ ID NO: 1006 - protein, 6 aa, Homo sapiens
QPSTFR

SEQ ID NO: 1007 - protein, 6 aa, Homo sapiens
AFQGMK

SEQ ID NO: 1008 - protein, 6 aa, Homo sapiens
CDVMYG

SEQ ID NO: 1009 - protein, 6 aa, Homo sapiens
QNGINK

SEQ ID NO: 1010 - protein, 6 aa, Homo sapiens
IGQDYK

SEQ ID NO: 1011 - protein, 6 aa, Homo sapiens
QLTHNK

SEQ ID NO: 1012 - protein, 6 aa, Homo sapiens
VSAAFK

SEQ ID NO: 1013 - protein, 6 aa, Homo sapiens
GLKSLE

SEQ ID NO: 1014 - protein, 6 aa, Homo sapiens
EDAGSR

SEQ ID NO: 1015 - protein, 6 aa, Homo sapiens
EFREVS

SEQ ID NO: 1016 - protein, 6 aa, Homo sapiens
VAQQDS

SEQ ID NO: 1017 - protein, 6 aa, Homo sapiens
SAKEFR

SEQ ID NO: 1018 - protein, 6 aa, Homo sapiens
LEPEYR

SEQ ID NO: 1019 - protein, 16 aa, Homo sapiens
KESDTSYVSLKAPLTK

SEQ ID NO: 1020 - protein, 16 aa, Homo sapiens
GGNFEGSQSLVGDIGN

SEQ ID NO: 1021 - protein, 16 aa, Homo sapiens
ALKYEVQGEVFTKPQL

SEQ ID NO: 1022 - protein, 14 aa, Homo sapiens
GIVEFWVDGKPRVR

SEQ ID NO: 1023 - protein, 10 aa, Homo sapiens
RKAFVFPKES

SEQ ID NO: 1024 - protein, 16 aa, Homo sapiens
KYEVQGEVFTKPQLWP

SEQ ID NO: 1025 - protein, 13 aa, Homo sapiens
DSFGGNFEGSQSL

SEQ ID NO: 1026 - protein, 12 aa, Homo sapiens
DFVLSPDEINTI

SEQ ID NO: 1027 - protein, 13 aa, Homo sapiens
SLKKGYTVGAEAS

SEQ ID NO: 1028 - protein, 12 aa, Homo sapiens
AFGQTDMSRKAF

SEQ ID NO: 1029 - protein, 14 aa, Homo sapiens
SLKKGYTVGAEASI

SEQ ID NO: 1030 - protein, 11 aa, Homo sapiens
GEVFTKPQLWP

SEQ ID NO: 1031 - protein, 15 aa, Homo sapiens
SIILGQEQDSFGGNF

SEQ ID NO: 1032 - protein, 14 aa, Homo sapiens
KYEVQGEVFTKPQL

SEQ ID NO: 1033 - protein, 6 aa, Homo sapiens
AFVFPK

SEQ ID NO: 1034 - protein, 8 aa, Homo sapiens
FGQTDMSR

SEQ ID NO: 1035 - protein, 9 aa, Homo sapiens
FGQTDMSRK

SEQ ID NO: 1036 - protein, 10 aa, Homo sapiens
FGQTDMSRKA

SEQ ID NO: 1037 - protein, 11 aa, Homo sapiens
FGQTDMSRKAF

SEQ ID NO: 1038 - protein, 16 aa, Homo sapiens
FGQTDMSRKAFVFPKE

SEQ ID NO: 1039 - protein, 20 aa, Homo sapiens
FGQTDMSRKAFVFPKESDTS

SEQ ID NO: 1040 - protein, 22 aa, Homo sapiens
FGQTDMSRKAFVFPKESDTSYV

SEQ ID NO: 1041 - protein, 23 aa, Homo sapiens
FGQTDMSRKAFVFPKESDTSYVS

SEQ ID NO: 1042 - protein, 19 aa, Homo sapiens
TDMSRKAFVFPKESDTSYV

SEQ ID NO: 1043 - protein, 15 aa, Homo sapiens
MSRKAFVFPKESDTS

SEQ ID NO: 1044 - protein, 16 aa, Homo sapiens
SRKAFVFPKESDTSYV

SEQ ID NO: 1045 - protein, 9 aa, Homo sapiens
RKAFVFPKE

SEQ ID NO: 1046 - protein, 15 aa, Homo sapiens
RKAFVFPKESDTSYV

SEQ ID NO: 1047 - protein, 16 aa, Homo sapiens
RKAFVFPKESDTSYVS

SEQ ID NO: 1048 - protein, 8 aa, Homo sapiens
KAFVFPKE

SEQ ID NO: 1049 - protein, 10 aa, Homo sapiens
KAFVFPKESD

SEQ ID NO: 1050 - protein, 11 aa, Homo sapiens
KAFVFPKESDT

SEQ ID NO: 1051 - protein, 12 aa, Homo sapiens
KAFVFPKESDTS

SEQ ID NO: 1052 - protein, 14 aa, Homo sapiens
KAFVFPKESDTSYV

SEQ ID NO: 1053 - protein, 15 aa, Homo sapiens
KAFVFPKESDTSYVS

SEQ ID NO: 1054 - protein, 7 aa, Homo sapiens
AFVFPKE

SEQ ID NO: 1055 - protein, 10 aa, Homo sapiens
AFVFPKESDT

SEQ ID NO: 1056 - protein, 13 aa, Homo sapiens
AFVFPKESDTSYV

SEQ ID NO: 1057 - protein, 14 aa, Homo sapiens
AFVFPKESDTSYVS

SEQ ID NO: 1058 - protein, 15 aa, Homo sapiens
AFVFPKESDTSYVSL

SEQ ID NO: 1059 - protein, 5 aa, Homo sapiens
FVFPK

SEQ ID NO: 1060 - protein, 6 aa, Homo sapiens
FVFPKE

SEQ ID NO: 1061 - protein, 8 aa, Homo sapiens
FVFPKESD

SEQ ID NO: 1062 - protein, 10 aa, Homo sapiens
FVFPKESDTS

SEQ ID NO: 1063 - protein, 11 aa, Homo sapiens
FVFPKESDTSY

SEQ ID NO: 1064 - protein, 12 aa, Homo sapiens
FVFPKESDTSYV

SEQ ID NO: 1065 - protein, 13 aa, Homo sapiens
FVFPKESDTSYVS

SEQ ID NO: 1066 - protein, 14 aa, Homo sapiens
FVFPKESDTSYVSL

SEQ ID NO: 1067 - protein, 9 aa, Homo sapiens
VFPKESDTS

SEQ ID NO: 1068 - protein, 11 aa, Homo sapiens
VFPKESDTSYV

SEQ ID NO: 1069 - protein, 12 aa, Homo sapiens
VFPKESDTSYVS

SEQ ID NO: 1070 - protein, 13 aa, Homo sapiens
VFPKESDTSYVSL

SEQ ID NO: 1071 - protein, 11 aa, Homo sapiens
FPKESDTSYVS

SEQ ID NO: 1072 - protein, 17 aa, Homo sapiens
KESDTSYVSLKAPLTKP

SEQ ID NO: 1073 - protein, 15 aa, Homo sapiens
SDTSYVSLKAPLTKP

SEQ ID NO: 1074 - protein, 9 aa, Homo sapiens
SLKAPLTKP

SEQ ID NO: 1075 - protein, 11 aa, Homo sapiens
SLKAPLTKPLK

SEQ ID NO: 1076 - protein, 10 aa, Homo sapiens
LKAPLTKPLK

SEQ ID NO: 1077 - protein, 12 aa, Homo sapiens
FYTELSSTRGYS

SEQ ID NO: 1078 - protein, 8 aa, Homo sapiens
LSSTRGYS

SEQ ID NO: 1079 - protein, 7 aa, Homo sapiens
SSTRGYS

SEQ ID NO: 1080 - protein, 6 aa, Homo sapiens
STRGYS

SEQ ID NO: 1081 - protein, 9 aa, Homo sapiens
IFSYATKRQ

SEQ ID NO: 1082 - protein, 15 aa, Homo sapiens
IFSYATKRQDNEILI

SEQ ID NO: 1083 - protein, 13 aa, Homo sapiens
SYATKRQDNEILI

SEQ ID NO: 1084 - protein, 11 aa, Homo sapiens
YATKRQDNEIL

SEQ ID NO: 1085 - protein, 12 aa, Homo sapiens
YATKRQDNEILI

SEQ ID NO: 1086 - protein, 13 aa, Homo sapiens
YATKRQDNEILIF

SEQ ID NO: 1087 - protein, 10 aa, Homo sapiens
TKRQDNEILI

SEQ ID NO: 1088 - protein, 11 aa, Homo sapiens
TKRQDNEILIF

SEQ ID NO: 1089 - protein, 16 aa, Homo sapiens
TKRQDNEILIFWSKDI

SEQ ID NO: 1090 - protein, 9 aa, Homo sapiens
KRQDNEILI

SEQ ID NO: 1091 - protein, 10 aa, Homo sapiens
KRQDNEILIF

SEQ ID NO: 1092 - protein, 8 aa, Homo sapiens
WSKDIGYS

SEQ ID NO: 1093 - protein, 7 aa, Homo sapiens
SKDIGYS

SEQ ID NO: 1094 - protein, 12 aa, Homo sapiens
IVEFWVDGKPRV

SEQ ID NO: 1095 - protein, 9 aa, Homo sapiens
EFWVDGKPR

SEQ ID NO: 1096 - protein, 8 aa, Homo sapiens
WVDGKPRV

SEQ ID NO: 1097 - protein, 7 aa, Homo sapiens
VDGKPRV

SEQ ID NO: 1098 - protein, 11 aa, Homo sapiens
SLKKGYTVGAE

SEQ ID NO: 1099 - protein, 12 aa, Homo sapiens
SLKKGYTVGAEA

SEQ ID NO: 1100 - protein, 13 aa, Homo sapiens
SLKKGYTVGAEAS

SEQ ID NO: 1101 - protein, 7 aa, Homo sapiens
LKKGYTV

SEQ ID NO: 1102 - protein, 8 aa, Homo sapiens
LKKGYTVG

SEQ ID NO: 1103 - protein, 9 aa, Homo sapiens
LKKGYTVGA

SEQ ID NO: 1104 - protein, 10 aa, Homo sapiens
LKKGYTVGAE

SEQ ID NO: 1105 - protein, 11 aa, Homo sapiens
LKKGYTVGAEA

SEQ ID NO: 1106 - protein, 12 aa, Homo sapiens
LKKGYTVGAEAS

SEQ ID NO: 1107 - protein, 13 aa, Homo sapiens
LKKGYTVGAEASI

SEQ ID NO: 1108 - protein, 14 aa, Homo sapiens
SIILGQEQDSFGGN

SEQ ID NO: 1109 - protein, 19 aa, Homo sapiens
SIILGQEQDSFGGNFEGSQ

SEQ ID NO: 1110 - protein, 20 aa, Homo sapiens
SIILGQEQDSFGGNFEGSQS

SEQ ID NO: 1111 - protein, 17 aa, Homo sapiens
IILGQEQDSFGGNFEGS

SEQ ID NO: 1112 - protein, 19 aa, Homo sapiens
IILGQEQDSFGGNFEGSQS

SEQ ID NO: 1113 - protein, 12 aa, Homo sapiens
ILGQEQDSFGGN

SEQ ID NO: 1114 - protein, 17 aa, Homo sapiens
ILGQEQDSFGGNFEGSQ

SEQ ID NO: 1115 - protein, 18 aa, Homo sapiens
ILGQEQDSFGGNFEGSQS

SEQ ID NO: 1116 - protein, 16 aa, Homo sapiens
LGQEQDSFGGNFEGSQ

SEQ ID NO: 1117 - protein, 17 aa, Homo sapiens
LGQEQDSFGGNFEGSQS

SEQ ID NO: 1118 - protein, 16 aa, Homo sapiens
GQEQDSFGGNFEGSQS

SEQ ID NO: 1119 - protein, 11 aa, Homo sapiens
SFGGNFEGSQS

SEQ ID NO: 1120 - protein, 11 aa, Homo sapiens
QSLVGDIGNVN

SEQ ID NO: 1121 - protein, 14 aa, Homo sapiens
INTIYLGGPFSPNV

SEQ ID NO: 1122 - protein, 16 aa, Homo sapiens
INTIYLGGPFSPNVLN

SEQ ID NO: 1123 - protein, 13 aa, Homo sapiens
IYLGGPFSPNVLN

SEQ ID NO: 1124 - protein, 12 aa, Homo sapiens
YLGGPFSPNVLN

SEQ ID NO: 1125 - protein, 8 aa, Homo sapiens
LGGPFSPN

SEQ ID NO: 1126 - protein, 26 aa, Homo sapiens
SPNVLNWRALKYEVQGEVFTKPQLWP

SEQ ID NO: 1127 - protein, 5 aa, Homo sapiens
LNWRA

SEQ ID NO: 1128 - protein, 6 aa, Homo sapiens
LNWRAL

SEQ ID NO: 1129 - protein, 7 aa, Homo sapiens
LNWRALK

SEQ ID NO: 1130 - protein, 7 aa, Homo sapiens
WRALKYE

SEQ ID NO: 1131 - protein, 8 aa, Homo sapiens
WRALKYEV

SEQ ID NO: 1132 - protein, 11 aa, Homo sapiens
WRALKYEVQGE

SEQ ID NO: 1133 - protein, 6 aa, Homo sapiens
ALKYEV

SEQ ID NO: 1134 - protein, 6 aa, Homo sapiens
LKYEVQ

SEQ ID NO: 1135 - protein, 7 aa, Homo sapiens
LKYEVQG

SEQ ID NO: 1136 - protein, 8 aa, Homo sapiens
LKYEVQGE

SEQ ID NO: 1137 - protein, 13 aa, Homo sapiens
LKYEVQGEVFTKP

SEQ ID NO: 1138 - protein, 14 aa, Homo sapiens
LKYEVQGEVFTKPQ

SEQ ID NO: 1139 - protein, 17 aa, Homo sapiens
LKYEVQGEVFTKPQLWP

SEQ ID NO: 1140 - protein, 7 aa, Homo sapiens
KYEVQGE

SEQ ID NO: 1141 - protein, 13 aa, Homo sapiens
KYEVQGEVFTKPQ

SEQ ID NO: 1142 - protein, 16 aa, Homo sapiens
KYEVQGEVFTKPQLWP

SEQ ID NO: 1143 - protein, 11 aa, Homo sapiens
YEVQGEVFTKP

SEQ ID NO: 1144 - protein, 12 aa, Homo sapiens
YEVQGEVFTKPQ

SEQ ID NO: 1145 - protein, 15 aa, Homo sapiens
YEVQGEVFTKPQLWP

SEQ ID NO: 1146 - protein, 10 aa, Homo sapiens
VQGEVFTKPQ

SEQ ID NO: 1147 - protein, 13 aa, Homo sapiens
VQGEVFTKPQLWP

SEQ ID NO: 1148 - protein, 9 aa, Homo sapiens
QGEVFTKPQ

SEQ ID NO: 1149 - protein, 7 aa, Homo sapiens
GEVFTKP

SEQ ID NO: 1150 - protein, 8 aa, Homo sapiens
GEVFTKPQ

SEQ ID NO: 1151 - protein, 7 aa, Homo sapiens
EVFTKPQ

SEQ ID NO: 1152 - protein, 10 aa, Homo sapiens
EVFTKPQLWP

SEQ ID NO: 1153 - protein, 6 aa, Homo sapiens
VFTKPQ

SEQ ID NO: 1154 - protein, 5 aa, Homo sapiens
FTKPQ

SEQ ID NO: 1155 - protein, 8 aa, Homo sapiens
FTKPQLWP

SEQ ID NO: 1156 - protein, 7 aa, Homo sapiens
TKPQLWP

SEQ ID NO: 1157 - protein, 6 aa, Homo sapiens
KPQLWP

SEQ ID NO: 1158 - protein, 9 aa, Homo sapiens
MSRKAFVFP

SEQ ID NO: 1159 - protein, 11 aa, Homo sapiens
MSRKAFVFPKE

SEQ ID NO: 1160 - protein, 13 aa, Homo sapiens
MSRKAFVFPKESD

SEQ ID NO: 1161 - protein, 18 aa, Homo sapiens
MSRKAFVFPKESDTSYVS

SEQ ID NO: 1162 - protein, 8 aa, Homo sapiens
SRKAFVFP

SEQ ID NO: 1163 - protein, 12 aa, Homo sapiens
SRKAFVFPKESD

SEQ ID NO: 1164 - protein, 14 aa, Homo sapiens
SRKAFVFPKESDTS

SEQ ID NO: 1165 - protein, 7 aa, Homo sapiens
RKAFVFP

SEQ ID NO: 1166 - protein, 11 aa, Homo sapiens
RKAFVFPKESD

SEQ ID NO: 1167 - protein, 6 aa, Homo sapiens
KAFVFP

SEQ ID NO: 1168 - protein, 11 aa, Homo sapiens
AFVFPKESDTS

SEQ ID NO: 1169 - protein, 7 aa, Homo sapiens
VFPKESD

SEQ ID NO: 1170 - protein, 7 aa, Homo sapiens
KESDTSY

SEQ ID NO: 1171 - protein, 9 aa, Homo sapiens
KESDTSYVS

SEQ ID NO: 1172 - protein, 6 aa, Homo sapiens
VSLKAP

SEQ ID NO: 1173 - protein, 6 aa, Homo sapiens
LKAPLT

SEQ ID NO: 1174 - protein, 8 aa, Homo sapiens
LKAPLTKP

SEQ ID NO: 1175 - protein, 11 aa, Homo sapiens
YTELSSTRGYS

SEQ ID NO: 1176 - protein, 9 aa, Homo sapiens
YATKRQDNE

SEQ ID NO: 1177 - protein, 10 aa, Homo sapiens
YATKRQDNEI

SEQ ID NO: 1178 - protein, 9 aa, Homo sapiens
TKRQDNEIL

SEQ ID NO: 1179 - protein, 8 aa, Homo sapiens
KRQDNEIL

SEQ ID NO: 1180 - protein, 8 aa, Homo sapiens
ILIFWSKD

SEQ ID NO: 1181 - protein, 6 aa, Homo sapiens
IFWSKD

SEQ ID NO: 1182 - protein, 9 aa, Homo sapiens
WVDGKPRVR

SEQ ID NO: 1183 - protein, 16 aa, Homo sapiens
VRKSLKKGYTVGAEAS

SEQ ID NO: 1184 - protein, 7 aa, Homo sapiens
SLKKGYT

SEQ ID NO: 1185 - protein, 9 aa, Homo sapiens
SLKKGYTVG

SEQ ID NO: 1186 - protein, 10 aa, Homo sapiens
SLKKGYTVGA

SEQ ID NO: 1187 - protein, 14 aa, Homo sapiens
SLKKGYTVGAEASI

SEQ ID NO: 1188 - protein, 11 aa, Homo sapiens
KKGYTVGAEAS

SEQ ID NO: 1189 - protein, 10 aa, Homo sapiens
KGYTVGAEAS

SEQ ID NO: 1190 - protein, 11 aa, Homo sapiens
KGYTVGAEASI

SEQ ID NO: 1191 - protein, 8 aa, Homo sapiens
IILGQEQD

SEQ ID NO: 1192 - protein, 13 aa, Homo sapiens
IILGQEQDSFGGN

SEQ ID NO: 1193 - protein, 12 aa, Homo sapiens
LVGDIGNVNMWD

SEQ ID NO: 1194 - protein, 10 aa, Homo sapiens
IYLGGPFSPN

SEQ ID NO: 1195 - protein, 13 aa, Homo sapiens
IYLGGPFSPNVLN

SEQ ID NO: 1196 - protein, 11 aa, Homo sapiens
LGGPFSPNVLN

SEQ ID NO: 1197 - protein, 10 aa, Homo sapiens
EVQGEVFTKP

SEQ ID NO: 1198 - protein, 14 aa, Homo sapiens
EVQGEVFTKPQLWP

SEQ ID NO: 1199 - protein, 9 aa, Homo sapiens
VQGEVFTKP

SEQ ID NO: 1200 - protein, 11 aa, Homo sapiens
GEVFTKPQLWP

SEQ ID NO: 1201 - protein, 6 aa, Homo sapiens
EVFTKP

SEQ ID NO: 1202 - protein, 7 aa, Homo sapiens
VFTKPQL

SEQ ID NO: 1203 - protein, 9 aa, Homo sapiens
VFTKPQLWP

SEQ ID NO: 1204 - protein, 7 aa, Homo sapiens
KAFVFPK

SEQ ID NO: 1205 - protein, 6 aa, Homo sapiens
VRKSLK

SEQ ID NO: 1206 - protein, 17 aa, Homo sapiens
MSRKAFVFPKESDTSYV

SEQ ID NO: 1207 - protein, 17 aa, Homo sapiens
SRKAFVFPKESDTSYVS

SEQ ID NO: 1208 - protein, 16 aa, Homo sapiens
KAFVFPKESDTSYVSL

SEQ ID NO: 1209 - protein, 17 aa, Homo sapiens
KAFVFPKESDTSYVSLK

SEQ ID NO: 1210 - protein, 18 aa, Homo sapiens
AFVFPKESDTSYVSLKAP

SEQ ID NO: 1211 - protein, 15 aa, Homo sapiens
FVFPKESDTSYVSLK

SEQ ID NO: 1212 - protein, 14 aa, Homo sapiens
VFPKESDTSYVSLK

SEQ ID NO: 1213 - protein, 13 aa, Homo sapiens
KESDTSYVSLKAP

SEQ ID NO: 1214 - protein, 12 aa, Homo sapiens
TKRQDNEILIFW

SEQ ID NO: 1215 - protein, 15 aa, Homo sapiens
IVEFWVDGKPRVRKS

SEQ ID NO: 1216 - protein, 14 aa, Homo sapiens
LKKGYTVGAEASII

SEQ ID NO: 1217 - protein, 15 aa, Homo sapiens
QEQDSFGGNFEGSQS

SEQ ID NO: 1218 - protein, 10 aa, Homo sapiens
FVLSPDEINT

SEQ ID NO: 1219 - protein, 15 aa, Homo sapiens
SKDIGYSFTVGGSEI

SEQ ID NO: 1220 - protein, 12 aa, Homo sapiens
FGQTDMSRKAFV

SEQ ID NO: 1221 - protein, 10 aa, Homo sapiens
FPKESDTSYV

SEQ ID NO: 1222 - protein, 6 aa, Homo sapiens
SLKAPL

SEQ ID NO: 1223 - protein, 12 aa, Homo sapiens
SLKAPLTKPLKA

SEQ ID NO: 1224 - protein, 9 aa, Homo sapiens
RGYSIFSYA

SEQ ID NO: 1225 - protein, 14 aa, Homo sapiens
FSYATKRQDNEILI

SEQ ID NO: 1226 - protein, 11 aa, Homo sapiens
ATKRQDNEILI

SEQ ID NO: 1227 - protein, 9 aa, Homo sapiens
FWSKDIGYS

SEQ ID NO: 1228 - protein, 11 aa, Homo sapiens
FWSKDIGYSFT

SEQ ID NO: 1229 - protein, 12 aa, Homo sapiens
FWSKDIGYSFTV

SEQ ID NO: 1230 - protein, 11 aa, Homo sapiens
WSKDIGYSFTV

SEQ ID NO: 1231 - protein, 13 aa, Homo sapiens
KSLKKGYTVGAEA

SEQ ID NO: 1232 - protein, 10 aa, Homo sapiens
KKGYTVGAEA

SEQ ID NO: 1233 - protein, 11 aa, Homo sapiens
GAEASIILGQE

SEQ ID NO: 1234 - protein, 13 aa, Homo sapiens
GAEASIILGQEQD

SEQ ID NO: 1235 - protein, 9 aa, Homo sapiens
SIILGQEQD

SEQ ID NO: 1236 - protein, 18 aa, Homo sapiens
IILGQEQDSFGGNFEGSQ

SEQ ID NO: 1237 - protein, 16 aa, Homo sapiens
ILGQEQDSFGGNFEGS

SEQ ID NO: 1238 - protein, 11 aa, Homo sapiens
LGQEQDSFGGN

SEQ ID NO: 1239 - protein, 15 aa, Homo sapiens
LGQEQDSFGGNFEGS

SEQ ID NO: 1240 - protein, 18 aa, Homo sapiens
LGQEQDSFGGNFEGSQSL

SEQ ID NO: 1241 - protein, 19 aa, Homo sapiens
LGQEQDSFGGNFEGSQSLV

SEQ ID NO: 1242 - protein, 13 aa, Homo sapiens
QDSFGGNFEGSQS

SEQ ID NO: 1243 - protein, 10 aa, Homo sapiens
SFGGNFEGSQ

SEQ ID NO: 1244 - protein, 13 aa, Homo sapiens
SFGGNFEGSQSLV

SEQ ID NO: 1245 - protein, 11 aa, Homo sapiens
LVGDIGNVNMW

SEQ ID NO: 1246 - protein, 13 aa, Homo sapiens
INTIYLGGPFSPN

SEQ ID NO: 1247 - protein, 11 aa, Homo sapiens
TIYLGGPFSPN

SEQ ID NO: 1248 - protein, 13 aa, Homo sapiens
YLGGPFSPNVSEQ

SEQ ID NO: 1249 - protein, 6 aa, Homo sapiens
VLNWRA

SEQ ID NO: 1250 - protein, 7 aa, Homo sapiens
VLNWRAL

SEQ ID NO: 1251 - protein, 8 aa, Homo sapiens
VLNWRALK

SEQ ID NO: 1252 - protein, 10 aa, Homo sapiens
LNWRALKYEV

SEQ ID NO: 1253 - protein, 5 aa, Homo sapiens
NWRAL

SEQ ID NO: 1254 - protein, 7 aa, Homo sapiens
NWRALKY

SEQ ID NO: 1255 - protein, 9 aa, Homo sapiens
NWRALKYEV

SEQ ID NO: 1256 - protein, 10 aa, Homo sapiens
NWRALKYEVQ

SEQ ID NO: 1257 - protein, 9 aa, Homo sapiens
WRALKYEVQ

SEQ ID NO: 1258 - protein, 7 aa, Homo sapiens
RALKYEV

SEQ ID NO: 1259 - protein, 8 aa, Homo sapiens
RALKYEVQ

SEQ ID NO: 1260 - protein, 10 aa, Homo sapiens
RALKYEVQGE

SEQ ID NO: 1261 - protein, 15 aa, Homo sapiens
ALKYEVQGEVFTKPQ

SEQ ID NO: 1262 - protein, 11 aa, Homo sapiens
EVQGEVFTKPQ

SEQ ID NO: 1263 - protein, 10 aa, Homo sapiens
QGEVFTKPQL

SEQ ID NO: 1264 - protein, 12 aa, Homo sapiens
QGEVFTKPQLWP

SEQ ID NO: 1265 - protein, 10 aa, Homo sapiens
ESDTSYVSLK

SEQ ID NO: 1266 - protein, 14 aa, Homo sapiens
QEQDSFGGNFEGSQ

SEQ ID NO: 1267 - protein, 18 aa, Homo sapiens
QEQDSFGGNFEGSQSLVG

SEQ ID NO: 1268 - protein, 11 aa, Homo sapiens
GNFEGSQSLVG

SEQ ID NO: 1269 - protein, 9 aa, Homo sapiens
YEVQGEVFT

SEQ ID NO: 1270 - protein, 7 aa, Homo sapiens
EINTIYL

SEQ ID NO: 1271 - protein, 5 aa, Homo sapiens
KYEVQ

SEQ ID NO: 1272 - protein, 14 aa, Homo sapiens
ESDTSYVSLKAPLT

SEQ ID NO: 1273 - protein, 9 aa, Homo sapiens
SDTSYVSLK

SEQ ID NO: 1274 - protein, 8 aa, Homo sapiens
DTSYVSLK

SEQ ID NO: 1275 - protein, 8 aa, Homo sapiens
IFWSKDIG

SEQ ID NO: 1276 - protein, 8 aa, Homo sapiens
KGYTVGAE

SEQ ID NO: 1277 - protein, 15 aa, Homo sapiens
AEASIILGQEQDSFG

SEQ ID NO: 1278 - protein, 9 aa, Homo sapiens
LGQEQDSFG

SEQ ID NO: 1279 - protein, 13 aa, Homo sapiens
LGQEQDSFGGNFE

SEQ ID NO: 1280 - protein, 8 aa, Homo sapiens
GQEQDSFG

SEQ ID NO: 1281 - protein, 12 aa, Homo sapiens
GQEQDSFGGNFE

SEQ ID NO: 1282 - protein, 15 aa, Homo sapiens
GQEQDSFGGNFEGSQ

SEQ ID NO: 1283 - protein, 9 aa, Homo sapiens
QEQDSFGGN

SEQ ID NO: 1284 - protein, 11 aa, Homo sapiens
QEQDSFGGNFE

SEQ ID NO: 1285 - protein, 12 aa, Homo sapiens
QEQDSFGGNFEG

SEQ ID NO: 1286 - protein, 13 aa, Homo sapiens
QEQDSFGGNFEGS

SEQ ID NO: 1287 - protein, 10 aa, Homo sapiens
GNFEGSQSLV

SEQ ID NO: 1288 - protein, 14 aa, Homo sapiens
GNFEGSQSLVGDIG

SEQ ID NO: 1289 - protein, 10 aa, Homo sapiens
GSQSLVGDIG

SEQ ID NO: 1290 - protein, 13 aa, Homo sapiens
GSQSLVGDIGNVN

SEQ ID NO: 1291 - protein, 9 aa, Homo sapiens
VLSPDEINT

SEQ ID NO: 1292 - protein, 9 aa, Homo sapiens
GPFSPNVLN

SEQ ID NO: 1293 - protein, 8 aa, Homo sapiens
SPNVLNWR

SEQ ID NO: 1294 - protein, 6 aa, Homo sapiens
KYEVQG

SEQ ID NO: 1295 - protein, 11 aa, Homo sapiens
TSWESASGIVE

SEQ ID NO: 1296 - protein, 6 aa, Homo sapiens
KGYTVG

SEQ ID NO: 1297 - protein, 17 aa, Homo sapiens
QEQDSFGGNFEGSQSLV

SEQ ID NO: 1298 - protein, 14 aa, Homo sapiens
SFGGNFEGSQSLVG

SEQ ID NO: 1299 - protein, 10 aa, Homo sapiens
SPDEINTIYL

SEQ ID NO: 1300 - protein, 11 aa, Homo sapiens
SPDEINTIYLG

SEQ ID NO: 1301 - protein, 10 aa, Homo sapiens
GGPFSPNVLN

SEQ ID NO: 1302 - protein, 5 aa, Homo sapiens
ALKYE

SEQ ID NO: 1303 - protein, 7 aa, Homo sapiens
ALKYEVQ

SEQ ID NO: 1304 - protein, 8 aa, Homo sapiens
YEVQGEVF

SEQ ID NO: 1305 - protein, 6 aa, Homo sapiens
SFGGNF

SEQ ID NO: 1306 - protein, 6 aa, Homo sapiens
FGQTDM

SEQ ID NO: 1307 - protein, 6 aa, Homo sapiens
TDMSRK

SEQ ID NO: 1308 - protein, 6 aa, Homo sapiens
MSRKAF

SEQ ID NO: 1309 - protein, 6 aa, Homo sapiens
SRKAFV

SEQ ID NO: 1310 - protein, 6 aa, Homo sapiens
VFPKES

SEQ ID NO: 1311 - protein, 6 aa, Homo sapiens
FPKESD

SEQ ID NO: 1312 - protein, 6 aa, Homo sapiens
KESDTS

SEQ ID NO: 1313 - protein, 6 aa, Homo sapiens
LSSTRG

SEQ ID NO: 1314 - protein, 6 aa, Homo sapiens
SSTRGY

SEQ ID NO: 1315 - protein, 6 aa, Homo sapiens
KRQDNE

SEQ ID NO: 1316 - protein, 6 aa, Homo sapiens
WSKDIG

SEQ ID NO: 1317 - protein, 6 aa, Homo sapiens
SKDIGY

SEQ ID NO: 1318 - protein, 6 aa, Homo sapiens
SIILGQ

SEQ ID NO: 1319 - protein, 6 aa, Homo sapiens
IILGQE

SEQ ID NO: 1320 - protein, 6 aa, Homo sapiens
ILGQEQ

SEQ ID NO: 1321 - protein, 6 aa, Homo sapiens
IYLGGP

SEQ ID NO: 1322 - protein, 6 aa, Homo sapiens
YLGGPF

SEQ ID NO: 1323 - protein, 6 aa, Homo sapiens
LGGPFS

SEQ ID NO: 1324 - protein, 6 aa, Homo sapiens
VQGEVF

SEQ ID NO: 1325 - protein, 6 aa, Homo sapiens
YTELSS

SEQ ID NO: 1326 - protein, 6 aa, Homo sapiens
ILIFWS

SEQ ID NO: 1327 - protein, 6 aa, Homo sapiens
LVGDIG

SEQ ID NO: 1328 - protein, 6 aa, Homo sapiens
QEQDSF

SEQ ID NO: 1329 - protein, 6 aa, Homo sapiens
RGYSIF

SEQ ID NO: 1330 - protein, 6 aa, Homo sapiens
GAEASI

SEQ ID NO: 1331 - protein, 6 aa, Homo sapiens
QDSFGG

SEQ ID NO: 1332 - protein, 6 aa, Homo sapiens
TIYLGG

SEQ ID NO: 1333 - protein, 6 aa, Homo sapiens
EINTIY

SEQ ID NO: 1334 - protein, 6 aa, Homo sapiens
DTSYVS

SEQ ID NO: 1335 - protein, 6 aa, Homo sapiens
AEASII

SEQ ID NO: 1336 - protein, 6 aa, Homo sapiens
TSWESA

SEQ ID NO: 1337 - protein, 6 aa, Homo sapiens
SPDEIN

SEQ ID NO: 1338 - protein, 6 aa, Homo sapiens
GGPFSP

SEQ ID NO: 1339 - protein, 6 aa, Homo sapiens
YEVQGE

SEQ ID NO: 1340 - protein, 6 aa, Homo sapiens
FVLSPD

SEQ ID NO: 1341 - protein, 6 aa, Homo sapiens
LKKGYT

SEQ ID NO: 1342 - protein, 6 aa, Homo sapiens
RKAFVF

SEQ ID NO: 1343 - protein, 6 aa, Homo sapiens
IVEFWV

SEQ ID NO: 1344 - protein, 6 aa, Homo sapiens
ESDTSY

SEQ ID NO: 1345 - protein, 6 aa, Homo sapiens
TKPQLW

SEQ ID NO: 1346 - protein, 6 aa, Homo sapiens
EVQGEV

SEQ ID NO: 1347 - protein, 6 aa, Homo sapiens
SDTSYV

SEQ ID NO: 1348 - protein, 6 aa, Homo sapiens
IFSYAT

SEQ ID NO: 1349 - protein, 6 aa, Homo sapiens
SYATKR

SEQ ID NO: 1350 - protein, 6 aa, Homo sapiens
YATKRQ

SEQ ID NO: 1351 - protein, 6 aa, Homo sapiens
EFWVDG

SEQ ID NO: 1352 - protein, 6 aa, Homo sapiens
WVDGKP

SEQ ID NO: 1353 - protein, 6 aa, Homo sapiens
VDGKPR

SEQ ID NO: 1354 - protein, 6 aa, Homo sapiens
LGQEQD

SEQ ID NO: 1355 - protein, 6 aa, Homo sapiens
GQEQDS

SEQ ID NO: 1356 - protein, 6 aa, Homo sapiens
QSLVGD

SEQ ID NO: 1357 - protein, 6 aa, Homo sapiens
SPNVLN

SEQ ID NO: 1358 - protein, 6 aa, Homo sapiens
QGEVFT

SEQ ID NO: 1359 - protein, 6 aa, Homo sapiens
GEVFTK

SEQ ID NO: 1360 - protein, 6 aa, Homo sapiens
KKGYTV

SEQ ID NO: 1361 - protein, 6 aa, Homo sapiens
FSYATK

SEQ ID NO: 1362 - protein, 6 aa, Homo sapiens
ATKRQD

SEQ ID NO: 1363 - protein, 6 aa, Homo sapiens
FWSKDI

SEQ ID NO: 1364 - protein, 6 aa, Homo sapiens
NWRALK

SEQ ID NO: 1365 - protein, 6 aa, Homo sapiens
GSQSLV

SEQ ID NO: 1366 - protein, 6 aa, Homo sapiens
DFVLSP

SEQ ID NO: 1367 - protein, 6 aa, Homo sapiens
VLSPDE

SEQ ID NO: 1368 - protein, 6 aa, Homo sapiens
TKRQDN

SEQ ID NO: 1369 - protein, 6 aa, Homo sapiens
GNFEGS

SEQ ID NO: 1370 - protein, 6 aa, Homo sapiens
SLKKGY

SEQ ID NO: 1371 - protein, 6 aa, Homo sapiens
KSLKKG

SEQ ID NO: 1372 - protein, 6 aa, Homo sapiens
INTIYL

SEQ ID NO: 1373 - protein, 6 aa, Homo sapiens
RALKYE

SEQ ID NO: 1374 - protein, 6 aa, Homo sapiens
FYTELS

SEQ ID NO: 1375 - protein, 6 aa, Homo sapiens
WRALKY

SEQ ID NO: 1376 - protein, 6 aa, Homo sapiens
GPFSPN

SEQ ID NO: 1377 - protein, 6 aa, Homo sapiens
PDEINT

SEQ ID NO: 1378 - protein, 6 aa, Homo sapiens
DSFGGN

SEQ ID NO: 1379 - protein, 6 aa, Homo sapiens
LTKPLK

SEQ ID NO: 1380 - protein, 6 aa, Homo sapiens
KDIGYS

SEQ ID NO: 1381 - protein, 6 aa, Homo sapiens
DGKPRV

SEQ ID NO: 1382 - protein, 6 aa, Homo sapiens
NFEGSQ

SEQ ID NO: 1383 - protein, 6 aa, Homo sapiens
NVNMWD

SEQ ID NO: 1384 - protein, 6 aa, Homo sapiens
PRVRKS

SEQ ID NO: 1385 - protein, 6 aa, Homo sapiens
TVGSEI

SEQ ID NO: 1386 - protein, 6 aa, Homo sapiens
GYSFTV

SEQ ID NO: 1387 - protein, 6 aa, Homo sapiens
EGSQSL

SEQ ID NO: 1388 - protein, 6 aa, Homo sapiens
EQDSFG

SEQ ID NO: 1389 - protein, 6 aa, Homo sapiens
NVLNWR

SEQ ID NO: 1390 - protein, 6 aa, Homo sapiens
ASGIVE

SEQ ID NO: 1391 - protein, 6 aa, Homo sapiens
NTIYLG

SEQ ID NO: 1392 - protein, 6 aa, Homo sapiens
VGAEAS

SEQ ID NO: 1393 - protein, 6 aa, Homo sapiens
APLTKP

SEQ ID NO: 1394 - protein, 6 aa, Homo sapiens
QTDMSR

SEQ ID NO: 1395 - protein, 6 aa, Homo sapiens
PKESDT

SEQ ID NO: 1396 - protein, 6 aa, Homo sapiens
TSYVSL

SEQ ID NO: 1397 - protein, 6 aa, Homo sapiens
DNEILI

SEQ ID NO: 1398 - protein, 6 aa, Homo sapiens
QDNEIL

SEQ ID NO: 1399 - protein, 6 aa, Homo sapiens
NEILIF

SEQ ID NO: 1400 - protein, 6 aa, Homo sapiens
YTVGAE

SEQ ID NO: 1401 - protein, 6 aa, Homo sapiens
TVGAEA

SEQ ID NO: 1402 - protein, 6 aa, Homo sapiens
PFSPNV

SEQ ID NO: 1403 - protein, 6 aa, Homo sapiens
FEGSQS

SEQ ID NO: 1404 - protein, 6 aa, Homo sapiens
DIGNVN

SEQ ID NO: 1405 - protein, 6 aa, Homo sapiens
RQDNEI

SEQ ID NO: 1406 - protein, 6 aa, Homo sapiens
FTKPQL

SEQ ID NO: 1407 - protein, 6 aa, Homo sapiens
SYVSLK

SEQ ID NO: 1408 - protein, 6 aa, Homo sapiens
TKPLKA

SEQ ID NO: 1409 - protein, 6 aa, Homo sapiens
SIFSYA

SEQ ID NO: 1410 - protein, 6 aa, Homo sapiens
GNVNMW

SEQ ID NO: 1411 - protein, 6 aa, Homo sapiens
SQSLVG

SEQ ID NO: 1412 - protein, 6 aa, Homo sapiens
FGGNFE

SEQ ID NO: 1413 - protein, 6 aa, Homo sapiens
GGNFEG

SEQ ID NO: 1414 - protein, 6 aa, Homo sapiens
GKPRVR

SEQ ID NO: 1415 - protein, 6 aa, Homo sapiens
DMSRKA

SEQ ID NO: 1416 - protein, 6 aa, Homo sapiens
EILIFW

SEQ ID NO: 1417 - protein, 6 aa, Homo sapiens
IGYSFT

SEQ ID NO: 1418 - protein, 12 aa, Homo sapiens
GVPGAIPGGVPG

SEQ ID NO: 1419 - protein, 18 aa, Homo sapiens
AIPGGVPGGVFYPGAGLG

SEQ ID NO: 1420 - protein, 19 aa, Homo sapiens
AIPGGVPGGVFYPGAGLGA

SEQ ID NO: 1421 - protein, 15 aa, Homo sapiens
GVPGGVFYPGAGLGA

SEQ ID NO: 1422 - protein, 17 aa, Homo sapiens
GVPGGVFYPGAGLGALG

SEQ ID NO: 1423 - protein, 17 aa, Homo sapiens
VPGGVFYPGAGLGALGG

SEQ ID NO: 1424 - protein, 21 aa, Homo sapiens
GVFYPGAGLGALGGGALGPGG

SEQ ID NO: 1425 - protein, 9 aa, Homo sapiens
VFYPGAGLG

SEQ ID NO: 1426 - protein, 10 aa, Homo sapiens
VFYPGAGLGA

SEQ ID NO: 1427 - protein, 11 aa, Homo sapiens
VFYPGAGLGAL

SEQ ID NO: 1428 - protein, 12 aa, Homo sapiens
VFYPGAGLGALG

SEQ ID NO: 1429 - protein, 13 aa, Homo sapiens
VFYPGAGLGALGG

SEQ ID NO: 1430 - protein, 14 aa, Homo sapiens
VFYPGAGLGALGGG

SEQ ID NO: 1431 - protein, 16 aa, Homo sapiens
VFYPGAGLGALGGGAL

SEQ ID NO: 1432 - protein, 17 aa, Homo sapiens
VFYPGAGLGALGGGALG

SEQ ID NO: 1433 - protein, 19 aa, Homo sapiens
VFYPGAGLGALGGGALGPG

SEQ ID NO: 1434 - protein, 20 aa, Homo sapiens
VFYPGAGLGALGGGALGPGG

SEQ ID NO: 1435 - protein, 29 aa, Homo sapiens
VFYPGAGLGALGGGALGPGGKPLKPVPGG

SEQ ID NO: 1436 - protein, 22 aa, Homo sapiens
LGALGGGALGPGGKPLKPVPGG

SEQ ID NO: 1437 - protein, 20 aa, Homo sapiens
ALGGGALGPGGKPLKPVPGG

SEQ ID NO: 1438 - protein, 18 aa, Homo sapiens
LGGGALGPGGKPLKPVPG

SEQ ID NO: 1439 - protein, 19 aa, Homo sapiens
LGGGALGPGGKPLKPVPGG

SEQ ID NO: 1440 - protein, 17 aa, Homo sapiens
GGALGPGGKPLKPVPGG

SEQ ID NO: 1441 - protein, 14 aa, Homo sapiens
LGPGGKPLKPVPGG

SEQ ID NO: 1442 - protein, 13 aa, Homo sapiens
GPGGKPLKPVPGG

SEQ ID NO: 1443 - protein, 12 aa, Homo sapiens
PGGKPLKPVPGG

SEQ ID NO: 1444 - protein, 10 aa, Homo sapiens
GKPLKPVPGG

SEQ ID NO: 1445 - protein, 8 aa, Homo sapiens
PLKPVPGG

SEQ ID NO: 1446 - protein, 7 aa, Homo sapiens
LKPVPGG

SEQ ID NO: 1447 - protein, 15 aa, Homo sapiens
GLAGAGLGAGLGAFP

SEQ ID NO: 1448 - protein, 16 aa, Homo sapiens
GLAGAGLGAGLGAFPA

SEQ ID NO: 1449 - protein, 11 aa, Homo sapiens
LAGAGLGAGLG

SEQ ID NO: 1450 - protein, 14 aa, Homo sapiens
LAGAGLGAGLGAFP

SEQ ID NO: 1451 - protein, 15 aa, Homo sapiens
LAGAGLGAGLGAFPA

SEQ ID NO: 1452 - protein, 17 aa, Homo sapiens
LAGAGLGAGLGAFPAVT

SEQ ID NO: 1453 - protein, 20 aa, Homo sapiens
LAGAGLGAGLGAFPAVTFPG

SEQ ID NO: 1454 - protein, 21 aa, Homo sapiens
LAGAGLGAGLGAFPAVTFPGA

SEQ ID NO: 1455 - protein, 26 aa, Homo sapiens
LAGAGLGAGLGAFPAVTFPGALVPGG

SEQ ID NO: 1456 - protein, 28 aa, Homo sapiens
LAGAGLGAGLGAFPAVTFPGALVPGGVA

SEQ ID NO: 1457 - protein, 33 aa, Homo sapiens
LAGAGLGAGLGAFPAVTFPGALVPGGVADAAAA

SEQ ID NO: 1458 - protein, 25 aa, Homo sapiens
AGAGLGAGLGAFPAVTFPGALVPGG

SEQ ID NO: 1459 - protein, 13 aa, Homo sapiens
GAGLGAGLGAFPA

SEQ ID NO: 1460 - protein, 19 aa, Homo sapiens
GAGLGAGLGAFPAVTFPGA

SEQ ID NO: 1461 - protein, 12 aa, Homo sapiens
AGLGAGLGAFPA

SEQ ID NO: 1462 - protein, 11 aa, Homo sapiens
GLGAGLGAFPA

SEQ ID NO: 1463 - protein, 10 aa, Homo sapiens
LGAGLGAFPA

SEQ ID NO: 1464 - protein, 16 aa, Homo sapiens
LGAGLGAFPAVTFPGA

SEQ ID NO: 1465 - protein, 21 aa, Homo sapiens
LGAGLGAFPAVTFPGALVPGG

SEQ ID NO: 1466 - protein, 28 aa, Homo sapiens
LGAGLGAFPAVTFPGALVPGGVADAAAA

SEQ ID NO: 1467 - protein, 13 aa, Homo sapiens
AGLGAFPAVTFPG

SEQ ID NO: 1468 - protein, 12 aa, Homo sapiens
LGAFPAVTFPGA

SEQ ID NO: 1469 - protein, 19 aa, Homo sapiens
LGAFPAVTFPGALVPGGVA

SEQ ID NO: 1470 - protein, 24 aa, Homo sapiens
LGAFPAVTFPGALVPGGVADAAAA

SEQ ID NO: 1471 - protein, 15 aa, Homo sapiens
AFPAVTFPGALVPGG

SEQ ID NO: 1472 - protein, 12 aa, Homo sapiens
AVTFPGALVPGG

SEQ ID NO: 1473 - protein, 19 aa, Homo sapiens
AVTFPGALVPGGVADAAAA

SEQ ID NO: 1474 - protein, 11 aa, Homo sapiens
VTFPGALVPGG

SEQ ID NO: 1475 - protein, 18 aa, Homo sapiens
VTFPGALVPGGVADAAAA

SEQ ID NO: 1476 - protein, 12 aa, Homo sapiens
LVPGGVADAAAA

SEQ ID NO: 1477 - protein, 14 aa, Homo sapiens
LVPGGVADAAAAYK

SEQ ID NO: 1478 - protein, 9 aa, Homo sapiens
VADAAAAYK

SEQ ID NO: 1479 - protein, 7 aa, Homo sapiens
KAAKAGA

SEQ ID NO: 1480 - protein, 14 aa, Homo sapiens
LGVSAGAVVPQPGA

SEQ ID NO: 1481 - protein, 19 aa, Homo sapiens
VPGVGLPGVYPGGVLPGAR

SEQ ID NO: 1482 - protein, 18 aa, Homo sapiens
PGVGLPGVYPGGVLPGAR

SEQ ID NO: 1483 - protein, 15 aa, Homo sapiens
GLPGVYPGGVLPGAR

SEQ ID NO: 1484 - protein, 13 aa, Homo sapiens
PGVYPGGVLPGAR

SEQ ID NO: 1485 - protein, 7 aa, Homo sapiens
ARFPGVG

SEQ ID NO: 1486 - protein, 11 aa, Homo sapiens
ARFPGVGVLPG

SEQ ID NO: 1487 - protein, 16 aa, Homo sapiens
RFPGVGVLPGVPTGAG

SEQ ID NO: 1488 - protein, 13 aa, Homo sapiens
FPGVGVLPGVPTG

SEQ ID NO: 1489 - protein, 14 aa, Homo sapiens
FPGVGVLPGVPTGA

SEQ ID NO: 1490 - protein, 16 aa, Homo sapiens
FPGVGVLPGVPTGAGV

SEQ ID NO: 1491 - protein, 19 aa, Homo sapiens
FPGVGVLPGVPTGAGVKPK

SEQ ID NO: 1492 - protein, 7 aa, Homo sapiens
KPKAPGV

SEQ ID NO: 1493 - protein, 6 aa, Homo sapiens
PKAPGV

SEQ ID NO: 1494 - protein, 13 aa, Homo sapiens
GAFAGIPGVGPFG

SEQ ID NO: 1495 - protein, 16 aa, Homo sapiens
VGPFGGPQPGVPLGYP

SEQ ID NO: 1496 - protein, 11 aa, Homo sapiens
GPQPGVPLGYP

SEQ ID NO: 1497 - protein, 10 aa, Homo sapiens
PQPGVPLGYP

SEQ ID NO: 1498 - protein, 8 aa, Homo sapiens
PGVPLGYP

SEQ ID NO: 1499 - protein, 8 aa, Homo sapiens
GYPIKAPK

SEQ ID NO: 1500 - protein, 7 aa, Homo sapiens
PKLPGGY

SEQ ID NO: 1501 - protein, 13 aa, Homo sapiens
YTTGKLPYGYGPG

SEQ ID NO: 1502 - protein, 21 aa, Homo sapiens
YTTGKLPYGYGPGGVAGAAGK

SEQ ID NO: 1503 - protein, 10 aa, Homo sapiens
TTGKLPYGYG

SEQ ID NO: 1504 - protein, 20 aa, Homo sapiens
TTGKLPYGYGPGGVAGAAGK

SEQ ID NO: 1505 - protein, 16 aa, Homo sapiens
LPYGYGPGGVAGAAGK

SEQ ID NO: 1506 - protein, 13 aa, Homo sapiens
GYGPGGVAGAAGK

SEQ ID NO: 1507 - protein, 12 aa, Homo sapiens
YGPGGVAGAAGK

SEQ ID NO: 1508 - protein, 20 aa, Homo sapiens
AGYPTGTGVGPQAAAAAAAK

SEQ ID NO: 1509 - protein, 14 aa, Homo sapiens
TGVGPQAAAAAAAK

SEQ ID NO: 1510 - protein, 10 aa, Homo sapiens
PQAAAAAAAK

SEQ ID NO: 1511 - protein, 29 aa, Homo sapiens
FGAGAAGVLPGVGGAGVPGVPGAIPGIGG

SEQ ID NO: 1512 - protein, 38 aa, Homo sapiens
FGAGAAGVLPGVGGAGVPGVPGAIPGIGGIAGVGTPAA

SEQ ID NO: 1513 - protein, 16 aa, Homo sapiens
GVLPGVGGAGVPGVPG

SEQ ID NO: 1514 - protein, 22 aa, Homo sapiens
VLPGVGGAGVPGVPGAIPGIGG

SEQ ID NO: 1515 - protein, 30 aa, Homo sapiens
VLPGVGGAGVPGVPGAIPGIGGIAGVGTPA

SEQ ID NO: 1516 - protein, 31 aa, Homo sapiens
VLPGVGGAGVPGVPGAIPGIGGIAGVGTPAA

SEQ ID NO: 1517 - protein, 13 aa, Homo sapiens
GAGVPGVPGAIPG

SEQ ID NO: 1518 - protein, 14 aa, Homo sapiens
AGVPGVPGAIPGIG

SEQ ID NO: 1519 - protein, 14 aa, Homo sapiens
AGVPGVPGAIPGIG

SEQ ID NO: 1520 - protein, 15 aa, Homo sapiens
AGVPGVPGAIPGIGG

SEQ ID NO: 1521 - protein, 18 aa, Homo sapiens
AGVPGVPGAIPGIGGIAG

SEQ ID NO: 1522 - protein, 23 aa, Homo sapiens
AGVPGVPGAIPGIGGIAGVGTPA

SEQ ID NO: 1523 - protein, 14 aa, Homo sapiens
GVPGVPGAIPGIGG

SEQ ID NO: 1524 - protein, 16 aa, Homo sapiens
GVPGVPGAIPGIGGIA

SEQ ID NO: 1525 - protein, 19 aa, Homo sapiens
GVPGVPGAIPGIGGIAGVG

SEQ ID NO: 1526 - protein, 13 aa, Homo sapiens
VPGVPGAIPGIGG

SEQ ID NO: 1527 - protein, 19 aa, Homo sapiens
GVPGAIPGIGGIAGVGTPA

SEQ ID NO: 1528 - protein, 15 aa, Homo sapiens
VPGAIPGIGGIAGVG

SEQ ID NO: 1529 - protein, 18 aa, Homo sapiens
VPGAIPGIGGIAGVGTPA

SEQ ID NO: 1530 - protein, 20 aa, Homo sapiens
VPGAIPGIGGIAGVGTPAAA

SEQ ID NO: 1531 - protein, 28 aa, Homo sapiens
VPGAIPGIGGIAGVGTPAAAAAAAAAAK

SEQ ID NO: 1532 - protein, 12 aa, Homo sapiens
AIPGIGGIAGVG

SEQ ID NO: 1533 - protein, 15 aa, Homo sapiens
AIPGIGGIAGVGTPA

SEQ ID NO: 1534 - protein, 16 aa, Homo sapiens
AIPGIGGIAGVGTPAA

SEQ ID NO: 1535 - protein, 17 aa, Homo sapiens
AIPGIGGIAGVGTPAAA

SEQ ID NO: 1536 - protein, 20 aa, Homo sapiens
AIPGIGGIAGVGTPAAAAAA

SEQ ID NO: 1537 - protein, 25 aa, Homo sapiens
AIPGIGGIAGVGTPAAAAAAAAAAK

SEQ ID NO: 1538 - protein, 16 aa, Homo sapiens
IPGIGGIAGVGTPAAA

SEQ ID NO: 1539 - protein, 14 aa, Homo sapiens
IGGIAGVGTPAAAA

SEQ ID NO: 1540 - protein, 12 aa, Homo sapiens
GIAGVGTPAAAA

SEQ ID NO: 1541 - protein, 16 aa, Homo sapiens
GIAGVGTPAAAAAAAA

SEQ ID NO: 1542 - protein, 19 aa, Homo sapiens
GIAGVGTPAAAAAAAAAAK

SEQ ID NO: 1543 - protein, 15 aa, Homo sapiens
IAGVGTPAAAAAAAA

SEQ ID NO: 1544 - protein, 16 aa, Homo sapiens
IAGVGTPAAAAAAAAA

SEQ ID NO: 1545 - protein, 18 aa, Homo sapiens
IAGVGTPAAAAAAAAAAK

SEQ ID NO: 1546 - protein, 13 aa, Homo sapiens
TPAAAAAAAAAAK

SEQ ID NO: 1547 - protein, 12 aa, Homo sapiens
PAAAAAAAAAAK

SEQ ID NO: 1548 - protein, 11 aa, Homo sapiens
AAAAAAAAAAK

SEQ ID NO: 1549 - protein, 10 aa, Homo sapiens
AAAAAAAAAK

SEQ ID NO: 1550 - protein, 9 aa, Homo sapiens
AAAAAAAAK

SEQ ID NO: 1551 - protein, 10 aa, Homo sapiens
AAAAAAAAKA

SEQ ID NO: 1552 - protein, 8 aa, Homo sapiens
AAAAAAAK

SEQ ID NO: 1553 - protein, 18 aa, Homo sapiens
LVPGGPGFGPGVVGVPGA

SEQ ID NO: 1554 - protein, 13 aa, Homo sapiens
GPGFGPGVVGVPG

SEQ ID NO: 1555 - protein, 20 aa, Homo sapiens
GPGFGPGVVGVPGAGVPGVG

SEQ ID NO: 1556 - protein, 31 aa, Homo sapiens
GPGFGPGVVGVPGAGVPGVGVPGAGIPVVPG

SEQ ID NO: 1557 - protein, 12 aa, Homo sapiens
PGFGPGVVGVPG

SEQ ID NO: 1558 - protein, 13 aa, Homo sapiens
PGFGPGVVGVPGA

SEQ ID NO: 1559 - protein, 14 aa, Homo sapiens
PGFGPGVVGVPGAG

SEQ ID NO: 1560 - protein, 13 aa, Homo sapiens
PGVVGVPGAGVPG

SEQ ID NO: 1561 - protein, 18 aa, Homo sapiens
PGVVGVPGAGVPGVGVPG

SEQ ID NO: 1562 - protein, 27 aa, Homo sapiens
PGVVGVPGAGVPGVGVPGAGIPVVPGA

SEQ ID NO: 1563 - protein, 17 aa, Homo sapiens
VVGVPGAGVPGVGVPGA

SEQ ID NO: 1564 - protein, 39 aa, Homo sapiens
VGVPGAGVPGVGVPGAGIPVVPGAGIPGAAVPGVVSPEA

SEQ ID NO: 1565 - protein, 18 aa, Homo sapiens
AGVPGVGVPGAGIPVVPG

SEQ ID NO: 1566 - protein, 17 aa, Homo sapiens
GVPGVGVPGAGIPVVPG

SEQ ID NO: 1567 - protein, 18 aa, Homo sapiens
GVPGVGVPGAGIPVVPGA

SEQ ID NO: 1568 - protein, 16 aa, Homo sapiens
VPGVGVPGAGIPVVPG

SEQ ID NO: 1569 - protein, 13 aa, Homo sapiens
VGVPGAGIPVVPG

SEQ ID NO: 1570 - protein, 18 aa, Homo sapiens
VGVPGAGIPVVPGAGIPG

SEQ ID NO: 1571 - protein, 11 aa, Homo sapiens
VPGAGIPVVPG

SEQ ID NO: 1572 - protein, 13 aa, Homo sapiens
AGIPVVPGAGIPG

SEQ ID NO: 1573 - protein, 27 aa, Homo sapiens
AGIPVVPGAGIPGAAVPGVVSPEAAAK

SEQ ID NO: 1574 - protein, 12 aa, Homo sapiens
GIPVVPGAGIPG

SEQ ID NO: 1575 - protein, 17 aa, Homo sapiens
IPGAAVPGVVSPEAAAK

SEQ ID NO: 1576 - protein, 15 aa, Homo sapiens
GAAVPGVVSPEAAAK

SEQ ID NO: 1577 - protein, 13 aa, Homo sapiens
AVPGVVSPEAAAK

SEQ ID NO: 1578 - protein, 12 aa, Homo sapiens
VPGVVSPEAAAK

SEQ ID NO: 1579 - protein, 8 aa, Homo sapiens
YGARPGVG

SEQ ID NO: 1580 - protein, 10 aa, Homo sapiens
YGARPGVGVG

SEQ ID NO: 1581 - protein, 14 aa, Homo sapiens
YGARPGVGVGGIPT

SEQ ID NO: 1582 - protein, 15 aa, Homo sapiens
YGARPGVGVGGIPTY

SEQ ID NO: 1583 - protein, 16 aa, Homo sapiens
YGARPGVGVGGIPTYG

SEQ ID NO: 1584 - protein, 18 aa, Homo sapiens
YGARPGVGVGGIPTYGVG

SEQ ID NO: 1585 - protein, 19 aa, Homo sapiens
YGARPGVGVGGIPTYGVGA

SEQ ID NO: 1586 - protein, 20 aa, Homo sapiens
YGARPGVGVGGIPTYGVGAG

SEQ ID NO: 1587 - protein, 8 aa, Homo sapiens
GARPGVGV

SEQ ID NO: 1588 - protein, 10 aa, Homo sapiens
GARPGVGVGG

SEQ ID NO: 1589 - protein, 12 aa, Homo sapiens
GARPGVGVGGIP

SEQ ID NO: 1590 - protein, 14 aa, Homo sapiens
GARPGVGVGGIPTY

SEQ ID NO: 1591 - protein, 16 aa, Homo sapiens
GARPGVGVGGIPTYGV

SEQ ID NO: 1592 - protein, 17 aa, Homo sapiens
GARPGVGVGGIPTYGVG

SEQ ID NO: 1593 - protein, 21 aa, Homo sapiens
GARPGVGVGGIPTYGVGAGGF

SEQ ID NO: 1594 - protein, 24 aa, Homo sapiens
GARPGVGVGGIPTYGVGAGGFPGF

SEQ ID NO: 1595 - protein, 25 aa, Homo sapiens
GARPGVGVGGIPTYGVGAGGFPGFG

SEQ ID NO: 1596 - protein, 29 aa, Homo sapiens
GARPGVGVGGIPTYGVGAGGFPGFGVGVG

SEQ ID NO: 1597 - protein, 9 aa, Homo sapiens
ARPGVGVGG

SEQ ID NO: 1598 - protein, 11 aa, Homo sapiens
ARPGVGVGGIP

SEQ ID NO: 1599 - protein, 13 aa, Homo sapiens
ARPGVGVGGIPTY

SEQ ID NO: 1600 - protein, 17 aa, Homo sapiens
ARPGVGVGGIPTYGVGA

SEQ ID NO: 1601 - protein, 19 aa, Homo sapiens
ARPGVGVGGIPTYGVGAGG

SEQ ID NO: 1602 - protein, 22 aa, Homo sapiens
ARPGVGVGGIPTYGVGAGGFPG

SEQ ID NO: 1603 - protein, 23 aa, Homo sapiens
ARPGVGVGGIPTYGVGAGGFPGF

SEQ ID NO: 1604 - protein, 7 aa, Homo sapiens
RPGVGVG

SEQ ID NO: 1605 - protein, 8 aa, Homo sapiens
RPGVGVGG

SEQ ID NO: 1606 - protein, 11 aa, Homo sapiens
PGVGVGGIPTY

SEQ ID NO: 1607 - protein, 12 aa, Homo sapiens
PGVGVGGIPTYG

SEQ ID NO: 1608 - protein, 16 aa, Homo sapiens
PGVGVGGIPTYGVGAG

SEQ ID NO: 1609 - protein, 12 aa, Homo sapiens
VGGIPTYGVGAG

SEQ ID NO: 1610 - protein, 21 aa, Homo sapiens
GVGAGGFPGFGVGVGGIPGVA

SEQ ID NO: 1611 - protein, 14 aa, Homo sapiens
VGAGGFPGFGVGVG

SEQ ID NO: 1612 - protein, 33 aa, Homo sapiens
VGVGGIPGVAGVPSVGGVPGVGGVPGVGISPEA

SEQ ID NO: 1613 - protein, 18 aa, Homo sapiens
VAGVPSVGGVPGVGGVPG

SEQ ID NO: 1614 - protein, 25 aa, Homo sapiens
VAGVPSVGGVPGVGGVPGVGISPEA

SEQ ID NO: 1615 - protein, 20 aa, Homo sapiens
SVGGVPGVGGVPGVGISPEA

SEQ ID NO: 1616 - protein, 19 aa, Homo sapiens
VGGVPGVGGVPGVGISPEA

SEQ ID NO: 1617 - protein, 14 aa, Homo sapiens
GVPGVGGVPGVGIS

SEQ ID NO: 1618 - protein, 17 aa, Homo sapiens
GVPGVGGVPGVGISPEA

SEQ ID NO: 1619 - protein, 19 aa, Homo sapiens
GVPGVGGVPGVGISPEAQA

SEQ ID NO: 1620 - protein, 18 aa, Homo sapiens
GVPGVGISPEAQAAAAAK

SEQ ID NO: 1621 - protein, 11 aa, Homo sapiens
GVGTPAAAAAK

SEQ ID NO: 1622 - protein, 8 aa, Homo sapiens
TPAAAAAK

SEQ ID NO: 1623 - protein, 14 aa, Homo sapiens
FGLVPGVGVAPGVG

SEQ ID NO: 1624 - protein, 18 aa, Homo sapiens
FGLVPGVGVAPGVGVAPG

SEQ ID NO: 1625 - protein, 24 aa, Homo sapiens
FGLVPGVGVAPGVGVAPGVGVAPG

SEQ ID NO: 1626 - protein, 26 aa, Homo sapiens
FGLVPGVGVAPGVGVAPGVGVAPGVG

SEQ ID NO: 1627 - protein, 30 aa, Homo sapiens
FGLVPGVGVAPGVGVAPGVGVAPGVGLAPG

SEQ ID NO: 1628 - protein, 36 aa, Homo sapiens
FGLVPGVGVAPGVGVAPGVGVAPGVGLAPGVGVAPG

SEQ ID NO: 1629 - protein, 37 aa, Homo sapiens
FGLVPGVGVAPGVGVAPGVGVAPGVGLAPGVGVAPGV

SEQ ID NO: 1630 - protein, 42 aa, Homo sapiens
FGLVPGVGVAPGVGVAPGVGVAPGVGLAPGVGVAPGVGVAPG

SEQ ID NO: 1631 - protein, 11 aa, Homo sapiens
GLVPGVGVAPG

SEQ ID NO: 1632 - protein, 12 aa, Homo sapiens
GLVPGVGVAPGV

SEQ ID NO: 1633 - protein, 15 aa, Homo sapiens
GLVPGVGVAPGVGVA

SEQ ID NO: 1634 - protein, 16 aa, Homo sapiens
GLVPGVGVAPGVGVAP

SEQ ID NO: 1635 - protein, 17 aa, Homo sapiens
GLVPGVGVAPGVGVAPG

SEQ ID NO: 1636 - protein, 19 aa, Homo sapiens
GLVPGVGVAPGVGVAPGVG

SEQ ID NO: 1637 - protein, 23 aa, Homo sapiens
GLVPGVGVAPGVGVAPGVGVAPG

SEQ ID NO: 1638 - protein, 26 aa, Homo sapiens
GLVPGVGVAPGVGVAPGVGVAPGVGL

SEQ ID NO: 1639 - protein, 27 aa, Homo sapiens
GLVPGVGVAPGVGVAPGVGVAPGVGLA

SEQ ID NO: 1640 - protein, 29 aa, Homo sapiens
GLVPGVGVAPGVGVAPGVGVAPGVGLAPG

SEQ ID NO: 1641 - protein, 31 aa, Homo sapiens
GLVPGVGVAPGVGVAPGVGVAPGVGLAPGVG

SEQ ID NO: 1642 - protein, 33 aa, Homo sapiens
GLVPGVGVAPGVGVAPGVGVAPGVGLAPGVGVA

SEQ ID NO: 1643 - protein, 35 aa, Homo sapiens
GLVPGVGVAPGVGVAPGVGVAPGVGLAPGVGVAPG

SEQ ID NO: 1644 - protein, 12 aa, Homo sapiens
LVPGVGVAPGVG

SEQ ID NO: 1645 - protein, 16 aa, Homo sapiens
LVPGVGVAPGVGVAPG

SEQ ID NO: 1646 - protein, 18 aa, Homo sapiens
LVPGVGVAPGVGVAPGVG

SEQ ID NO: 1647 - protein, 24 aa, Homo sapiens
LVPGVGVAPGVGVAPGVGVAPGVG

SEQ ID NO: 1648 - protein, 36 aa, Homo sapiens
LVPGVGVAPGVGVAPGVGVAPGVGLAPGVGVAPGVG

SEQ ID NO: 1649 - protein, 14 aa, Homo sapiens
PGVGVAPGVGVAPG

SEQ ID NO: 1650 - protein, 15 aa, Homo sapiens
VGVAPGVGVAPGVGV

SEQ ID NO: 1651 - protein, 20 aa, Homo sapiens
VGVAPGVGVAPGVGVAPGVG

SEQ ID NO: 1652 - protein, 30 aa, Homo sapiens
VGVAPGVGVAPGVGVAPGVGLAPGVGVAPG

SEQ ID NO: 1653 - protein, 16 aa, Homo sapiens
VAPGVGVAPGVGVAPG

SEQ ID NO: 1654 - protein, 18 aa, Homo sapiens
VAPGVGVAPGVGVAPGVG

SEQ ID NO: 1655 - protein, 24 aa, Homo sapiens
VAPGVGVAPGVGVAPGVGLAPGVG

SEQ ID NO: 1656 - protein, 28 aa, Homo sapiens
VAPGVGVAPGVGVAPGVGLAPGVGVAPG

SEQ ID NO: 1657 - protein, 16 aa, Homo sapiens
VGVAPGVGVAPGVGLA

SEQ ID NO: 1658 - protein, 24 aa, Homo sapiens
VGVAPGVGVAPGVGLAPGVGVAPG

SEQ ID NO: 1659 - protein, 41 aa, Homo sapiens
VGVAPGVGVAPGVGLAPGVGVAPGVGVAPGVGVAPGIGPGG

SEQ ID NO: 1660 - protein, 24 aa, Homo sapiens
VAPGVGVAPGVGLAPGVGVAPGVG

SEQ ID NO: 1661 - protein, 26 aa, Homo sapiens
VAPGVGVAPGVGLAPGVGVAPGVGVA

SEQ ID NO: 1662 - protein, 28 aa, Homo sapiens
VAPGVGVAPGVGLAPGVGVAPGVGVAPG

SEQ ID NO: 1663 - protein, 37 aa, Homo sapiens
VAPGVGVAPGVGLAPGVGVAPGVGVAPGVGVAPGIGP

SEQ ID NO: 1664 - protein, 39 aa, Homo sapiens
VAPGVGVAPGVGLAPGVGVAPGVGVAPGVGVAPGIGPGG

SEQ ID NO: 1665 - protein, 14 aa, Homo sapiens
PGVGVAPGVGLAPG

SEQ ID NO: 1666 - protein, 19 aa, Homo sapiens
PGVGVAPGVGLAPGVGVAP

SEQ ID NO: 1667 - protein, 22 aa, Homo sapiens
PGVGVAPGVGLAPGVGVAPGVG

SEQ ID NO: 1668 - protein, 16 aa, Homo sapiens
VGVAPGVGLAPGVGVA

SEQ ID NO: 1669 - protein, 17 aa, Homo sapiens
VGVAPGVGLAPGVGVAP

SEQ ID NO: 1670 - protein, 24 aa, Homo sapiens
VGVAPGVGLAPGVGVAPGVGVAPG

SEQ ID NO: 1671 - protein, 26 aa, Homo sapiens
VGVAPGVGLAPGVGVAPGVGVAPGVG

SEQ ID NO: 1672 - protein, 30 aa, Homo sapiens
VGVAPGVGLAPGVGVAPGVGVAPGVGVAPG

SEQ ID NO: 1673 - protein, 35 aa, Homo sapiens
VGVAPGVGLAPGVGVAPGVGVAPGVGVAPGIGPGG

SEQ ID NO: 1674 - protein, 34 aa, Homo sapiens
GVAPGVGLAPGVGVAPGVGVAPGVGVAPGIGPGG

SEQ ID NO: 1675 - protein, 14 aa, Homo sapiens
VAPGVGLAPGVGVA

SEQ ID NO: 1676 - protein, 16 aa, Homo sapiens
VAPGVGLAPGVGVAPG

SEQ ID NO: 1677 - protein, 18 aa, Homo sapiens
VAPGVGLAPGVGVAPGVG

SEQ ID NO: 1678 - protein, 20 aa, Homo sapiens
VAPGVGLAPGVGVAPGVGVA

SEQ ID NO: 1679 - protein, 22 aa, Homo sapiens
VAPGVGLAPGVGVAPGVGVAPG

SEQ ID NO: 1680 - protein, 26 aa, Homo sapiens
VAPGVGLAPGVGVAPGVGVAPGVGVA

SEQ ID NO: 1681 - protein, 33 aa, Homo sapiens
VAPGVGLAPGVGVAPGVGVAPGVGVAPGIGPGG

SEQ ID NO: 1682 - protein, 14 aa, Homo sapiens
PGVGLAPGVGVAPG

SEQ ID NO: 1683 - protein, 19 aa, Homo sapiens
GVGLAPGVGVAPGVGVAPG

SEQ ID NO: 1684 - protein, 14 aa, Homo sapiens
VGLAPGVGVAPGVG

SEQ ID NO: 1685 - protein, 18 aa, Homo sapiens
VGLAPGVGVAPGVGVAPG

SEQ ID NO: 1686 - protein, 26 aa, Homo sapiens
VGLAPGVGVAPGVGVAPGVGVAPGIG

SEQ ID NO: 1687 - protein, 29 aa, Homo sapiens
VGLAPGVGVAPGVGVAPGVGVAPGIGPGG

SEQ ID NO: 1688 - protein, 28 aa, Homo sapiens
VGLAPGVGVAPGVGVAPGVGVAPGIGPG

SEQ ID NO: 1689 - protein, 33 aa, Homo sapiens
VGLAPGVGVAPGVGVAPGVGVAPGIGPGGVAAA

SEQ ID NO: 1690 - protein, 18 aa, Homo sapiens
LAPGVGVAPGVGVAPGVG

SEQ ID NO: 1691 - protein, 20 aa, Homo sapiens
LAPGVGVAPGVGVAPGVGVA

SEQ ID NO: 1692 - protein, 25 aa, Homo sapiens
LAPGVGVAPGVGVAPGVGVAPGIGP

SEQ ID NO: 1693 - protein, 27 aa, Homo sapiens
LAPGVGVAPGVGVAPGVGVAPGIGPGG

SEQ ID NO: 1694 - protein, 24 aa, Homo sapiens
GVGVAPGVGVAPGVGVAPGIGPGG

SEQ ID NO: 1695 - protein, 16 aa, Homo sapiens
VGVAPGVGVAPGVGVA

SEQ ID NO: 1696 - protein, 18 aa, Homo sapiens
VGVAPGVGVAPGVGVAPG

SEQ ID NO: 1697 - protein, 22 aa, Homo sapiens
VGVAPGVGVAPGVGVAPGIGPG

SEQ ID NO: 1698 - protein, 23 aa, Homo sapiens
VGVAPGVGVAPGVGVAPGIGPGG

SEQ ID NO: 1699 - protein, 27 aa, Homo sapiens
VGVAPGVGVAPGVGVAPGIGPGGVAAA

SEQ ID NO: 1700 - protein, 15 aa, Homo sapiens
VAPGVGVAPGVGVAP

SEQ ID NO: 1701 - protein, 18 aa, Homo sapiens
VAPGVGVAPGVGVAPGIG

SEQ ID NO: 1702 - protein, 21 aa, Homo sapiens
VAPGVGVAPGVGVAPGIGPGG

SEQ ID NO: 1703 - protein, 18 aa, Homo sapiens
PGVGVAPGVGVAPGIGPG

SEQ ID NO: 1704 - protein, 19 aa, Homo sapiens
PGVGVAPGVGVAPGIGPGG

SEQ ID NO: 1705 - protein, 17 aa, Homo sapiens
VGVAPGVGVAPGIGPGG

SEQ ID NO: 1706 - protein, 20 aa, Homo sapiens
VGVAPGVGVAPGIGPGGVAA

SEQ ID NO: 1707 - protein, 14 aa, Homo sapiens
VAPGVGVAPGIGPG

SEQ ID NO: 1708 - protein, 12 aa, Homo sapiens
PGVGVAPGIGPG

SEQ ID NO: 1709 - protein, 14 aa, Homo sapiens
VGVAPGIGPGGVAA

SEQ ID NO: 1710 - protein, 9 aa, Homo sapiens
PGGVAAAAK

SEQ ID NO: 1711 - protein, 7 aa, Homo sapiens
LRAAAGL

SEQ ID NO: 1712 - protein, 8 aa, Homo sapiens
LRAAAGLG

SEQ ID NO: 1713 - protein, 9 aa, Homo sapiens
LRAAAGLGA

SEQ ID NO: 1714 - protein, 15 aa, Homo sapiens
AAAGLGAGIPGLGVG

SEQ ID NO: 1715 - protein, 17 aa, Homo sapiens
AAAGLGAGIPGLGVGVG

SEQ ID NO: 1716 - protein, 11 aa, Homo sapiens
LGAGIPGLGVG

SEQ ID NO: 1717 - protein, 13 aa, Homo sapiens
LGAGIPGLGVGVG

SEQ ID NO: 1718 - protein, 20 aa, Homo sapiens
LGAGIPGLGVGVGVPGLGVG

SEQ ID NO: 1719 - protein, 16 aa, Homo sapiens
LGAGIPGLGVGVGVPG

SEQ ID NO: 1720 - protein, 21 aa, Homo sapiens
LGAGIPGLGVGVGVPGLGVGA

SEQ ID NO: 1721 - protein, 17 aa, Homo sapiens
LGAGIPGLGVGVGVPGL

SEQ ID NO: 1722 - protein, 18 aa, Homo sapiens
LGAGIPGLGVGVGVPGLG

SEQ ID NO: 1723 - protein, 25 aa, Homo sapiens
LGAGIPGLGVGVGVPGLGVGAGVPG

SEQ ID NO: 1724 - protein, 27 aa, Homo sapiens
LGAGIPGLGVGVGVPGLGVGAGVPGLG

SEQ ID NO: 1725 - protein, 29 aa, Homo sapiens
LGAGIPGLGVGVGVPGLGVGAGVPGLGVG

SEQ ID NO: 1726 - protein, 36 aa, Homo sapiens
LGAGIPGLGVGVGVPGLGVGAGVPGLGVGAGVPGFG

SEQ ID NO: 1727 - protein, 17 aa, Homo sapiens
GAGIPGLGVGVGVPGLG

SEQ ID NO: 1728 - protein, 14 aa, Homo sapiens
AGIPGLGVGVGVPG

SEQ ID NO: 1729 - protein, 18 aa, Homo sapiens
GIPGLGVGVGVPGLGVGA

SEQ ID NO: 1730 - protein, 14 aa, Homo sapiens
LGVGVGVPGLGVGA

SEQ ID NO: 1731 - protein, 14 aa, Homo sapiens
VGVPGLGVGAGVPG

SEQ ID NO: 1732 - protein, 15 aa, Homo sapiens
VGVPGLGVGAGVPGL

SEQ ID NO: 1733 - protein, 16 aa, Homo sapiens
VGVPGLGVGAGVPGLG

SEQ ID NO: 1734 - protein, 18 aa, Homo sapiens
VGVPGLGVGAGVPGLGVG

SEQ ID NO: 1735 - protein, 19 aa, Homo sapiens
VGVPGLGVGAGVPGLGVGA

SEQ ID NO: 1736 - protein, 18 aa, Homo sapiens
VGAGVPGLGVGAGVPGFG

SEQ ID NO: 1737 - protein, 8 aa, Homo sapiens
PGALAAAK

SEQ ID NO: 1738 - protein, 16 aa, Homo sapiens
AKYGAAVPGVLGGLGA

SEQ ID NO: 1739 - protein, 11 aa, Homo sapiens
YGAAVPGVLGG

SEQ ID NO: 1740 - protein, 13 aa, Homo sapiens
YGAAVPGVLGGLG

SEQ ID NO: 1741 - protein, 14 aa, Homo sapiens
YGAAVPGVLGGLGA

SEQ ID NO: 1742 - protein, 16 aa, Homo sapiens
YGAAVPGVLGGLGALG

SEQ ID NO: 1743 - protein, 23 aa, Homo sapiens
YGAAVPGVLGGLGALGGVGIPGG

SEQ ID NO: 1744 - protein, 31 aa, Homo sapiens
YGAAVPGVLGGLGALGGVGIPGGVVGAGPAA

SEQ ID NO: 1745 - protein, 12 aa, Homo sapiens
GAAVPGVLGGLG

SEQ ID NO: 1746 - protein, 22 aa, Homo sapiens
GAAVPGVLGGLGALGGVGIPGG

SEQ ID NO: 1747 - protein, 11 aa, Homo sapiens
AVPGVLGGLGA

SEQ ID NO: 1748 - protein, 20 aa, Homo sapiens
AVPGVLGGLGALGGVGIPGG

SEQ ID NO: 1749 - protein, 16 aa, Homo sapiens
VLGGLGALGGVGIPGG

SEQ ID NO: 1750 - protein, 21 aa, Homo sapiens
GGLGALGGVGIPGGVVGAGPA

SEQ ID NO: 1751 - protein, 23 aa, Homo sapiens
GGLGALGGVGIPGGVVGAGPAAA

SEQ ID NO: 1752 - protein, 12 aa, Homo sapiens
LGALGGVGIPGG

SEQ ID NO: 1753 - protein, 19 aa, Homo sapiens
LGALGGVGIPGGVVGAGPA

SEQ ID NO: 1754 - protein, 20 aa, Homo sapiens
LGALGGVGIPGGVVGAGPAA

SEQ ID NO: 1755 - protein, 21 aa, Homo sapiens
LGALGGVGIPGGVVGAGPAAA

SEQ ID NO: 1756 - protein, 22 aa, Homo sapiens
LGALGGVGIPGGVVGAGPAAAA

SEQ ID NO: 1757 - protein, 18 aa, Homo sapiens
ALGGVGIPGGVVGAGPAA

SEQ ID NO: 1758 - protein, 19 aa, Homo sapiens
ALGGVGIPGGVVGAGPAAA

SEQ ID NO: 1759 - protein, 13 aa, Homo sapiens
LGGVGIPGGVSEQ

SEQ ID NO: 1760 - protein, 16 aa, Homo sapiens
LGGVGIPGGVVGAGPA

SEQ ID NO: 1761 - protein, 18 aa, Homo sapiens
LGGVGIPGGVVGAGPAAA

SEQ ID NO: 1762 - protein, 20 aa, Homo sapiens
LGGVGIPGGVVGAGPAAAAA

SEQ ID NO: 1763 - protein, 23 aa, Homo sapiens
LGGVGIPGGVVGAGPAAAAAAAK

SEQ ID NO: 1764 - protein, 17 aa, Homo sapiens
GVGIPGGVVGAGPAAAA

SEQ ID NO: 1765 - protein, 21 aa, Homo sapiens
GVGIPGGVVGAGPAAAAAAAK

SEQ ID NO: 1766 - protein, 15 aa, Homo sapiens
VGIPGGVVGAGPAAA

SEQ ID NO: 1767 - protein, 20 aa, Homo sapiens
VGIPGGVVGAGPAAAAAAAK

SEQ ID NO: 1768 - protein, 14 aa, Homo sapiens
IPGGVVGAGPAAAA

SEQ ID NO: 1769 - protein, 14 aa, Homo sapiens
VVGAGPAAAAAAAK

SEQ ID NO: 1770 - protein, 13 aa, Homo sapiens
VGAGPAAAAAAAK

SEQ ID NO: 1771 - protein, 11 aa, Homo sapiens
AGPAAAAAAAK

SEQ ID NO: 1772 - protein, 10 aa, Homo sapiens
GPAAAAAAAK

SEQ ID NO: 1773 - protein, 9 aa, Homo sapiens
PAAAAAAAK

SEQ ID NO: 1774 - protein, 24 aa, Homo sapiens
FGLVGAAGLGGLGVGGLGVPGVGG

SEQ ID NO: 1775 - protein, 12 aa, Homo sapiens
GLVGAAGLGGLG

SEQ ID NO: 1776 - protein, 15 aa, Homo sapiens
GLVGAAGLGGLGVGG

SEQ ID NO: 1777 - protein, 22 aa, Homo sapiens
GLVGAAGLGGLGVGGLGVPGVG

SEQ ID NO: 1778 - protein, 23 aa, Homo sapiens
GLVGAAGLGGLGVGGLGVPGVGG

SEQ ID NO: 1779 - protein, 13 aa, Homo sapiens
LVGAAGLGGLGVG

SEQ ID NO: 1780 - protein, 13 aa, Homo sapiens
LVGAAGLGGLGVG

SEQ ID NO: 1781 - protein, 15 aa, Homo sapiens
LVGAAGLGGLGVGGL

SEQ ID NO: 1782 - protein, 24 aa, Homo sapiens
LVGAAGLGGLGVGGLGVPGVGGLG

SEQ ID NO: 1783 - protein, 31 aa, Homo sapiens
LVGAAGLGGLGVGGLGVPGVGGLGGIPPAAA

SEQ ID NO: 1784 - protein, 13 aa, Homo sapiens
VGAAGLGGLGVGG

SEQ ID NO: 1785 - protein, 13 aa, Homo sapiens
LGGLGVGGLGVPG

SEQ ID NO: 1786 - protein, 15 aa, Homo sapiens
LGGLGVGGLGVPGVG

SEQ ID NO: 1787 - protein, 17 aa, Homo sapiens
LGGLGVGGLGVPGVGGL

SEQ ID NO: 1788 - protein, 18 aa, Homo sapiens
LGGLGVGGLGVPGVGGLG

SEQ ID NO: 1789 - protein, 15 aa, Homo sapiens
LGVGGLGVPGVGGLG

SEQ ID NO: 1790 - protein, 20 aa, Homo sapiens
GLGVPGVGGLGGIPPAAAAK

SEQ ID NO: 1791 - protein, 11 aa, Homo sapiens
LGGIPPAAAAK

SEQ ID NO: 1792 - protein, 13 aa, Homo sapiens
LGGVLGGAGQFPL

SEQ ID NO: 1793 - protein, 19 aa, Homo sapiens
LGGVLGGAGQFPLGGVAAR

SEQ ID NO: 1794 - protein, 21 aa, Homo sapiens
LGGVLGGAGQFPLGGVAARPG

SEQ ID NO: 1795 - protein, 23 aa, Homo sapiens
LGGVLGGAGQFPLGGVAARPGFG

SEQ ID NO: 1796 - protein, 20 aa, Homo sapiens
GGVLGGAGQFPLGGVAARPG

SEQ ID NO: 1797 - protein, 13 aa, Homo sapiens
GAGQFPLGGVAAR

SEQ ID NO: 1798 - protein, 17 aa, Homo sapiens
GAGQFPLGGVAARPGFG

SEQ ID NO: 1799 - protein, 16 aa, Homo sapiens
AGQFPLGGVAARPGFG

SEQ ID NO: 1800 - protein, 11 aa, Homo sapiens
FPLGGVAARPG

SEQ ID NO: 1801 - protein, 8 aa, Homo sapiens
PLGGVAAR

SEQ ID NO: 1802 - protein, 10 aa, Homo sapiens
PLGGVAARPG

SEQ ID NO: 1803 - protein, 12 aa, Homo sapiens
PLGGVAARPGFG

SEQ ID NO: 1804 - protein, 13 aa, Homo sapiens
PLGGVAARPGFGL

SEQ ID NO: 1805 - protein, 19 aa, Homo sapiens
PLGGVAARPGFGLSPIFPG

SEQ ID NO: 1806 - protein, 7 aa, Homo sapiens
LGGVAAR

SEQ ID NO: 1807 - protein, 8 aa, Homo sapiens
LGGVAARP

SEQ ID NO: 1808 - protein, 9 aa, Homo sapiens
LGGVAARPG

SEQ ID NO: 1809 - protein, 10 aa, Homo sapiens
LGGVAARPGF

SEQ ID NO: 1810 - protein, 11 aa, Homo sapiens
LGGVAARPGFG

SEQ ID NO: 1811 - protein, 12 aa, Homo sapiens
LGGVAARPGFGL

SEQ ID NO: 1812 - protein, 14 aa, Homo sapiens
LGGVAARPGFGLSP

SEQ ID NO: 1813 - protein, 18 aa, Homo sapiens
LGGVAARPGFGLSPIFPG

SEQ ID NO: 1814 - protein, 19 aa, Homo sapiens
LGGVAARPGFGLSPIFPGG

SEQ ID NO: 1815 - protein, 20 aa, Homo sapiens
LGGVAARPGFGLSPIFPGGA

SEQ ID NO: 1816 - protein, 10 aa, Homo sapiens
GGVAARPGFG

SEQ ID NO: 1817 - protein, 11 aa, Homo sapiens
GGVAARPGFGL

SEQ ID NO: 1818 - protein, 19 aa, Homo sapiens
GGVAARPGFGLSPIFPGGA

SEQ ID NO: 1819 - protein, 14 aa, Homo sapiens
GVAARPGFGLSPIF

SEQ ID NO: 1820 - protein, 15 aa, Homo sapiens
GVAARPGFGLSPIFP

SEQ ID NO: 1821 - protein, 8 aa, Homo sapiens
VAARPGFG

SEQ ID NO: 1822 - protein, 14 aa, Homo sapiens
VAARPGFGLSPIFP

SEQ ID NO: 1823 - protein, 15 aa, Homo sapiens
VAARPGFGLSPIFPG

SEQ ID NO: 1824 - protein, 12 aa, Homo sapiens
RPGFGLSPIFPG

SEQ ID NO: 1825 - protein, 12 aa, Homo sapiens
PGFGLSPIFPGG

SEQ ID NO: 1826 - protein, 13 aa, Homo sapiens
PGFGLSPIFPGGA

SEQ ID NO: 1827 - protein, 19 aa, Homo sapiens
PGVGLPGVYPGGVLPGARF

SEQ ID NO: 1828 - protein, 18 aa, Homo sapiens
GVGLPGVYPGGVLPGARF

SEQ ID NO: 1829 - protein, 16 aa, Homo sapiens
GLPGVYPGGVLPGARF

SEQ ID NO: 1830 - protein, 14 aa, Homo sapiens
PGVYPGGVLPGARF

SEQ ID NO: 1831 - protein, 22 aa, Homo sapiens
KAGYPTGTGVGPQAAAAAAAKA

SEQ ID NO: 1832 - protein, 26 aa, Homo sapiens
GGPGFGPGVVGVPGAGVPGVGVPGAG

SEQ ID NO: 1833 - protein, 22 aa, Homo sapiens
GFGPGVVGVPGAGVPGVGVPGA

SEQ ID NO: 1834 - protein, 21 aa, Homo sapiens
FGPGVVGVPGAGVPGVGVPGA

SEQ ID NO: 1835 - protein, 18 aa, Homo sapiens
GVPGVGVPGAGIPVVPGA

SEQ ID NO: 1836 - protein, 18 aa, Homo sapiens
GARPGVGVGGIPTYGVGA

SEQ ID NO: 1837 - protein, 21 aa, Homo sapiens
GARPGVGVGGIPTYGVGAGGF

SEQ ID NO: 1838 - protein, 19 aa, Homo sapiens
ARPGVGVGGIPTYGVGAGG

SEQ ID NO: 1839 - protein, 24 aa, Homo sapiens
GGVPGVGGVPGVGISPEAQAAAAA

SEQ ID NO: 1840 - protein, 19 aa, Homo sapiens
GVPGVGISPEAQAAAAAKA

SEQ ID NO: 1841 - protein, 16 aa, Homo sapiens
GVGISPEAQAAAAAKA

SEQ ID NO: 1842 - protein, 25 aa, Homo sapiens
VPGVGVAPGVGVAPGVGVAPGVGLA

SEQ ID NO: 1843 - protein, 30 aa, Homo sapiens
GVAPGVGVAPGVGVAPGVGLAPGVGVAPGV

SEQ ID NO: 1844 - protein, 22 aa, Homo sapiens
GVGVAPGVGVAPGVGLAPGVGV

SEQ ID NO: 1845 - protein, 28 aa, Homo sapiens
GVGVAPGVGVAPGVGLAPGVGVAPGVGV

SEQ ID NO: 1846 - protein, 26 aa, Homo sapiens
APGVGVAPGVGVAPGVGVAPGIGPGG

SEQ ID NO: 1847 - protein, 22 aa, Homo sapiens
GVAPGVGVAPGVGVAPGIGPGG

SEQ ID NO: 1848 - protein, 21 aa, Homo sapiens
AAVPGVLGGLGALGGVGIPGG

SEQ ID NO: 1849 - protein, 23 aa, Homo sapiens
GAAGLGGLGVGGLGVPGVGGLGG

SEQ ID NO: 1850 - protein, 23 aa, Homo sapiens
GGAGVPGVPGAIPGIGGIAGVGT

SEQ ID NO: 1851 - protein, 22 aa, Homo sapiens
GAGVPGVPGAIPGIGGIAGVGT

SEQ ID NO: 1852 - protein, 18 aa, Homo sapiens
AGVGTPAAAAAAAAAAKA

SEQ ID NO: 1853 - protein, 17 aa, Homo sapiens
GVGTPAAAAAAAAAAKA

SEQ ID NO: 1854 - protein, 25 aa, Homo sapiens
GGPGFGPGVVGVPGAGVPGVGVPGA

SEQ ID NO: 1855 - protein, 19 aa, Homo sapiens
GARPGVGVGGIPTYGVGAG

SEQ ID NO: 1856 - protein, 20 aa, Homo sapiens
ARPGVGVGGIPTYGVGAGGF

SEQ ID NO: 1857 - protein, 28 aa, Homo sapiens
GVGVAPGVGVAPGVGVAPGVGLAPGVGV

SEQ ID NO: 1858 - protein, 26 aa, Homo sapiens
APGVGVAPGVGLAPGVGVAPGVGVAP

SEQ ID NO: 1859 - protein, 22 aa, Homo sapiens
GVGVAPGVGLAPGVGVAPGVGV

SEQ ID NO: 1860 - protein, 27 aa, Homo sapiens
LAPGVGVAPGVGVAPGVGVAPGIGPGG

SEQ ID NO: 1861 - protein, 23 aa, Homo sapiens
YGAAVPGVLGGLGALGGVGIPGG

SEQ ID NO: 1862 - protein, 20 aa, Homo sapiens
GGAGQFPLGGVAARPGFGLS

SEQ ID NO: 1863 - protein, 15 aa, Homo sapiens
LVPGGVADAAAAYKA

SEQ ID NO: 1864 - protein, 12 aa, Homo sapiens
VYPGGVLPGARF

SEQ ID NO: 1865 - protein, 26 aa, Homo sapiens
VAPGVGVAPGVGVAPGVGLAPGVGVA

SEQ ID NO: 1866 - protein, 20 aa, Homo sapiens
LAPGVGVAPGVGVAPGVGVA

SEQ ID NO: 1867 - protein, 23 aa, Homo sapiens
LAPGVGVAPGVGVAPGVGVAPGI

SEQ ID NO: 1868 - protein, 25 aa, Homo sapiens
LAPGVGVAPGVGVAPGVGVAPGIGP

SEQ ID NO: 1869 - protein, 26 aa, Homo sapiens
LAPGVGVAPGVGVAPGVGVAPGIGPG

SEQ ID NO: 1870 - protein, 31 aa, Homo sapiens
LAPGVGVAPGVGVAPGVGVAPGIGPGGVAAA

SEQ ID NO: 1871 - protein, 24 aa, Homo sapiens
GVGVAPGVGVAPGVGVAPGIGPGG

SEQ ID NO: 1872 - protein, 23 aa, Homo sapiens
GAAVPGVLGGLGALGGVGIPGGV

SEQ ID NO: 1873 - protein, 21 aa, Homo sapiens
AAVPGVLGGLGALGGVGIPGG

SEQ ID NO: 1874 - protein, 21 aa, Homo sapiens
AVPGVLGGLGALGGVGIPGGV

SEQ ID NO: 1875 - protein, 18 aa, Homo sapiens
AGQFPLGGVAARPGFGLS

SEQ ID NO: 1876 - protein, 17 aa, Homo sapiens
GALVPGGVADAAAAYKA

SEQ ID NO: 1877 - protein, 17 aa, Homo sapiens
GLPYTTGKLPYGYGPGG

SEQ ID NO: 1878 - protein, 16 aa, Homo sapiens
AAAAAAAKAAAKFGAG

SEQ ID NO: 1879 - protein, 18 aa, Homo sapiens
AAAAAAAAAAKAAKYGAA

SEQ ID NO: 1880 - protein, 26 aa, Homo sapiens
GVAPGVGVAPGVGVAPGVGLAPGVGV

SEQ ID NO: 1881 - protein, 20 aa, Homo sapiens
TFPGALVPGGVADAAAAYKA

SEQ ID NO: 1882 - protein, 21 aa, Homo sapiens
GLPGVYPGGVLPGARFPGVGV

SEQ ID NO: 1883 - protein, 20 aa, Homo sapiens
GYPTGTGVGPQAAAAAAAKA

SEQ ID NO: 1884 - protein, 18 aa, Homo sapiens
GTPAAAAAAAAAAKAAKY

SEQ ID NO: 1885 - protein, 22 aa, Homo sapiens
GVPGAGVPGVGVPGAGIPVVPG

SEQ ID NO: 1886 - protein, 28 aa, Homo sapiens
GVPGAGVPGVGVPGAGIPVVPGAGIPGA

SEQ ID NO: 1887 - protein, 17 aa, Homo sapiens
GISPEAQAAAAAKAAKY

SEQ ID NO: 1888 - protein, 20 aa, Homo sapiens
VPGVGVAPGVGVAPGVGVAP

SEQ ID NO: 1889 - protein, 25 aa, Homo sapiens
GVAPGVGVAPGVGVAPGIGPGGVAA

SEQ ID NO: 1890 - protein, 20 aa, Homo sapiens
GIPGGVVGAGPAAAAAAAKA

SEQ ID NO: 1891 - protein, 23 aa, Homo sapiens
GGVLPGARFPGVGVLPGVPTGAG

SEQ ID NO: 1892 - protein, 19 aa, Homo sapiens
GGVPGVGGVPGVGISPEAQ

SEQ ID NO: 1893 - protein, 22 aa, Homo sapiens
GVGVAPGVGVAPGVGVAPGVGL

SEQ ID NO: 1894 - protein, 20 aa, Homo sapiens
GVPGVPGAIPGIGGIAGVGT

SEQ ID NO: 1895 - protein, 22 aa, Homo sapiens
FGPGVVGVPGAGVPGVGVPGAG

SEQ ID NO: 1896 - protein, 19 aa, Homo sapiens
GVPGVGVPGAGIPVVPGAG

SEQ ID NO: 1897 - protein, 19 aa, Homo sapiens
GVGVAPGVGVAPGVGVAPG

SEQ ID NO: 1898 - protein, 6 aa, Homo sapiens
GVPGAI

SEQ ID NO: 1899 - protein, 6 aa, Homo sapiens
AIPGGV

SEQ ID NO: 1900 - protein, 6 aa, Homo sapiens
GVPGGV

SEQ ID NO: 1901 - protein, 6 aa, Homo sapiens
ALGGGA

SEQ ID NO: 1902 - protein, 6 aa, Homo sapiens
LGGGAL

SEQ ID NO: 1903 - protein, 6 aa, Homo sapiens
GGALGP

SEQ ID NO: 1904 - protein, 6 aa, Homo sapiens
PLKPVP

SEQ ID NO: 1905 - protein, 6 aa, Homo sapiens
LKPVPG

SEQ ID NO: 1906 - protein, 6 aa, Homo sapiens
GLAGAG

SEQ ID NO: 1907 - protein, 6 aa, Homo sapiens
GLGAGL

SEQ ID NO: 1908 - protein, 6 aa, Homo sapiens
LGAGLG

SEQ ID NO: 1909 - protein, 6 aa, Homo sapiens
AGLGAF

SEQ ID NO: 1910 - protein, 6 aa, Homo sapiens
LVPGGV

SEQ ID NO: 1911 - protein, 6 aa, Homo sapiens
VADAAA

SEQ ID NO: 1912 - protein, 6 aa, Homo sapiens
KAAKAG

SEQ ID NO: 1913 - protein, 6 aa, Homo sapiens
PVGYPG

SEQ ID NO: 1914 - protein, 6 aa, Homo sapiens
ARFPGV

SEQ ID NO: 1915 - protein, 6 aa, Homo sapiens
RFPGVG

SEQ ID NO: 1916 - protein, 6 aa, Homo sapiens
VGPFGG

SEQ ID NO: 1917 - protein, 6 aa, Homo sapiens
GPQPGV

SEQ ID NO: 1918 - protein, 6 aa, Homo sapiens
PQPGVP

SEQ ID NO: 1919 - protein, 6 aa, Homo sapiens
TTGKLP

SEQ ID NO: 1920 - protein, 6 aa, Homo sapiens
LPYGYG

SEQ ID NO: 1921 - protein, 6 aa, Homo sapiens
GYGPGG

SEQ ID NO: 1922 - protein, 6 aa, Homo sapiens
FGAGAA

SEQ ID NO: 1923 - protein, 6 aa, Homo sapiens
GVLPGV

SEQ ID NO: 1924 - protein, 6 aa, Homo sapiens
VLPGVG

SEQ ID NO: 1925 - protein, 6 aa, Homo sapiens
AGIPGL

SEQ ID NO: 1926 - protein, 6 aa, Homo sapiens
VPGAIP

SEQ ID NO: 1927 - protein, 6 aa, Homo sapiens
AIPGIG

SEQ ID NO: 1928 - protein, 6 aa, Homo sapiens
TPAAAA

SEQ ID NO: 1929 - protein, 6 aa, Homo sapiens
PAAAAA

SEQ ID NO: 1930 - protein, 6 aa, Homo sapiens
AAAAAA

SEQ ID NO: 1931 - protein, 6 aa, Homo sapiens
VGVPGA

SEQ ID NO: 1932 - protein, 6 aa, Homo sapiens
AVGPGV

SEQ ID NO: 1933 - protein, 6 aa, Homo sapiens
GVPGVG

SEQ ID NO: 1934 - protein, 6 aa, Homo sapiens
GIPVVP

SEQ ID NO: 1935 - protein, 6 aa, Homo sapiens
IPGAAV

SEQ ID NO: 1936 - protein, 6 aa, Homo sapiens
GAAVPG

SEQ ID NO: 1937 - protein, 6 aa, Homo sapiens
ARPGVG

SEQ ID NO: 1938 - protein, 6 aa, Homo sapiens
RPGVGV

SEQ ID NO: 1939 - protein, 6 aa, Homo sapiens
VGGIPT

SEQ ID NO: 1940 - protein, 6 aa, Homo sapiens
SVGGVP

SEQ ID NO: 1941 - protein, 6 aa, Homo sapiens
VGGVPG

SEQ ID NO: 1942 - protein, 6 aa, Homo sapiens
GVGTPA

SEQ ID NO: 1943 - protein, 6 aa, Homo sapiens
VGVAPG

SEQ ID NO: 1944 - protein, 6 aa, Homo sapiens
VAPGVG

SEQ ID NO: 1945 - protein, 6 aa, Homo sapiens
GVAPGV

SEQ ID NO: 1946 - protein, 6 aa, Homo sapiens
GVPVAP

SEQ ID NO: 1947 - protein, 6 aa, Homo sapiens
GAGIPG

SEQ ID NO: 1948 - protein, 6 aa, Homo sapiens
PGGVAA

SEQ ID NO: 1949 - protein, 6 aa, Homo sapiens
LGAGIP

SEQ ID NO: 1950 - protein, 6 aa, Homo sapiens
PGFGPG

SEQ ID NO: 1951 - protein, 6 aa, Homo sapiens
PGVVGV

SEQ ID NO: 1952 - protein, 6 aa, Homo sapiens
PGALAA

SEQ ID NO: 1953 - protein, 6 aa, Homo sapiens
AKYGAA

SEQ ID NO: 1954 - protein, 6 aa, Homo sapiens
YGAAVP

SEQ ID NO: 1955 - protein, 6 aa, Homo sapiens
ALGGVG

SEQ ID NO: 1956 - protein, 6 aa, Homo sapiens
LGGVGI

SEQ ID NO: 1957 - protein, 6 aa, Homo sapiens
GVGIPG

SEQ ID NO: 1958 - protein, 6 aa, Homo sapiens
AGPAAA

SEQ ID NO: 1959 - protein, 6 aa, Homo sapiens
GPAAAA

SEQ ID NO: 1960 - protein, 6 aa, Homo sapiens
FGLVGA

SEQ ID NO: 1961 - protein, 6 aa, Homo sapiens
GLGVPG

SEQ ID NO: 1962 - protein, 6 aa, Homo sapiens
LGGIPP

SEQ ID NO: 1963 - protein, 6 aa, Homo sapiens
LGGVLG

SEQ ID NO: 1964 - protein, 6 aa, Homo sapiens
PLGGVA

SEQ ID NO: 1965 - protein, 6 aa, Homo sapiens
LGGVAA

SEQ ID NO: 1966 - protein, 6 aa, Homo sapiens
GGVAAR

SEQ ID NO: 1967 - protein, 6 aa, Homo sapiens
GVGLPG

SEQ ID NO: 1968 - protein, 6 aa, Homo sapiens
VGLPGV

SEQ ID NO: 1969 - protein, 6 aa, Homo sapiens
LPGVYP

SEQ ID NO: 1970 - protein, 6 aa, Homo sapiens
VPGVPV

SEQ ID NO: 1971 - protein, 6 aa, Homo sapiens
VPGVGI

SEQ ID NO: 1972 - protein, 6 aa, Homo sapiens
VGISPE

SEQ ID NO: 1973 - protein, 6 aa, Homo sapiens
APGVGV

SEQ ID NO: 1974 - protein, 6 aa, Homo sapiens
VPGGVA

SEQ ID NO: 1975 - protein, 6 aa, Homo sapiens
YPGGVL

SEQ ID NO: 1976 - protein, 6 aa, Homo sapiens
GPGFGP

SEQ ID NO: 1977 - protein, 6 aa, Homo sapiens
YPTGTG

SEQ ID NO: 1978 - protein, 6 aa, Homo sapiens
VPGAGV

SEQ ID NO: 1979 - protein, 6 aa, Homo sapiens
VPGGVF

SEQ ID NO: 1980 - protein, 6 aa, Homo sapiens
GVFYPG

SEQ ID NO: 1981 - protein, 6 aa, Homo sapiens
VFYPGA

SEQ ID NO: 1982 - protein, 6 aa, Homo sapiens
LGPGGK

SEQ ID NO: 1983 - protein, 6 aa, Homo sapiens
GPGGKP

SEQ ID NO: 1984 - protein, 6 aa, Homo sapiens
PGGKPL

SEQ ID NO: 1985 - protein, 6 aa, Homo sapiens
LAGAGL

SEQ ID NO: 1986 - protein, 6 aa, Homo sapiens
AGAGLG

SEQ ID NO: 1987 - protein, 6 aa, Homo sapiens
GAGLGA

SEQ ID NO: 1988 - protein, 6 aa, Homo sapiens
LGAFPA

SEQ ID NO: 1989 - protein, 6 aa, Homo sapiens
AFPAVT

SEQ ID NO: 1990 - protein, 6 aa, Homo sapiens
AVTFPG

SEQ ID NO: 1991 - protein, 6 aa, Homo sapiens
LGVSAG

SEQ ID NO: 1992 - protein, 6 aa, Homo sapiens
VPGVGL

SEQ ID NO: 1993 - protein, 6 aa, Homo sapiens
PGVGLP

SEQ ID NO: 1994 - protein, 6 aa, Homo sapiens
FPGVGV

SEQ ID NO: 1995 - protein, 6 aa, Homo sapiens
KPGAPG

SEQ ID NO: 1996 - protein, 6 aa, Homo sapiens
PGVPLG

SEQ ID NO: 1997 - protein, 6 aa, Homo sapiens
GYPIKA

SEQ ID NO: 1998 - protein, 6 aa, Homo sapiens
PKLPGG

SEQ ID NO: 1999 - protein, 6 aa, Homo sapiens
YGPGGV

SEQ ID NO: 2000 - protein, 6 aa, Homo sapiens
AGYPTG

SEQ ID NO: 2001 - protein, 6 aa, Homo sapiens
TGVGPQ

SEQ ID NO: 2002 - protein, 6 aa, Homo sapiens
GAGVPG

SEQ ID NO: 2003 - protein, 6 aa, Homo sapiens
AGVPGV

SEQ ID NO: 2004 - protein, 6 aa, Homo sapiens
GVPGVP

SEQ ID NO: 2005 - protein, 6 aa, Homo sapiens
IPGIGG

SEQ ID NO: 2006 - protein, 6 aa, Homo sapiens
IGGIAG

SEQ ID NO: 2007 - protein, 6 aa, Homo sapiens
GIAGVG

SEQ ID NO: 2008 - protein, 6 aa, Homo sapiens
VPGVGV

SEQ ID NO: 2009 - protein, 6 aa, Homo sapiens
VPVGVA

SEQ ID NO: 2010 - protein, 6 aa, Homo sapiens
VPGAGI

SEQ ID NO: 2011 - protein, 6 aa, Homo sapiens
AVPGVV

SEQ ID NO: 2012 - protein, 6 aa, Homo sapiens
VPGVVS

SEQ ID NO: 2013 - protein, 6 aa, Homo sapiens
YGARPG

SEQ ID NO: 2014 - protein, 6 aa, Homo sapiens
GVGAGG

SEQ ID NO: 2015 - protein, 6 aa, Homo sapiens
VGAGGF

SEQ ID NO: 2016 - protein, 6 aa, Homo sapiens
VGVGGI

SEQ ID NO: 2017 - protein, 6 aa, Homo sapiens
FGLVPG

SEQ ID NO: 2018 - protein, 6 aa, Homo sapiens
GLVPGV

SEQ ID NO: 2019 - protein, 6 aa, Homo sapiens
LVPGVG

SEQ ID NO: 2020 - protein, 6 aa, Homo sapiens
PGVGLA

SEQ ID NO: 2021 - protein, 6 aa, Homo sapiens
GVGLAP

SEQ ID NO: 2022 - protein, 6 aa, Homo sapiens
VGLAPG

SEQ ID NO: 2023 - protein, 6 aa, Homo sapiens
LRAAAG

SEQ ID NO: 2024 - protein, 6 aa, Homo sapiens
LVGAAG

SEQ ID NO: 2025 - protein, 6 aa, Homo sapiens
LVPGGP

SEQ ID NO: 2026 - protein, 6 aa, Homo sapiens
GIPGLG

SEQ ID NO: 2027 - protein, 6 aa, Homo sapiens
LGVGVG

SEQ ID NO: 2028 - protein, 6 aa, Homo sapiens
VGVPGL

SEQ ID NO: 2029 - protein, 6 aa, Homo sapiens
AAAGLG

SEQ ID NO: 2030 - protein, 6 aa, Homo sapiens
AVPGVL

SEQ ID NO: 2031 - protein, 6 aa, Homo sapiens
VLGGLG

SEQ ID NO: 2032 - protein, 6 aa, Homo sapiens
VGIPGG

SEQ ID NO: 2033 - protein, 6 aa, Homo sapiens
IPGGVV

SEQ ID NO: 2034 - protein, 6 aa, Homo sapiens
VVGAGP

SEQ ID NO: 2035 - protein, 6 aa, Homo sapiens
GLVGAA

SEQ ID NO: 2036 - protein, 6 aa, Homo sapiens
VGAAGL

SEQ ID NO: 2037 - protein, 6 aa, Homo sapiens
LGGLGV

SEQ ID NO: 2038 - protein, 6 aa, Homo sapiens
GGVLGG

SEQ ID NO: 2039 - protein, 6 aa, Homo sapiens
GAGQFP

SEQ ID NO: 2040 - protein, 6 aa, Homo sapiens
AFQFPL

SEQ ID NO: 2041 - protein, 6 aa, Homo sapiens
GVAARP

SEQ ID NO: 2042 - protein, 6 aa, Homo sapiens
VAARPG

SEQ ID NO: 2043 - protein, 6 aa, Homo sapiens
RPGFGL

SEQ ID NO: 2044 - protein, 6 aa, Homo sapiens
GVYPGG

SEQ ID NO: 2045 - protein, 6 aa, Homo sapiens
LPYTTG

SEQ ID NO: 2046 - protein, 6 aa, Homo sapiens
FGPGVV

SEQ ID NO: 2047 - protein, 6 aa, Homo sapiens
AAVPGV

SEQ ID NO: 2048 - protein, 6 aa, Homo sapiens
AAGLGG

SEQ ID NO: 2049 - protein, 6 aa, Homo sapiens
FPGALV

SEQ ID NO: 2050 - protein, 6 aa, Homo sapiens
VPGVLG

SEQ ID NO: 2051 - protein, 6 aa, Homo sapiens
GQFPLG

SEQ ID NO: 2052 - protein, 6 aa, Homo sapiens
ALVPGG

SEQ ID NO: 2053 - protein, 6 aa, Homo sapiens
ISPEAQ

SEQ ID NO: 2054 - protein, 6 aa, Homo sapiens
GVLPGA

SEQ ID NO: 2055 - protein, 6 aa, Homo sapiens
VGAGVP

SEQ ID NO: 2056 - protein, 6 aa, Homo sapiens
LGALGG

SEQ ID NO: 2057 - protein, 6 aa, Homo sapiens
VPGVPG

SEQ ID NO: 2058 - protein, 6 aa, Homo sapiens
GGLGAL

SEQ ID NO: 2059 - protein, 6 aa, Homo sapiens
GKPLKP

SEQ ID NO: 2060 - protein, 6 aa, Homo sapiens
IAGVGT

SEQ ID NO: 2061 - protein, 6 aa, Homo sapiens
VGAGPA

SEQ ID NO: 2062 - protein, 6 aa, Homo sapiens
AGLGAG

SEQ ID NO: 2063 - protein, 6 aa, Homo sapiens
VVGVPG

SEQ ID NO: 2064 - protein, 6 aa, Homo sapiens
LGVGGL

SEQ ID NO: 2065 - protein, 6 aa, Homo sapiens
VTFPGA

SEQ ID NO: 2066 - protein, 6 aa, Homo sapiens
AGIPVV

SEQ ID NO: 2067 - protein, 6 aa, Homo sapiens
FPLGGV

SEQ ID NO: 2068 - protein, 6 aa, Homo sapiens
GLPGVY

SEQ ID NO: 2069 - protein, 6 aa, Homo sapiens
GARPGV

SEQ ID NO: 2070 - protein, 6 aa, Homo sapiens
PGFGLS

SEQ ID NO: 2071 - protein, 6 aa, Homo sapiens
GAFAGI

SEQ ID NO: 2072 - protein, 6 aa, Homo sapiens
VAGVPS

SEQ ID NO: 2073 - protein, 6 aa, Homo sapiens
GPGVVG

SEQ ID NO: 2074 - protein, 6 aa, Homo sapiens
YTTGKL

SEQ ID NO: 2075 - protein, 6 aa, Homo sapiens
PGVGVA

SEQ ID NO: 2076 - protein, 6 aa, Homo sapiens
VGTPAA

SEQ ID NO: 2077 - protein, 6 aa, Homo sapiens
PQAAAA

SEQ ID NO: 2078 - protein, 6 aa, Homo sapiens
LAPGVG

SEQ ID NO: 2079 - protein, 6 aa, Homo sapiens
PGGVPG

SEQ ID NO: 2080 - protein, 6 aa, Homo sapiens
PGAGLG

SEQ ID NO: 2081 - protein, 6 aa, Homo sapiens
GALGGG

SEQ ID NO: 2082 - protein, 6 aa, Homo sapiens
GGGALG

SEQ ID NO: 2083 - protein, 6 aa, Homo sapiens
GLGAFP

SEQ ID NO: 2084 - protein, 6 aa, Homo sapiens
ADAAAA

SEQ ID NO: 2085 - protein, 6 aa, Homo sapiens
PGVLGG

SEQ ID NO: 2086 - protein, 6 aa, Homo sapiens
VGVLPG

SEQ ID NO: 2087 - protein, 6 aa, Homo sapiens
VPTGAG

SEQ ID NO: 2088 - protein, 6 aa, Homo sapiens
GVGPFG

SEQ ID NO: 2089 - protein, 6 aa, Homo sapiens
VPLGYP

SEQ ID NO: 2090 - protein, 6 aa, Homo sapiens
AAAAAK

SEQ ID NO: 2091 - protein, 6 aa, Homo sapiens
AAAAKA

SEQ ID NO: 2092 - protein, 6 aa, Homo sapiens
GVGVPG

SEQ ID NO: 2093 - protein, 6 aa, Homo sapiens
PVVPGA

SEQ ID NO: 2094 - protein, 6 aa, Homo sapiens
VVSPEA

SEQ ID NO: 2095 - protein, 6 aa, Homo sapiens
GGIPTY

SEQ ID NO: 2096 - protein, 6 aa, Homo sapiens
GIPTYG

SEQ ID NO: 2097 - protein, 6 aa, Homo sapiens
GVGVGG

SEQ ID NO: 2098 - protein, 6 aa, Homo sapiens
GVGGIP

SEQ ID NO: 2099 - protein, 6 aa, Homo sapiens
GFPGFG

SEQ ID NO: 2100 - protein, 6 aa, Homo sapiens
FGVGVG

SEQ ID NO: 2101 - protein, 6 aa, Homo sapiens
PGVGIS

SEQ ID NO: 2102 - protein, 6 aa, Homo sapiens
SPEAQA

SEQ ID NO: 2103 - protein, 6 aa, Homo sapiens
GVGVAP

SEQ ID NO: 2104 - protein, 6 aa, Homo sapiens
APGVGL

SEQ ID NO: 2105 - protein, 6 aa, Homo sapiens
GIGPGG

SEQ ID NO: 2106 - protein, 6 aa, Homo sapiens
APGIGP

SEQ ID NO: 2107 - protein, 6 aa, Homo sapiens
VAPGIG

SEQ ID NO: 2108 - protein, 6 aa, Homo sapiens
RAAAGL

SEQ ID NO: 2109 - protein, 6 aa, Homo sapiens
AAGLGA

SEQ ID NO: 2110 - protein, 6 aa, Homo sapiens
GVPGLG

SEQ ID NO: 2111 - protein, 6 aa, Homo sapiens
GVPGFG

SEQ ID NO: 2112 - protein, 6 aa, Homo sapiens
AGVPGL

SEQ ID NO: 2113 - protein, 6 aa, Homo sapiens
GAGPAA

SEQ ID NO: 2114 - protein, 6 aa, Homo sapiens
VPGVGG

SEQ ID NO: 2115 - protein, 6 aa, Homo sapiens
GLGGLG

SEQ ID NO: 2116 - protein, 6 aa, Homo sapiens
PGVGGL

SEQ ID NO: 2117 - protein, 6 aa, Homo sapiens
PAAAAK

SEQ ID NO: 2118 - protein, 6 aa, Homo sapiens
AARPGF

SEQ ID NO: 2119 - protein, 6 aa, Homo sapiens
LSPIFP

SEQ ID NO: 2120 - protein, 6 aa, Homo sapiens
AQAAAA

SEQ ID NO: 2121 - protein, 6 aa, Homo sapiens
GPGIPG

SEQ ID NO: 2122 - protein, 6 aa, Homo sapiens
GPGGVA

SEQ ID NO: 2123 - protein, 6 aa, Homo sapiens
GLGALG

SEQ ID NO: 2124 - protein, 6 aa, Homo sapiens
ALGPGG

SEQ ID NO: 2125 - protein, 6 aa, Homo sapiens
GALGPG

SEQ ID NO: 2126 - protein, 6 aa, Homo sapiens
VAPVGV

SEQ ID NO: 2127 - protein, 6 aa, Homo sapiens
KPVPGG

SEQ ID NO: 2128 - protein, 6 aa, Homo sapiens
AAAAYK

SEQ ID NO: 2129 - protein, 6 aa, Homo sapiens
AAKAGA

SEQ ID NO: 2130 - protein, 6 aa, Homo sapiens
VPQPGA

SEQ ID NO: 2131 - protein, 6 aa, Homo sapiens
PGVPTG

SEQ ID NO: 2132 - protein, 6 aa, Homo sapiens
GVPTGA

SEQ ID NO: 2133 - protein, 6 aa, Homo sapiens
AGVKPK

SEQ ID NO: 2134 - protein, 6 aa, Homo sapiens
PIKAPK

SEQ ID NO: 2135 - protein, 6 aa, Homo sapiens
KLPGGY

SEQ ID NO: 2136 - protein, 6 aa, Homo sapiens
YGYGPG

SEQ ID NO: 2137 - protein, 6 aa, Homo sapiens
GIGGIA

SEQ ID NO: 2138 - protein, 6 aa, Homo sapiens
GTPAAA

SEQ ID NO: 2139 - protein, 6 aa, Homo sapiens
IPVVPG

SEQ ID NO: 2140 - protein, 6 aa, Homo sapiens
GVPGAG

SEQ ID NO: 2141 - protein, 6 aa, Homo sapiens
PEAAAK

SEQ ID NO: 2142 - protein, 6 aa, Homo sapiens
PTYGVG

SEQ ID NO: 2143 - protein, 6 aa, Homo sapiens
TYGVGA

SEQ ID NO: 2144 - protein, 6 aa, Homo sapiens
YGVGAG

SEQ ID NO: 2145 - protein, 6 aa, Homo sapiens
IPTYGV

SEQ ID NO: 2146 - protein, 6 aa, Homo sapiens
PGAIPG

SEQ ID NO: 2147 - protein, 6 aa, Homo sapiens
AGGFPG

SEQ ID NO: 2148 - protein, 6 aa, Homo sapiens
GIPGVA

SEQ ID NO: 2149 - protein, 6 aa, Homo sapiens
GISPEA

SEQ ID NO: 2150 - protein, 6 aa, Homo sapiens
VPGAPG

SEQ ID NO: 2151 - protein, 6 aa, Homo sapiens
GGVAAA

SEQ ID NO: 2152 - protein, 6 aa, Homo sapiens
PGIGPG

SEQ ID NO: 2153 - protein, 6 aa, Homo sapiens
GLGVGG

SEQ ID NO: 2154 - protein, 6 aa, Homo sapiens
PGLGVG

SEQ ID NO: 2155 - protein, 6 aa, Homo sapiens
GLGVGA

SEQ ID NO: 2156 - protein, 6 aa, Homo sapiens
ALAAAK

SEQ ID NO: 2157 - protein, 6 aa, Homo sapiens
LGGLGA

SEQ ID NO: 2158 - protein, 6 aa, Homo sapiens
GGLGVG

SEQ ID NO: 2159 - protein, 6 aa, Homo sapiens
GVGGLG

SEQ ID NO: 2160 - protein, 6 aa, Homo sapiens
AGQFPL

SEQ ID NO: 2161 - protein, 6 aa, Homo sapiens
GFGLSP

SEQ ID NO: 2162 - protein, 6 aa, Homo sapiens
PIFPGG

SEQ ID NO: 2163 - protein, 6 aa, Homo sapiens
IFPGGA

SEQ ID NO: 2164 - protein, 6 aa, Homo sapiens
AAKFGA

SEQ ID NO: 2165 - protein, 6 aa, Homo sapiens
AAKYGA

SEQ ID NO: 2166 - protein, 6 aa, Homo sapiens
AAKAAK

SEQ ID NO: 2167 - protein, 6 aa, Homo sapiens
AGLGAL

SEQ ID NO: 2168 - protein, 6 aa, Homo sapiens
GIPGGV

SEQ ID NO: 2169 - protein, 6 aa, Homo sapiens
PGVGVG

SEQ ID NO: 2170 - protein, 6 aa, Homo sapiens
IPPAAA

SEQ ID NO: 2171 - protein, 6 aa, Homo sapiens
ARPGFG

SEQ ID NO: 2172 - protein, 6 aa, Homo sapiens
VLPGAR

SEQ ID NO: 2173 - protein, 6 aa, Homo sapiens
GGFPGF

SEQ ID NO: 2174 - protein, 6 aa, Homo sapiens
GLSPIF

SEQ ID NO: 2175 - protein, 6 aa, Homo sapiens
PTGAGV

SEQ ID NO: 2176 - protein, 6 aa, Homo sapiens
AGAAGK

SEQ ID NO: 2177 - protein, 10 aa, Homo sapiens
RLRSSVPGVR

SEQ ID NO: 2178 - protein, 10 aa, Homo sapiens
RLRSSVPGVL

SEQ ID NO: 2179 - protein, 10 aa, Homo sapiens
LLQDSVDFSL

SEQ ID NO: 2180 - protein, 10 aa, Homo sapiens
FADLSEAANR

SEQ ID NO: 2181 - protein, 10 aa, Homo sapiens
ISLPLPTFSS

SEQ ID NO: 2182 - protein, 6 aa, Homo sapiens
LLQDSV

SEQ ID NO: 2183 - protein, 6 aa, Homo sapiens
FADLSE

SEQ ID NO: 2184 - protein, 6 aa, Homo sapiens
ISLPLP

SEQ ID NO: 2185 - protein, 6 aa, Homo sapiens
SVPGVR

SEQ ID NO: 2186 - protein, 6 aa, Homo sapiens
SVPGVL

SEQ ID NO: 2187 - protein, 6 aa, Homo sapiens
GPPGIC

SEQ ID NO: 2188 - protein, 6 aa, Homo sapiens
LPGAAG

SEQ ID NO: 2189 - protein, 6 aa, Homo sapiens
APGPLG

SEQ ID NO: 2190 - protein, 9 aa, Homo sapiens
ILGHVPGML

SEQ ID NO: 2191 - protein, 17 aa, Homo sapiens
PGLPGQPGPPGLPVPGQ

SEQ ID NO: 2192 - protein, 42 aa, Homo sapiens
SGYPGNPGLPGIPGQDGPPGPPGIPGCNGTKGERGPLGPPGL

SEQ ID NO: 2193 - protein, 11 aa, Homo sapiens
VSGPPGVPGQA

SEQ ID NO: 2194 - protein, 12 aa, Homo sapiens
VSGPPGVPGQAQ

SEQ ID NO: 2195 - protein, 20 aa, Homo sapiens
KRGPPGPPGLPGPPGPDGFL

SEQ ID NO: 2196 - protein, 15 aa, Homo sapiens
LHGFPGAPGQEGPLG

SEQ ID NO: 2197 - protein, 18 aa, Homo sapiens
LPGPDGPPGERGLPGEVL

SEQ ID NO: 2198 - protein, 7 aa, Homo sapiens
LRGIPGF

SEQ ID NO: 2199 - protein, 21 aa, Homo sapiens
PGFPGAPGTVGAPGIAGIPQK

SEQ ID NO: 2200 - protein, 9 aa, Homo sapiens
QQGNRGLGF

SEQ ID NO: 2201 - protein, 14 aa, Homo sapiens
VGQPGPNGIPSDTL

SEQ ID NO: 2202 - protein, 43 aa, Homo sapiens
GEPGMQGEPGPPGPPGNLGPCGPRGKPGKDGKPGTPGPAGEKG

SEQ ID NO: 2203 - protein, 39 aa, Homo sapiens
GEPGPPGPPGNLGPCGPRGKPGKDGKPGTPGPAGEKGNK

SEQ ID NO: 2204 - protein, 23 aa, Homo sapiens
PGIPGTPGPPGLPGLQGPVGPPG

SEQ ID NO: 2205 - protein, 8 aa, Homo sapiens
PGDIVFRK

SEQ ID NO: 2206 - protein, 17 aa, Homo sapiens
GNKGDPASHFGPPGPKG

SEQ ID NO: 2207 - protein, 9 aa, Homo sapiens
PGPRGKPGM

SEQ ID NO: 2208 - protein, 12 aa, Homo sapiens
PGLPGQPGTRGL

SEQ ID NO: 2209 - protein, 40 aa, Homo sapiens
PGPPGPLGIPGRSGVPGLKGDDGLQGQPGLPGPTGEKGSK

SEQ ID NO: 2210 - protein, 41 aa, Homo sapiens
PGPPGPLGIPGRSGVPGLKGDDGLQGQPGLPGPTGEKGSKG

SEQ ID NO: 2211 - protein, 40 aa, Homo sapiens
SKGEKGEPGLPGIPGVSGPKGYQGLPGDPGQPGLSGQPGL

SEQ ID NO: 2212 - protein, 6 aa, Homo sapiens
ILGHVP

SEQ ID NO: 2213 - protein, 6 aa, Homo sapiens
PGLPGQ

SEQ ID NO: 2214 - protein, 6 aa, Homo sapiens
LPGPDG

SEQ ID NO: 2215 - protein, 6 aa, Homo sapiens
PGDIVF

SEQ ID NO: 2216 - protein, 6 aa, Homo sapiens
GNKGDP

SEQ ID NO: 2217 - protein, 6 aa, Homo sapiens
SGYPGN

SEQ ID NO: 2218 - protein, 6 aa, Homo sapiens
PGFPGA

SEQ ID NO: 2219 - protein, 6 aa, Homo sapiens
PGPRGK

SEQ ID NO: 2220 - protein, 6 aa, Homo sapiens
VSGPPG

SEQ ID NO: 2221 - protein, 6 aa, Homo sapiens
QQGNRG

SEQ ID NO: 2222 - protein, 6 aa, Homo sapiens
VGQPGP

SEQ ID NO: 2223 - protein, 6 aa, Homo sapiens
KRGPPG

SEQ ID NO: 2224 - protein, 6 aa, Homo sapiens
GEPGMQ

SEQ ID NO: 2225 - protein, 6 aa, Homo sapiens
LHGFPG

SEQ ID NO: 2226 - protein, 6 aa, Homo sapiens
SKGEKG

SEQ ID NO: 2227 - protein, 6 aa, Homo sapiens
PGIPGT

SEQ ID NO: 2228 - protein, 6 aa, Homo sapiens
HVPGML

SEQ ID NO: 2229 - protein, 6 aa, Homo sapiens
LPVPGQ

SEQ ID NO: 2230 - protein, 6 aa, Homo sapiens
LGPPGL

SEQ ID NO: 2231 - protein, 6 aa, Homo sapiens
GVPGQA

SEQ ID NO: 2232 - protein, 6 aa, Homo sapiens
VPGQAQ

SEQ ID NO: 2233 - protein, 6 aa, Homo sapiens
GPDGFL

SEQ ID NO: 2234 - protein, 6 aa, Homo sapiens
QEGPLG

SEQ ID NO: 2235 - protein, 6 aa, Homo sapiens
LPGEVL

SEQ ID NO: 2236 - protein, 6 aa, Homo sapiens
RGIPGF

SEQ ID NO: 2237 - protein, 6 aa, Homo sapiens
AGIPQK

SEQ ID NO: 2238 - protein, 6 aa, Homo sapiens
NRGLGF

SEQ ID NO: 2239 - protein, 6 aa, Homo sapiens
IPSDTL

SEQ ID NO: 2240 - protein, 6 aa, Homo sapiens
PAGEKG

SEQ ID NO: 2241 - protein, 6 aa, Homo sapiens
GEKGNK

SEQ ID NO: 2242 - protein, 6 aa, Homo sapiens
PVGPPG

SEQ ID NO: 2243 - protein, 6 aa, Homo sapiens
DIVFRK

SEQ ID NO: 2244 - protein, 6 aa, Homo sapiens
RGKPGM

SEQ ID NO: 2245 - protein, 6 aa, Homo sapiens
PGTRGL

SEQ ID NO: 2246 - protein, 6 aa, Homo sapiens
GEKGSK

SEQ ID NO: 2247 - protein, 6 aa, Homo sapiens
EKGSKG

SEQ ID NO: 2248 - protein, 6 aa, Homo sapiens
SGQPGL